European Patent Specification EP 3 414 343 B1, published April 3, 2024. Title: METHODS FOR ASSESSING THE TREATMENT RESPONSE OF TNBC PATIENTS TO NEO-ADJUVANT CHEMOTHERAPY BY ANALYSING CpG METHYLATION. Applicant: Therawis Diagnostics GmbH. The sequence listing filed with the application follows.

SEQUENCE LISTING (71 sequences)

SEQ ID NO: 1 - DNA, 32001 bp, Homo sapiens
catggactgcgtgatcactaaacttggcacttcagggggcatatcttttttgagtaactctcataaacatgcctgcctgcaggacatccagattttctggtttggtagtaaagcaacataagaataatcttgaacctgatgttcatccttgccttctttctaattccaggagccctctgaggtctggactaactcactgattaggaaatagtatttggaaaggctaaacaaaatactatttccagggaaatagtatttggaaaggctaaacaaaatatactttcttagttttctcaaacctctcagaagatatattttttaaaaaataaactaagctagcaacatttaaactaaatctttgccttgcttacaatacaaaagatgataaaaaaattgttgggaaggtgagaaattaacttcacctataattagaagtaaagttttcatttaaaaatgtaataccacttaaattcaatttgggaaacaaaaaggactcaaaaaacagtctgctaaagccaatttgcaaacaagtgcgctctctttttctttaagttgtatctcaggttcagagcacatgtgcaggtttgttatgtaggtaaacctgtcacagggatttgttgtacagattattttgtcacccaggtactaagcctcgtacccaatagttattttttctgatcctctcccctctcccatccgccaccttccaataggccccagtgtctgttgttcctctctttgtatctatgagttctcctcatttagctcccacttataagtgagaacatgcgttatttggttttctggtcctgatttagtttgctaaggataatggcctccagctccatccatatttctgcaaaaggcatgatctcattctttttttaactattccactctctctattactctttcttcttcccccaatcctgaaccctaccatgtcagtttaaccactccttttctttcctttttctttgctcatttgcacatagttaaaagatgccatgaatttttctttttaattcagcatatgcccattaaagatctaaaaatattatttacatcatccagaactcagcttaagaaattaccaaaaaataaagctaccagaaagtaactgaatcatcttgttgagccacaatcctagacctcgactctgctttttcctcattttaggcaggtcattccttttcctttcttaaattgttttctctgtattcaataacacattcttgtggattcagaaagggtggagtatgaggaaaaggaatatgatatatgtaccctagaggaaaacaataaataaatatttcaggatggaaaacattatttttatttttattgagttttctagagtctatttgatttgtgtaaatcagaaaccagtagaatgacattaatgaattaatgaaaagcagaatgagttatcagttgtaacaaaaagaataaagaatttcaagaacacagctttaatcatgcatggctgcggggagagaaaaataacaaaatgctctcagtgaatacatctctgagagaagaaaggaaatacttaaggagaggataaaaagagcaaatatcaaaaataggagtaagaaccctattgctttttttagttgacaaataaaaattgtatatatttactgtggacaacatgatattttgaggattacgatcacttttgattcataaattacattcaagaaaaagaaattctcaaaaagtttgggaacatatgaagttgaaagaacattaatactcagataaggacagtacatgacaaattattcttgctccaacattttctctcaggaaatttaaacatctttcagtgaagcaccagtttcttgaaatcaagcatgagaaaaaaaactaaattcacctgtggaaaaaaagacacagctaaacaaaaaagcggttgttataacctcaagagtggcatgaacaaaatgatcaacattctcccaagtgacagcacaaatatcaaaagtcctaataagtggaagtggtcctgtcatgacaaaaggtgtggtatttgtacaatttccagataagaacaaagtcatgacgctaagacagtagcagcactgtttgttacacgtgatatttgaaaaatatgacaaccatctcaatctgctcaagtagcactcatggtgagggtgaaattttatcaacattggttaacttatggtgttttaaaaaactagcaaggagataaattgatggattaaaagataaactactcacaggcagacaaacagaaggacagatagagttacaatcaaacatgtactttactcaggcagaaagataataaccagcccccaagaagtgatgtgtctgctagaaaagccctgaacatagaatttcctgactttgtttttaatttagttctttcaggcatcacgctgcataaccaggtgtaactctctaaaagtctctatgacagaattttccatctgttaaattaggctaataatattttcatctttttttagggtaaagatgtgaaatatttggagaactctggaaaacatgccccctactaattagagctttttgatgtgacatcattttcttcagtacttggagtttagtcaatagatatacagtgtagctgtgaaattatgaagcatgagaatgcattaccaagggaccgtaggaggctctttactgaaaagtgtagctggctatatttctggaagtaatttaaacataggctgagggagaggagtaccctctagatcctttccagaccttactttctatgaattctaatttctctttcccatttagaaaaaacaatgagatccacagcgtagagatagaaaataaggctctgtgtgccctcaaaccttactttcaaaaataccacagcattctggacgagatagtcttgaattcttgcaacagcacaggtatgagagtttttaccagaaaacaggagactggattgattctttcattctcctcctatgcttcctaaaactgaaaagccatatatacaaattatatttatctatccctcctggaaaaggccaaaatgaatccaattttggatcattttcaataatgggacaaacctgaattgagaataacctttagaatcagtcctgtctttttgtgataaaatggacttgtagaaagctacctggtgttctcccctagctaacattctaccacaaacaacgggtatgtaatccagtattgctccccacaggctatgtccttggaatcactatctttgcactccatttgtctgctgacatccttccacccaagatgtcttcttcagcacaagaagtcatttctcttaaaatttcaaatgactttactacaataatagagttgctaactagacctaggcaagtaatgataataaaaatctgatttctacttagagtgtagcatggtttaacacaacaaccagagtcctaacaggtttttctagatttcactcctactcaacttgcatgttcttgcaatatagatgttcttattactcggtccttacttccatctctctttgcttctggaataaaactacttaaacccaattcagagattttattctcccttggaattactgggaaacagttctagtaaaccatattcctgagatcctatattaggcttagtccaaactgaccatctaagcattaattttcctgtggctcaggaatatccctgagcttacctttctcttcctaaactgcccaggacaaataccggagtttggcttttctgctttctcatccaatcatttctcgtttcctcctctttagcatttaaaacatttctgactttctccatccctcaagaaatatatttgctttcctgtctctgcattattcttttgtttatgaaatattccataggtaagttctatatttccttcccccagaggcccctggtcttctggttccagttgccattggttcagtgtactagttaacattttggactttggagttacacaaacctagattcaaattcccactatgccacttactgcctacgtgacctgaagcaatatcctatccactgtggcctccagcagttataagcttgtgctctaaccagctgggtgaccttgggccagtgacacaatcatggcaaacctcactgtcttcatttgtaaaatgacagtacctaccttgtagtgttggcataaggaataagtgtgattgtcaatacaaaagtgtttagtacaatagctaaattaactaagcactctgtaaatattagtttttaccattattactaattcaaatgactagatgcattttgtgtataccaggtttcctgagttcactttgttctcaacaaatactattattcctagcatgtggcctatatcacacttcattagccagaggacatgtgaagcttagagtggaaagctagggcagcaggaagcattgccacactttacacagtcaaagccatttaaacatgtctgaatttgagctctgctgagtccttacttgcccccatctctcctgtgtgctccagcttactaataaagcaggtttaatataaatacactaaaagcctaaacattgagatcatgataatgaatatgagggctatgactataaaatatcattgaaccagagacctgctacgaaaccacatggtgaagaccacaagggaggaatctgcatacacaccgagtgccttgggatcccaaagtgggaagagtcagtgccccaattaaagagaaactcggggtagggaatcaaccacaacatcagtcaccttactgaacccaggcttgtttcagctgacgtagctgccaatttccaatgtcccctccctccctaattgctctcaatctattcctccagaaactgaaagcccatcaaagaggatatcttcccagagagttgttccagttactacaagctcttgctagaaattccaagaaagtttacaaggtacctttataaggtggcattgagtaagtcagaagcattccaagtaccaattatcatgcaaataagggctttacttttagattttgttgtttgtggtggtggtgatgctggtgttctctctggaatccagcccaatctccaaaaaagtaaaaggagtacaaatagtaatacaaattattattacttacaccaattaaaatagaagttttgaatgagcaaggagctagaggaggtaaaaactgggaacttcgtatattaaaaggtttttataatttgaaaactaagattatgctggccaaataggctgttttaaaatcagcatagtaatcaaatttgcttgtaatgaatgtagacccaaacagtgatgtcagacctgataaggacttgcaaaccctaaaagagtgcaaaaagaccatagaagaacaatattatattcctgcacttacagaaatggtcagctcaagagatgtatccagttcagggtggctgtaagcttcattttctgaacttgctaccagaagttaaaagaaattctgtataactgcttttgatggaaacacaaattggttgatgtaaatgaaatacataaagcagttggtgtcttattcattcccacaattataaatgaaattaaatgatcaaaaattatagactttggggatcttcttttcactgaggagcccatggaatttgtcttctctagtaccaataactgtgttgacctattttttcctgtctaactctgtatatattaaaactaggtggttacgaacaaaacccagaaatacaatttacattctaataaaatgactttaaaattattccactttttactgtggctttacctgttgtcccacaatgcaggtttctctgggcctctgcttagaatgactctgtcaatgtagatgacagccagagttgaatggggaatccagaaactggggattcgggctcttgatgcaatctatatgccaatctacttcattagttcttcttttatttacagtttggtaaagaatatgggtggagctgttctgggctcacttgcacacatgtccaaactgctttgaaaaaggaagggcaagaaagagtggtatccaagttggaatcaggcaggcatttcagatcaagagacgaactggaaagggaacatctgttagataccctgggtttgaaggcagtctgtgtaagttttcatatctctgagtgtgtgcacacagtggagagggtggagcctgccatcctcaaatctgaaaagattgagagatttcagagggcccagatgtgccaaaggtcagagggatcaatatacaggccctaccacggaaaggcggggaaaaggttcgaatagaaaactgctgcagaagggaagccactgagaggtaagggagtttctgaataattaaaaagttaagaataagcaaaaggaaggaggtcgggtgggggataaaaaaaagcagttgatgtggtaattaagaatttggtgggagcctgggcaggtcacctcctttctcagatcagagccccatcagaaattctttcaagtgtccttctgcgtcgccaaagatgacaacagcaaatcaataagtgcttgaaatgaaaggggatgttgactagcccccaggctacagatttcccgccgccagccttttctgaactcctatagcgtgcctttgcaccgcctctcttaagaagagctaccttttattcctattctcaggacgaaggtaagtgctcagttagcatatctattaaatgtcagctttggttccagctctccgtttgcgcggaaagctcactgccatagcgcgcccagcctgccggaggggcagacagaaaaagcaagcttggcctggcgacttgcggggccacgcacctccagggctggcccggagtcttccagagtttaacgctcctgggttagaactgtaaggtcccggtccgagcaaagggcctgagccaccgtagccgtgggagcgttccttccacttgaatgcactcactcacaaacaagcacaaaatctttttaacagcagaggagaaagacccctgctccaaaattaaagctgggaatcaccggaaactccgttttgagtgcgagatattggtctgttacctttctaatcttcatatccctcctgtaatatgtcttgatttaacaatctttccagcgcccagcattgcccggacgttttaattgggtaattcattagtgagtcaatacaggcatttatatattcttttagctcaagtggttaagtactaatttcgaaatgattataaaacaccggaatcggcaacgcatagtaattttaatttatatgcaaatcaattggttcatcttaaatgccttttttaaaaaaacaattattgtattgtagcatcggaggcatggatcaaacctctagaatagacaattcggaaacaagacctggactaggaagacaatttagaacagccaacaaatcaataatgtttgaggcagttaaacatcgctagccattggtatttacatactcgcttgttgtcagataaggagctggggaaattgcttgccagggttgagatcataatccagagtgaagaaagtaaatggtagcacacagcccgtcacagcgggctctgaaataatactgtacctttcccaaatcctgactcttgggtgacagggagttggcggaggtcaccccacatttgtccacggttttgccccaatttgatcacgaaattgttgttctccctgagctttccaatttgattaccattctaacggttctgtcacttgtctcaacatattggggggaggagtgtaattgagattctcattaaaaattatctgaacccacttagccagcactgtttcatctaagcttagttttatgggctgtatttaattccctgtgccccccacacattaaaatcagatcatcaaaatgtcggtaggaaagggtgaaggaaatggtccaatgctccagtttactggaagactattatctttagacatagttcaaaattttgaggaaataaaaaggatatacgctttggggggaaaatgttttaatattctagaatgggggtattactccccccattccagagaatccgcactggagttgtttatgtaaaaatgtaacatccttgaaattcacagatacgtaaggttagtgtctccccttccccaggctcccagtccaggcgatctagccctaaaggagctagtacctttgatgctacaatcttgtttacatctgcagggcagagaattgcttgctttgcttggacgctccctccacccccttctaatttgaagtaatcggaatctaaatacagtcgccaaggcccgctcttcctttactgctttgacaagggaaaaacctgaaatccacgtcttaaatcagctcggtggtttgtagccccccagcaccctgcttctacgattgcatgcctaatgtattccctggtgattctgggcattaattagttgtttaataggagtatgactaaaaatgtaaaagaaggattaggagcgtgaaacgtatgtccagctccttccacacactcgaggagggaatgagaatcattctgtatcttctatttctccaggagccatttgcatttcccaccagctgctcacttcagctgcactggcgctgggcaaggcgaggacccaaaagctcagcgcagtgtctgcggcggccgggactggggttaaccagcctctggcgggcgagactccagacagaaggggggcgagaggaacgtgagcttcccgagccccttcctctcagccctggtttgcaaacctctgaaacctgaaaggggagggagttgcacgcgcgtatctttgcgtcttttcagcgcaactcccttccctctccctgtgtctctccgcggatctctgaatctttctgtctttggttttctcattctcttccaacttttccatgagattgcctatcctcgccaccagctgaaggcaaggccgttctgctacgagcgcctcttaatctctacaaaatgaaaagaaaaaaagggaggattattagcccattactcagaggaatggggaggctgcaaaaatcgtcgatgggcagaggtgaagatgtctttctcggactgcactttccggtgtcctgtaactagagttcagttgtgggacttgttgaagaaatttgattttcttgcctcggcgagatttcaaaaaccagaaatagaaattctcagagtcagagaggaaatacaattaaacagcacgtgggcattttccccctcatttctctccccttaaataacactgctttgagtttccactgggtaaagagagaaagtttgagttttcacggatgttacgtggaggttagaaatggcttaaaatgtagatctctaatcagttttcttcgtggctgaagaggctaaccctttccataaaatgagtccatctgtcgactgttagctatttcaaagtgaagggatttagcactcaaaacaaattgagcaagtttgtttgcctgtttttactgctaactcaaatgaattcaaaacacggagtaattcaagaaaacacataacatgttccagacagcccccaaaagtagggaaagcccagcacctatatagtgactagggttagttttaagcgccaagcttttttaaacgtatctattttatgcacattctcccgagtcactatatatttctaaaattgcgagtattggtatattgatttaggaagagcaatacaacttttagagggaactttattctcaattagggaccaaagagatgtctttttaatagcgggcctgagttttgctctcaagcaggaattaatattggtgggaaaatccgaatccaggagcaatggctgtgttccggcactttccaaaaacatacattaacaggatgcccttgagattgaaaaaacattgtcccatatgcctggcagaagccttcacacctggtcctccaggcgaattatatttatagtccttccactcagaggcaggacagagccaaaatattctgctcactaccaaaatacacatctttgctcaagtcaagaaatcagaaaatcagggttcagaagtaaggcacacttttcgagtgagaatatgccctgtaatttcacatactctttgctttgcaggagcaaatgtggacttgagggaaactctctcccccacccccacttctatcccgtgcaatttaataccatcctcgccaggaaccttaacctcgtcattttaaaaaatgagatatccgtgacccagggtgaacttgttgaatgtaggtacagcagaggaaattctagactctatgagcgtctgagccttgtccagtgcaaacccttcgtgaacactgggtcagtgcgtggccgtgcccacctgtgcgccgacactctcagcatgcctggtccacccgccttgacctcgggcgcggtgtcccagctaagctgggcccagcgtcccggccttccccagctgacaagcctagctcgttcgctcccggctgtggccctcccaccctctcccactagctcactccattcttctagatttctcttcactcatcctctcccatccccaccgcgcccacctccactcccgccctctaccggtctctcactttcctccctccgcagtccctctttgctgtgacctctttcctcaactctgcaggcctgaaagaaggtcacacacgcacgctcacacccacactccacacgcctcgtcccaaacaaccccatgaacattgtcctttgttccgtctcttgggccactttccctgtcgcttcctcccagcccgtcctgatttgctccccaaaagtacgtttctgtctccccgctgccctggcgctccccctttgatttattagggctgccgggttggcgcagattgctttttcttctcttccatcccatcctcccttctggtcctcctttccacagtgggagtccgtgctcctgctcctcggttggctcctaagtgccccgccaggtcccctctcctttcgctctcccggctccggctcccgactcttcggcccgctggcatctgcttccctcccctgcctcgtttctcgtcgcccctgctcgctccccccggcgctcgcccgggcgctgtgctcgctcctggatcgccagccgcgcagccgggctcggccggccgcccgcgcgccactgtgcagtggagtttggtggaatctctgctgacgtcacgtcactccccacacggagtaggagcagagggaagagagagggatgagagggagggagaggagagagagtgcgagaccgagcgagaaagctggagaggagcagaaagaaactgccagtggcggctagatttcggaggccccagtgcacccgtggactccttcggaacttggcaccctcaggagccctgcagtcctctcaggcccggctttcgggcgcttgccgtgcagccggaggctcggctcgctggaaatcgccccgggaagcagtgggacgcggagacagcagctctctcccggtagccggtaagtggaggccatctatcccgcagggatgtgagataatgcgagtctggaaatttgttccacttcggagaatcttcaccgtaggtgatttgtggcttttggggctaagtttcgcccaaggtaacgcagtcggcaaacagaccttgcaaagccctgttcctttcgtcccccgccacagacactaacaatctacagggtgctgaagtcgagagggaagccagaccgtggctggcatttaaaacgaggtatcttcccttaaatctcggtgccaacactgcaggaacaaatcctcgggccaaggattagcattctcaagataaagggctgggtacaaagtttcagctactggaagattagcccccttcccattgttatccattgggaaaaaaaagaaaagaaaaagattccatcttaactggcagttagtgacctctcaggcccaagcgaattacctgggagccaggcctggatgccaagctctcaccatttctttggattgtaactcctttaaattgatcaccagtcaactccaatctggcacttcaggagatacactttaaatggatgcagagaattattttccagctggagattaagaaaaaaattttcgattctaaacctccgaaatatgttcctcttttccagtttaaccactttactttcttaagcaatttagaaatcaaactatcataaggtggtgtgatttttttttactcttttgtgtgagtattgtcttactaaactaaacggaaaaaacttttaccattataaatgtaaatatcagaattcatacattctaaaatatttttatgaaaaattaatctgatttaaagaaatttccttgcatttgttttagtctatcaatcaaaactaaagatgcttttatcacacaaaatatcattttggcagaaatccatctaaaattcaaataccaataatatcaagaaaacaaagcacataagcaaaataaattgaagatttttgttgatgtaacatgagcatacaacatttcaataaccaaactttccctaaaaaattaaatagccacttcatttgtggaatgttttactttaactcagcaaaattacacttaaattatttaggtgctttgttccttaagttaagcgtgtttgtcttcaaatgttcctaaagcacttatattaattggttgtaaagaacgcatacacatggtaaaatacagaactgaactgagcagtattttaatttccttaaataattacttactacaaattaatttactggctaatttcacaatttagttcatttaaaacacatgttcctgtgctgtttatttttaaactttccattaaagattttgttatggggtaacaaagtgtatgaaaaggggggaaatgtgaaaggatctgggattattcgaactgtatttttcctgcactttcagtcttgcggtagtcatcagaaattattttttagcaaattgttttatttcttagggcttgcctgcctgctttgccatggttcctcgtcctccgttagccgtgtagtgctttttgtgtgctcacaatataaaacccaagttggccaaaacaagagtccttggcatatacattccaactagaacatgaactttgggggtgagaactacctcccatcaggaaaagtctcccatctcaatttgtgagattagccattgaagccagttccgaagtctggcagccaaatttctcacagaagacttgtcttgatagggcaagtttaaggatcagcaggcgggaattggaggtctctttttaaaaaattatcttccccagttatttagactcagttcttctagtaggcctggtcattaaatgaagcataaaaatgcaagtctcaaggctcattttgactgcaaaataaatctccaagtcacaaggacatgtaggagtgagctaaggaacacgccttgaccttcttttcagtccttagagtggagctctatgagttcttgaagatttgttttgtattgctttgtttggtcttcagcactgaagcacggggaagtggggggaagaatgtgtaataattgactgactttacaccaagcaacgcaatctttttcttttgtatatttcattctttaaaaaaaataaataaataaaaactatttgcagttaccatctgcagtgctccggctaccagctaataatgcagccagttcagacatataaaaaaaaaagattatcgaaatgatgatgacatgcaaatttcctccgaaattatcataagtaaacatttgaagtctggactaataaaatcccatctgtgttacttcatatcgagttagtagaaagctgtgataatgaattttgtaatatctcacgaacagacatctcaatcagggactaatcctgtgattttactgcagaatcactaaatctggagccgccaaactgctacttctgggcccacgggcccacaaggatcgaatcggcagagtccccgcccgcgttctcgctagcgggtgggggaaccgcctggccgtccccaccctggatccccacgccacagcgccgggcagcccctcctgtaggcagcgaccttggccagaggctccccagggcccagctcccttcaggagaggccgagacgcagggaaacggtactcaggccagaggcaggcccgcagctccctgccccgcctctgtgcctccgccaacccgacaacgcttgctcccaccccgatccccgcacccgcgcgaagtgggccctccggtcgtcggcgtaccctggttagcgtggagagaggcaggcgctgagatcgaaggggcctagggagccctggaccttcttttcttgtctttaaagcaaccgcggctcttctacccacccggtggagcccctcgagacccacctctcccggcttgcctgtggcagagaagggggagcgcgttaaatgcttggctcgctgcgttgtggttgaaaacgtgaaaaagatttggctcgcccgggagagaaagggggagaactgggtagcagttataccagagctatttctccgtccttggcgggcagtaaaccctccaagaacgtttgccctgctctcctcagtctcgctcagtccacccagtgtctctcctctgcgatcttaaatcatactttagggtaattatttgtagtaagtaaataaatggccgggttagtatctctaggagaaagtgtggctaaatatggaaaagtggctcctgatggatgagaggcccgaactcagctcgctcctgaaacaccctaggccaagagcccgttcgtttcagaattacagaaaaccgagggaaactgctgtctaggacaggggcacgttggcgctgatgttctacaaatgtttaccgagctccaactaatggacaagcactgaagggtggtctttgcatacagcttcccaaagagaaaagtcctctccacccacccactcccgctgccattgcgttcagatgagttcttaaccccggcaccgagattcttgaaagtaggtccacagcctccccagcacactgtggctttatagtcctctaacctctgggcacttttgcggcaactctggagggagatcccctcttgataaataaatgtcctgggcccgaggctaggctggagatgctgctgcacagccagaggctgtcaggtcggaaaaacacgcctgaagcctagcacacagtaggcgcctaacagctagtgtaacgtagtctcatctgagccctgctcactcgacggccgccgcttcttacagccttccttctcttctgttttgcagataacggggaatggagaccaactgccgcaaactggtgtcggcgtgtgtgcaattaggtaagaacccccttctcctgcccgggtcatcggacgggaggccgcgccacgtgagggcggcaagagggcactggccctgcggcgaggccccagcgaggggcgcttccccgaggggccagcctgggcaggaaggaaatcagaaccaaatcgccagtggcctctccctgtggcggggcggtggactaggaagcagcggcgcgctgtgtaccgaagccccccagcctactcctcccggctggaaccgccggcaaccggggaggcgcagaaagagtacgccatcctgccccgggttgccagagggtccgggggacggggatgccgtcagctctttcctctaactgggtctttgctctttgtccctctttctcctccggcctgcctcgcccctccccctcctcccgtccccggctcctttcggccgcggtccgggacgcctctctccgcacgtggggcgggcgcgcgcgtggcccaggcgtgcagccggcggccgttgaatgtctcttctccaaagactccgaaatcaaaaaggtcgagttcacggactctcctgagagccgaaaagaggcagccagcagcaagttcttcccgcggcagcatcctggcgccaatggtaaggccgggagggaagcgcaggccgcgcgctgggcacccgcctccgggactctgggcctcgggcgaagcgcaagaaggcgaggccgccagacctgacgcgcctgctgcttgaacttagacactccgcctctgggtgggacgggaagcagccgtcccagggacgttaattcctttccccaaattatactgcactcctgagacccaacacctctctctccctctcgctcgctccctgtggtctgatcccctgcgcacgctccagcaaacctcggcgtctaggctggcgtggaaaagtggtccaacagcgacctctgtcgctcgttatatcccgctgcgcgcagcaccaccagggcccactcagtcactcaggctctcagccacgccccacccagacttgtgggtgcgcggttcatcgcgggaggcaagcaagggaaacttgagttggcgaaggtttgctttggctggttgggggaggggcggggggccgacaacatccctgaagagctggagggcagccactgtgcttagcagcccagggtagaatggaggtttgcccctgtcgacgcgaacctgcctgaagtactggttgccaggccttgggttttggcgatgtcgttgcttgattggctggtttcactctggaggaatcgagggacattgccagaggaggtctacaggcttatgtaaaaagttaaaaagtctccaacctacgccacaggcctttcctgaattgaaacttgttctatggggcggaggggggggtgtaagggatggaggagggaagatgcctttcttttcaaatacatggaaaaaaacccctcaaatttactgttcctctattttcctggctccgtagtaaataagtgcctagccttaggaggctattgacctttgataatgtgagcagataaagcccccccccccccacagccctcggcccctaaccccctctttccggattaaagtgtaagaatacaaatgtaatatgggatggaggggggcgatttgggaccccggtcaaaaaaacaaaccgtattactaagaagaaaacaaaggtcttgcattggagtttccccgtgaatctgagagaaaatgatcatttgttgaaatgaagcgtctaaagcgatccagtgcttcacgcccggacactgcactacaccgccagtcgccctgctgggccagttaaacgctcacttgtccgggattaaccccatggggttaaatgggggcaatgcagagataacgtcgcgtgatttctgtcatttagattgtgttaaattcttcttctgtttgataatcggtagtaaaaataaattattagaccgtagtatgtttgggatatggttaaaaatcaagagcagcgatgacttctggggagaatgctttgcgcgggctcagccctggctccggccagactagaggagctccccaatctcgcttcgcgcggggcgggctcgcagtcgccaagccgaggctgacatttcttattgtgctgggagccagagagacgcaaaatgtctccttcccccagtccctaccccaggtttcctagacatggggaatgcattctgaggacaggtggagaagcctacggtaggatggggtcctcgtaggtgagcaggaaacggctaagagcagaggagttctgcttgcgccagtcacaagccgcgcaggcgcccctggtcgttcgcttttgataactagcacataaagaactagaaataatgaatgattgctttcttaaccattactttcaggcccgcattgttttagtgcacgtgaaaggctcttcccctacactcaatatgtctttttctactttttgaccgaaaagaaaaattgctgcctaaacacgtttaatgccattaattaagaaaaggcatgtaatgggaagaaatgctgaaaatcttgatttaattggcttttaaggaactagtagacgacaaaaaaaaatcacacgagtgggcaaagctatagcactgctgaaggatagagcacctatccttccctgattttaagttaacttatggaatatccaaagtcctggccacagcctgcttgtaaaacaaaaggatttatttcttgtgtttttttaaagtttttctttgcttttaaagagaaaaaaagttcacaatgacatatgacttcttcaaaaggccgtgatagtctattacgctaccctctccgcctctgcccccaacgccgcccaaaaataccatgtcctcgttaaagactaaacgttctgtataggcagagtccacctctaagcagtccaggctctgccttccttccctagtgagtcccattctccttggtatccattgggcggatgcccagcctggatagaaccccgaaacgggggtagcacgagagcgactggagacccctaaaagccagaggtttgagagagggtggacgcagctagcagaagatggtgtagaagccagctgagaacgaccccctagagcaaagagacctttctttggcttttcttgctttgggggtcctgaaaggaactcataaaatggtcttcaccctcaggaggaggacggactgaccctcctctgtcactggcttaaaaagtttcagggcggcggctctgggttccgtgctgaaatcggactgcactgcagcccctttggacctgacgcctggctttgcgtcccgacaaggggcgggtacttcccccggcctcccccaggaacgcattaattgttaaatagctttggcccagtggatgggctgaaagtgttcgacccaagtcgctggtgtgcacagacttcctccctctgggaggtgggctccatggcccgttgtggcacccccagccgcgacacacaccttcacacgcggcagcagctcggtcccaaccttcttcgaaggacctgggttaaccctggcggccttggcggccgcagacccctctccgccgccccgcccccgcgcctctcattcaatcagcgaatgtttgcggagcatatactacgtggactcctaatgtaccccctgaaagcaaataatacagttttcctcgccgtcatgaagggattttaatcctaacatggacaccagcgagatcagcccagaccgtctctagcaaaacgcaaaatggtggtgcgtggggtggtgaccaaggtcctgagccttgtcagaaagaaggggatgtgtagagaaaggtggagaactctagctgtggctagcgcggaagggacaggtgcttgccgaagggggcatgaggcttgaggaaaaagcaacgaaataggggtaaggagagttttccattttctttcctccgcccgacctccgccatcccattctcccctcccctcccccaccccccgcgccaatcaaatctgcagctcacttgaaaggtgccccgccgcgttgtggtttttcacccccaggggaaattgtaccagttgtccgaaagtagtcagtccctgcggatccctgcccgcaaaagtggtcttcacaggtcgcgttcctcgctgctgactcggtacacaaagtttcttaaggctggttcggctgttattcctcaccgcccgctgctaatatatgcagcagttgttagagcggctcgggggaaaaggaaatgtataacgaaagcttattcgtgagcaggaatatactaatggaacaatctgatgtcttcttaatcctatgtaaaaagctttgtcgtcttcctaatattgactgaatgggtaattaatggctcttcatctaggcgaataccctgtaatccaagataggcaaaagacaacaagcccaaggtagaagacaaaaggcccaactgcagcggcgtttgcccgcctcctaccccccagggtctctgactaggaaagttttctctcagaggagaaaaaggcaggagtgggagaatatatacctatcatttcggggctagacttcaccgcagcacctgaccacccagctcagttttctgttactctgtctttccacctccagtccttctccctgcatttttttttcttcttaactcctctaggatgacctcctaccaccaccgccattatggtcctaataacctttccccctaaaccccacatctttcacttcagcaaccaatgaggctgttttctgatccaggaggagattcttttcttttagaacccaatgcgtagagtctttgagaactaaagtagttggtaggggaggaagaaattaatagaaagggagagagcatacagaattgtgtgtgtatgttaaagagcgaccaggaatgacagagtcaacttctttgtgaggatctgacgggaagagtgtccaagactctaccagcatgtttttaacaggctgacattttaatttaaacctttagaagtaatatattacttgggttactacaatgaggtgggttcctttttttttgtcagctgacagcttttaaaatattatttcgctagggaaataaaagcttcatctcagattataggtgggtatttttggatttaggtgatttatggtcaccatgacaactaatgctgaatgttagctaccagcatgtctgggagagagaaaacagaaagaagggagagcaaaagaaatagaaaagggagatggacataagctggagagggaagaaaagagaaaaagaggaagacagatgagtgtttaatccaactgttgtttaaaaaagtggcgggggggtgggacttcatttagccccttgccacttccttctttcctgacctggatatctatgctcaatttcatattccacccttccttccccttctccaaacacatgtgctataccattctccttattttacttagttcggcaagtagttgctttctggagactcagtgacacctaggaaaactgtggcagtaacatgcaaatgtgaggaagcattaacagcatgttcgttgagtgattttagcaaatgccccctcctctaatctctttctcttctcttccccaggccactgtgaggtggtaactcccactgccatctgaacactgttcccccaggtagttaccccaaatctcaaatggttgagcagctagagctgtgggttggaaaaatgggtaccatttgcagggacccagagagggtggctgttgctcaatatatctacagacttccaattcagaaaataatcttccccttttgacaagccagagctttttaaattccatttaggaaatggggaaaaggacagctacagtgaagcttttaatttctgggttatttggttccatagctatgaggggtggtgggtagtggactgttttcagcttggtttgtatgcagagaaaagccagatattggagggggtggggcacttctcgggcaggatgcaaggtctccatctgacctctgcgccttaccaggagctcacacactcacgcccatcacgtggctccaagctgagtccaggcgggcctcgtccttgagctagcttgggcagggcaggactcccacccgtctaaggcctaacagctcagggagatgtctaattaagccatcttctgggtgaactctgaagacagactctttccaaaagtcagagatcacttggttgagtcccaggccagattgatacggagagtttggcggcacagcccaaccgctcactgccatggccagagggactttgcacaactaacactgaagagtgtgaaattaaataagactttaagactggtaatcggtggcaaataccagcacaaaacacggctgaccccatgtcacacatttccctcctctagggtctttctttgaaagaataagcaagaaaccccaatcgagacaacccctgatgtctcccagactcaaaacctcacgccggcactgggctttccttctttgccccacgtgagccatgcagcacctctagtttccctaccaggatcccaccaatgttctccgtattggaaatttctgtgttagaggctgaactcatagtaatttctaaaaccaattaagaagaacttagccagaggtcacagtaatgctggaatcacaaaatgcataagatttattttcttctggcccctttctcatccatgctgcctatgcctgtgcacccacaagtcttatgtacattaaatctccaaaatcaaccaccaccatgccacagagttttcactggacagtgtttcttagttcccaccacatacctccttttccccatgcagacttatcatgttggtgtcctgccacacagggggcctgagaagaatgtcacccaatcgccgctgctgtgagtgtgtaaagtgattaggagattaggagaatgttgaaactcctgctggaaaaatgcaaagaaaatcctcactttgagtcagttgtttacagagccagtgtgtgtgtgcgtgtgtgtgtctgtaatataaaatggatgtgaatatatatatacaaatagatatggttttgcttttactttaatctgaattatctagataattgtctttattcaccacttgacttcaatgggtccacacaaattaggacaccttatctttttaggcatctaggctgctgctgatccccagtgcttccaacatctcgcacacgttggcactatgaggagcagtcacgtgcccttgggtttttcaaccactttggaggctgattgaggtccttcatacatgtatatttgtcgtgatgaaagttccatcggtagagtggagccaccagagcttttatcaaaattctgtgggtttatgagagatgggtttagaaatctatatggctctgtggggcttctcggctttctaaaataaggcattaacacccaagcttccaaaaatatttgcagctctggggtttgaatcttgaaaaacaaggagtgaggggctgtgtatactaactacagtggagatttttttcattctttaatgtgatggagtcccttcatgaaatgaagctttaaggggcatggtattgtggggaccacagctattctgaggtttaaaagaagaaactggaatatgattagtaaacacattcagcagaaaagagctggattcttattgacttagttataggtcatcggctggcagtgcaatgggaggaaatatttactttacacatatactttatgatcttgggggaattagaggaaattcaataagaaaacggctagaaacatttaaaacccttatttaaaagacttaagcaaattagagtcttatcagattaaaaaccactacaaatgtaagagcattgtcttcagtgaaacgctgtggggtctgagaaggagattctccgccaaatctccgggataaaatgcgtcatttaagcaccagataatgagcagaatgtaaattaatttaaccttctttaccaacaggctgctagtgtaatgtgtataatttagtgataagattgcaggacctaatatagctggatgtatgagcctcagctaatgcagacctgtcacatgaggatgtgttttactctgagcaggtgtctgtatgtgtggaatggggtaaagtggaataaaaggttaaaagcagaaatgctgatttaaagcttactatgaagaaattcctcccttgcagctaaattattcttaaagtgggatgatactggtgaagaaagactgaaaaacaattctcatgtgcgtctttggactgcaagtttaaaatggggaggagttgcagatagggtttgggggtggtcagggcaaaggagagacacataagttgcaaatatatttgtagtctgcttcatccactttgttccacatcgaataagtttcccaatcttgtgaacaaggacaaggagggagtgttttaaagatacttcatgctggcattgcaaatcattgactgtaatgtcaaacaaatacacattcagagatgataacactaactccatagtaaaacaatcgcccatgcagaaacccagaggagattagtttgtcctctccagctgacctatgctgggggacaaaaggactttcaaaaattattttgaatatgtttggatttctttctttaatttctttggaaattaaatttgcttggaaacagtgctataaagagttgatgtctccaaaggtgattttttttgttttatataaataaggttttgcttttgctagttgagcgcagttctaggcttttcgcccttagctcacacacaccccttctgcctgcttggactttaatggctcaagacagccttgagctcactgggaaaagaaaatgactgttaaaaattatccttgaaattggttatttggcaacattcttaattgtatggaaattcattaaggcatatttcatatataattagctcaaggttgttgattctacaggctttatggatttaaatctgattgataataaagtaaacaagagagtcgaatttaaagcgtggctctctcgggttaggacgagcttaatacagtgtacaaggaatttgaaagatctaggatatgtgtcttaatcaacgttaagtagaatggataagctttcagcattttgaaaacgctgggttagggtttctcttctattgtgtgttttctgtctggggactaataagcatcacagagaacgtgatctgaggcgactttttattcttgtataaatccagagtgaaccaccaaacagttgttcgtttaaagtcaaggtaattttcttttgacgggtccatttgcttctcgatttctaatttattagcctgccttttcagggctctgtcttctttgcaattaaagcttcttcagattagcgcagcattcacttgacaggctgtttggaaaatttaagatcggagaggtgatttgttgctgtttttcaaattttctagttttaagtaacgtgtctcctttttatatggggtgggggattggaaatggatgtagtgagacacaaagagtgggtgtcttgttgatccttgtacctttctcttcttgaccattccactctcttctcccaagccttcgactcctagcctcatctcttcacctttgggttcgtactaaaagccggatcgccttgggctgggcaggagctgaattcccgggagcttgcctgtgtagacccagtgcgcacggcgaggcagtagcccggccccgcactgctgataggtgcaggcaggacagtccctccaccgcggctcggggcgtcctgattggtgcggagccacgtcagtcgcacccggagaagggtctgggaggaggcggaggcggagagggctggggagggccgcggcggagtgacgtctcggcaccaggaagcccgcctctggttttaagatgttaggccaacagggaagcgcggagccgcagatctggtccgtcgctcgcctgggtgcctggagctgagctgcggcaaggcccggctcctgttcgaccgcccgaggggtgtgcgtgtgcgcgttgcggagggtgcgctcagagggccgcgtcgtggctgcagcggctgctgccgccgcaggggatctaatatcacctacctgtccctgtcactcttgacacttctctgtcagggctgccgcgtggggggggggcgggcagagcgcggtcggcgttagctttccttattggaggggttcttgggggagggagggagagaagaagggggtctttgcccactcttgtttcgctttggagcttggaagcctgctccctaaagacgctctgagtggtgcccttctgcccacatcccatgtcttcgtttgcccgctgactttccgtctccggactttttcgcttgagccttccggaggagacgggggcagcttggcttgagaactcggcgggggttgcgtcccctggctctccccgcagcggggaaactccgcgcctagagcgcgacccggagcgggcagcggcggctacgggggctcggcggggcagtagccaaggactagtagagcgtcgcgctccctcgtccatgaactgcatgaaaggcccgcttcacttggagcaccgagcagcggggaccaagctgtcggccgtctcctcatcttcctgtcaccatccccagccgttagccatggcttcggttctggctcccggtcagccccggtcgctggactcctccaagcacaggctggaggtgcacaccatctccgacacctccagcccggaggccgcaggtaaggcgccgcgccgccctgcagacattcccgctcagctgctctgcgccacccgctccctctcgccccaaggaagtcagcccctccggggggaggcgtggtgggagtggtcgttcgcctggctccccgcagaacttccgggagccggaattttgactaccccgcatccctttagttctccctcgaccggcccggctcctggggcgctaagggcgcgagcaattctgccgccctctctattcgtaccctggcctcccttctgtttcctgggtcacaaaaatcccagcatcttgattcgaggaccttcagaggccgccgacctctgtccctgttttcctctcggctttcagctcccgaggagctccactcgttaggaaattgcctgaaaccactcagaaatgcccttcgcgaagaggcattttttttttttttttgggaaagggccggcgaacttcggtgcccaaccgaatccccacatcttttcctagccttcccaaaccgcatggaaatctgagctttctgcgagggggaggggggtctgtaaaccacgcgcgtgtgcgcgtcccaggagatttggtgtgtctgcgcagaggtgtataaatatacttgaaagcacaggctataaaagtgaatgtgccgctgcagtgagataaacatgtaaataaaacgtgcggcgctgggggaggggaggaaatggggcgcggacacccacacttgcgcctgcacaccccacaggcgcagcgctcctcgcggcccggagccgccgcgcgcaccctcctccggcgccaggcagcccagctcttccacggcttctgccgccggtccagttggcgtccgcgttgcaggtgggcatgctgacgggaaagtgtgtgtgtttcgttttcagagaaagataaaagccagcaggggaagaatgaggacgtgggcgccgaggacccgtctaagaagaagcggcaaaggcggcagcggactcactttaccagccagcagctccaggagctggaggccactttccagaggaaccgctacccggacatgtccacacgcgaagaaatcgctgtgtggaccaaccttacggaagcccgagtccgggtaggagccagcacggagtctgggagggatggggggaggatgttgtggaggtacaggccaagtagaccaggagagaatgtggaaggcagcgccgcctgggagggcgccggtggggcgcagctttgcaaaggcagaaggcctcgcggcggcctggttgcgagattacagttccctctccgaggccgacaggactgccgccctggctcaggctcccagagcggcaccggctcactgccccgccatcccgcgatctcacgagctgggctgcatgggcaatcccctgcacaggacattgtgttcctggcttgcagttgccagagcagagctaataaaatccctaccaggccaagagccgcgaacaggctccaacctgtgagcctttaacaaggaaaacccgccagagacacggaagagttggccctccctgggaaacctttgtcccggccctggcccagctttttccctcctgggctcgcgcttcttacaccttctttacggttgtttcggccattcaggtctctcccacacaccctatttcctagttttgtgatctccgggagcaaagttttaatacacaactactagtcctcttagaaggagaaagaaaaaaagaagaaagacttttctgcttggtttatttatcttctctcaggagttgaactctggaaattgaaactcacaccccctcttctaaattataatcatagttttgtaaaaagggcttaccttaactttgtagcaaatctgtactttatggattggcaaaaatgagctcaaataaataacccaatagcaacgtcctggtttatgctggtcggtggaagattccaaatttgttaggattctggaagcagaaaacagaatcaagcaaatcaagcggcatccagaggctttgctgttaaaaaaaaaaaattaagtgctctgggtagaaaaaataaagcccccggttagagcagagcaaacaaaaagaagaaaacaacgataaaaagaataaagaccaaaatgctctcccaaatcagagggaatgaagacactctctgggtggcatttgtgcaaggcatgaggctatgctggtggataaaaggccgggaagaagttgaaaatggttttagtttaactgtccagagccagagctgggtcctgggcggcgtggttttgagcaaggtcagtctttcattagctctcttgcacatcaagggaacgggcctctcacgtactcttctcgcctgagcaaagtttagatggcctagggtagaaatggcaagtaattaaagacagagtctatgggttttctgggatccttcgaaaacgccctcccaccccgcccgctattccgcagctccaccctagtgctttgtagccgcggcgctgggctctccttgcagctgcctctccttccagggcggctgcttgtcgagccaagtgggagtgaggcgtgctttttatagcagtcgggtgcaaagaggaagggggataaaaaggaaatcaagaatgaaaggaaaaagagaaaaagcggattacacggctgggcccggcggagatgtgtaatgtgaaacatcactggtgtcagctcggatatctcaggccaggcctctctccaatacacaaaagccgccgtctggggcgacagggaggcccgatgtggattgggatcggggttgcggctgggccaccggacacgggtggaagccggccggcctgggtggccgcctgcaaagccaaacgacccggctgggcctggcgcgcggacaggcctgtggtgggcttagggtaaagaagaggcagagcgaaagaagggggaatctccaaaactaccctttccgggttcccggagtttaatatgccaagctcctggagttaacgagctgacgaagaggtggtcttttgctctttatttggttgttttgctaggcgagaaagagtgttggcggcctagtccctgttaagggagcacgtaccagggggtgggggacgacagtggaggtcagggaaggaagggaggaattgcgtgggagaaagagcgatcctctagtgcccttccagccccttctcctcatccgtgggtctgtggctttggaatggaagcaagtttgcaaggtgccccgggaagggttggaaaagcctgctgccccgcgtttgttttacattaagtgtttttggacctggagaaacgcctggctgagtgatcaaaccgtccgcaggtctccatgcgttcggctgaggtttgtggcgtagctccgagtcccagctcgcaggccagagcagaccaggtctcctgcgcttggtggagacccgggccagtaactgaaagctggccctggtatcttggtgtgcagggcggtgcagtgaagcgaggccagggtgtgtgagtgcgctagcgtgtgtgtcgggggaaggcgggggttggcctccgatggaagttttagtaatctgcactgtggcatctgtttgctcccttgccccaaccgcccccaggtttggttcaagaatcgtcgggccaaatggagaaagagggagcgcaaccagcaggccgagctatgcaagaatggcttcgggccgcagttcaatgggctcatgcagccctacgacgacatgtacccaggctattcctacaacaactgggccgccaagggccttacatccgcctccctatccaccaagagcttccccttcttcaactctatgaacgtcaaccccctgtcatcacagagcatgttttccccacccaactctatctcgtccatgagcatgtcgtccagcatggtgccctcagcagtgacaggcgtcccgggctccagtctcaacagcctgaataacttgaacaacctgagtagcccgtcgctgaattccgcggtgccgacgcctgcctgtccttacgcgccgccgactcctccgtatgtttatagggacacgtgtaactcgagcctggccagcctgagactgaaagcaaagcagcactccagcttcggctacgccagcgtgcagaacccggcctccaacctgagtgcttgccagtatgcagtggaccggcccgtgtgagccgcacccacagcgccgggatcctaggaccttgccggatggggcaactccgcccttgaaagactgggaattatgctagaaggtcgtgggcactaaagaaagggagagaaagagaagctatatagagaaaaggaaaccactgaatcaaagagagagctcctttgatttcaaagggatgtcctcagtgtctgacatctttcactacaagtatttctaacagttgcaaggacacatacacaaacaaatgtttgactggatatgacattttaacattactataagcttgttattttttaagtttagcattgttaacatttaaatgactgaaaggatgtatatatatcgaaatgtcaaattaattttataaaagcagttgttagtaatatcacaacagtgtttttaaaggttaggctttaaaataaagcatgttatacagaagcgattaggatttttcgcttgcgagcaagggagtgtatatactaaatgccacactgtatgtttctaacatattattattattataaaaaatgtgtgaatatcagttttagaatagtttctctggtggatgcaatgatgtttctgaaactgctatgtacaacctaccctgtgtataacatttcgtacaatattattgttttacttttcagcaaatatgaaacaaatgtgttttatttcatgggagtaaaatatactgcatacaaattggtctggattctttctcccctcctctgtcactaacttggccaggacatctcagtcactgcttcctaaacaaaccagttccctctgcctgcctagttaaacatacaaggcagcagtccttatttaaatttggtagaaataaatgatagccattcatcagaaactaaaaagaaaaaaaaaggcattcccgggggggaaaagggctacaaaatctaattttgtctctccaatttttctttggcttaaacctagaggattccattatggctagcaaataatatgaaaaagaaaaaagaagaaagaaatttagcaagtccatcagcttaaaatgactctcaagtttactcctttacggggaaacctacacctctagcaaattgttctggagaaatatttgtgcatgtatacatgtatagtttatatgcatttctctcaggaggaatacatctataataaatttacagggaaacatctccagttcaaaatatttaggcttccacgtttatcttcaggcttaagtagagagatccttcatgttatattgcattactatttccaaatcctttggagacattaaaagaaacaaagatgatttctaataactacagcccttcagtttctcaaagaactcaggggttgagaggttagagtggagtttcctgagtcttgtcgagcaatatgtagttgaggcaaaggtcatgctcccggtgttttgttttaaataatattgacccattaattctaaacctgcttgttcctgaaattatacaggattatagtttgcaaactgcaggacaatgaagcaaatcaagatgaattacagccctggccctccctgccatcctctgacatctaaacagggaatgagttcggtgtgagtgtttaaatgaactttaagcacccgatccttctttatccgcgattttcagctttaaaaaaatgtgaaatttgatttcataacaaatagaaacaaataccacttagtcccagagaattcatcctcatggcgctaggagggtcgttgtggaggtggggggagggatgtgctgagatcttttgttatgcttgtcaaccccccgcacaaccaaagtgggcgagaacaaacaccacgctggggaacttagagcaaaaagtaaccgccgattttctggagccgacaatatcattgttttttcgccttagt

SEQ ID NO: 2 - DNA, 12001 bp, Homo sapiens
catggactgcgtgatcactaaacttggcacttcagggggcatatcttttttgagtaactctcataaacatgcctgcctgcaggacatccagattttctggtttggtagtaaagcaacataagaataatcttgaacctgatgttcatccttgccttctttctaattccaggagccctctgaggtctggactaactcactgattaggaaatagtatttggaaaggctaaacaaaatactatttccagggaaatagtatttggaaaggctaaacaaaatatactttcttagttttctcaaacctctcagaagatatattttttaaaaaataaactaagctagcaacatttaaactaaatctttgccttgcttacaatacaaaagatgataaaaaaattgttgggaaggtgagaaattaacttcacctataattagaagtaaagttttcatttaaaaatgtaataccacttaaattcaatttgggaaacaaaaaggactcaaaaaacagtctgctaaagccaatttgcaaacaagtgcgctctctttttctttaagttgtatctcaggttcagagcacatgtgcaggtttgttatgtaggtaaacctgtcacagggatttgttgtacagattattttgtcacccaggtactaagcctcgtacccaatagttattttttctgatcctctcccctctcccatccgccaccttccaataggccccagtgtctgttgttcctctctttgtatctatgagttctcctcatttagctcccacttataagtgagaacatgcgttatttggttttctggtcctgatttagtttgctaaggataatggcctccagctccatccatatttctgcaaaaggcatgatctcattctttttttaactattccactctctctattactctttcttcttcccccaatcctgaaccctaccatgtcagtttaaccactccttttctttcctttttctttgctcatttgcacatagttaaaagatgccatgaatttttctttttaattcagcatatgcccattaaagatctaaaaatattatttacatcatccagaactcagcttaagaaattaccaaaaaataaagctaccagaaagtaactgaatcatcttgttgagccacaatcctagacctcgactctgctttttcctcattttaggcaggtcattccttttcctttcttaaattgttttctctgtattcaataacacattcttgtggattcagaaagggtggagtatgaggaaaaggaatatgatatatgtaccctagaggaaaacaataaataaatatttcaggatggaaaacattatttttatttttattgagttttctagagtctatttgatttgtgtaaatcagaaaccagtagaatgacattaatgaattaatgaaaagcagaatgagttatcagttgtaacaaaaagaataaagaatttcaagaacacagctttaatcatgcatggctgcggggagagaaaaataacaaaatgctctcagtgaatacatctctgagagaagaaaggaaatacttaaggagaggataaaaagagcaaatatcaaaaataggagtaagaaccctattgctttttttagttgacaaataaaaattgtatatatttactgtggacaacatgatattttgaggattacgatcacttttgattcataaattacattcaagaaaaagaaattctcaaaaagtttgggaacatatgaagttgaaagaacattaatactcagataaggacagtacatgacaaattattcttgctccaacattttctctcaggaaatttaaacatctttcagtgaagcaccagtttcttgaaatcaagcatgagaaaaaaaactaaattcacctgtggaaaaaaagacacagctaaacaaaaaagcggttgttataacctcaagagtggcatgaacaaaatgatcaacattctcccaagtgacagcacaaatatcaaaagtcctaataagtggaagtggtcctgtcatgacaaaaggtgtggtatttgtacaatttccagataagaacaaagtcatgacgctaagacagtagcagcactgtttgttacacgtgatatttgaaaaatatgacaaccatctcaatctgctcaagtagcactcatggtgagggtgaaattttatcaacattggttaacttatggtgttttaaaaaactagcaaggagataaattgatggattaaaagataaactactcacaggcagacaaacagaaggacagatagagttacaatcaaacatgtactttactcaggcagaaagataataaccagcccccaagaagtgatgtgtctgctagaaaagccctgaacatagaatttcctgactttgtttttaatttagttctttcaggcatcacgctgcataaccaggtgtaactctctaaaagtctctatgacagaattttccatctgttaaattaggctaataatattttcatctttttttagggtaaagatgtgaaatatttggagaactctggaaaacatgccccctactaattagagctttttgatgtgacatcattttcttcagtacttggagtttagtcaatagatatacagtgtagctgtgaaattatgaagcatgagaatgcattaccaagggaccgtaggaggctctttactgaaaagtgtagctggctatatttctggaagtaatttaaacataggctgagggagaggagtaccctctagatcctttccagaccttactttctatgaattctaatttctctttcccatttagaaaaaacaatgagatccacagcgtagagatagaaaataaggctctgtgtgccctcaaaccttactttcaaaaataccacagcattctggacgagatagtcttgaattcttgcaacagcacaggtatgagagtttttaccagaaaacaggagactggattgattctttcattctcctcctatgcttcctaaaactgaaaagccatatatacaaattatatttatctatccctcctggaaaaggccaaaatgaatccaattttggatcattttcaataatgggacaaacctgaattgagaataacctttagaatcagtcctgtctttttgtgataaaatggacttgtagaaagctacctggtgttctcccctagctaacattctaccacaaacaacgggtatgtaatccagtattgctccccacaggctatgtccttggaatcactatctttgcactccatttgtctgctgacatccttccacccaagatgtcttcttcagcacaagaagtcatttctcttaaaatttcaaatgactttactacaataatagagttgctaactagacctaggcaagtaatgataataaaaatctgatttctacttagagtgtagcatggtttaacacaacaaccagagtcctaacaggtttttctagatttcactcctactcaacttgcatgttcttgcaatatagatgttcttattactcggtccttacttccatctctctttgcttctggaataaaactacttaaacccaattcagagattttattctcccttggaattactgggaaacagttctagtaaaccatattcctgagatcctatattaggcttagtccaaactgaccatctaagcattaattttcctgtggctcaggaatatccctgagcttacctttctcttcctaaactgcccaggacaaataccggagtttggcttttctgctttctcatccaatcatttctcgtttcctcctctttagcatttaaaacatttctgactttctccatccctcaagaaatatatttgctttcctgtctctgcattattcttttgtttatgaaatattccataggtaagttctatatttccttcccccagaggcccctggtcttctggttccagttgccattggttcagtgtactagttaacattttggactttggagttacacaaacctagattcaaattcccactatgccacttactgcctacgtgacctgaagcaatatcctatccactgtggcctccagcagttataagcttgtgctctaaccagctgggtgaccttgggccagtgacacaatcatggcaaacctcactgtcttcatttgtaaaatgacagtacctaccttgtagtgttggcataaggaataagtgtgattgtcaatacaaaagtgtttagtacaatagctaaattaactaagcactctgtaaatattagtttttaccattattactaattcaaatgactagatgcattttgtgtataccaggtttcctgagttcactttgttctcaacaaatactattattcctagcatgtggcctatatcacacttcattagccagaggacatgtgaagcttagagtggaaagctagggcagcaggaagcattgccacactttacacagtcaaagccatttaaacatgtctgaatttgagctctgctgagtccttacttgcccccatctctcctgtgtgctccagcttactaataaagcaggtttaatataaatacactaaaagcctaaacattgagatcatgataatgaatatgagggctatgactataaaatatcattgaaccagagacctgctacgaaaccacatggtgaagaccacaagggaggaatctgcatacacaccgagtgccttgggatcccaaagtgggaagagtcagtgccccaattaaagagaaactcggggtagggaatcaaccacaacatcagtcaccttactgaacccaggcttgtttcagctgacgtagctgccaatttccaatgtcccctccctccctaattgctctcaatctattcctccagaaactgaaagcccatcaaagaggatatcttcccagagagttgttccagttactacaagctcttgctagaaattccaagaaagtttacaaggtacctttataaggtggcattgagtaagtcagaagcattccaagtaccaattatcatgcaaataagggctttacttttagattttgttgtttgtggtggtggtgatgctggtgttctctctggaatccagcccaatctccaaaaaagtaaaaggagtacaaatagtaatacaaattattattacttacaccaattaaaatagaagttttgaatgagcaaggagctagaggaggtaaaaactgggaacttcgtatattaaaaggtttttataatttgaaaactaagattatgctggccaaataggctgttttaaaatcagcatagtaatcaaatttgcttgtaatgaatgtagacccaaacagtgatgtcagacctgataaggacttgcaaaccctaaaagagtgcaaaaagaccatagaagaacaatattatattcctgcacttacagaaatggtcagctcaagagatgtatccagttcagggtggctgtaagcttcattttctgaacttgctaccagaagttaaaagaaattctgtataactgcttttgatggaaacacaaattggttgatgtaaatgaaatacataaagcagttggtgtcttattcattcccacaattataaatgaaattaaatgatcaaaaattatagactttggggatcttcttttcactgaggagcccatggaatttgtcttctctagtaccaataactgtgttgacctattttttcctgtctaactctgtatatattaaaactaggtggttacgaacaaaacccagaaatacaatttacattctaataaaatgactttaaaattattccactttttactgtggctttacctgttgtcccacaatgcaggtttctctgggcctctgcttagaatgactctgtcaatgtagatgacagccagagttgaatggggaatccagaaactggggattcgggctcttgatgcaatctatatgccaatctacttcattagttcttcttttatttacagtttggtaaagaatatgggtggagctgttctgggctcacttgcacacatgtccaaactgctttgaaaaaggaagggcaagaaagagtggtatccaagttggaatcaggcaggcatttcagatcaagagacgaactggaaagggaacatctgttagataccctgggtttgaaggcagtctgtgtaagttttcatatctctgagtgtgtgcacacagtggagagggtggagcctgccatcctcaaatctgaaaagattgagagatttcagagggcccagatgtgccaaaggtcagagggatcaatatacaggccctaccacggaaaggcggggaaaaggttcgaatagaaaactgctgcagaagggaagccactgagaggtaagggagtttctgaataattaaaaagttaagaataagcaaaaggaaggaggtcgggtgggggataaaaaaaagcagttgatgtggtaattaagaatttggtgggagcctgggcaggtcacctcctttctcagatcagagccccatcagaaattctttcaagtgtccttctgcgtcgccaaagatgacaacagcaaatcaataagtgcttgaaatgaaaggggatgttgactagcccccaggctacagatttcccgccgccagccttttctgaactcctatagcgtgcctttgcaccgcctctcttaagaagagctaccttttattcctattctcaggacgaaggtaagtgctcagttagcatatctattaaatgtcagctttggttccagctctccgtttgcgcggaaagctcactgccatagcgcgcccagcctgccggaggggcagacagaaaaagcaagcttggcctggcgacttgcggggccacgcacctccagggctggcccggagtcttccagagtttaacgctcctgggttagaactgtaaggtcccggtccgagcaaagggcctgagccaccgtagccgtgggagcgttccttccacttgaatgcactcactcacaaacaagcacaaaatctttttaacagcagaggagaaagacccctgctccaaaattaaagctgggaatcaccggaaactccgttttgagtgcgagatattggtctgttacctttctaatcttcatatccctcctgtaatatgtcttgatttaacaatctttccagcgcccagcattgcccggacgttttaattgggtaattcattagtgagtcaatacaggcatttatatattcttttagctcaagtggttaagtactaatttcgaaatgattataaaacaccggaatcggcaacgcatagtaattttaatttatatgcaaatcaattggttcatcttaaatgccttttttaaaaaaacaattattgtattgtagcatcggaggcatggatcaaacctctagaatagacaattcggaaacaagacctggactaggaagacaatttagaacagccaacaaatcaataatgtttgaggcagttaaacatcgctagccattggtatttacatactcgcttgttgtcagataaggagctggggaaattgcttgccagggttgagatcataatccagagtgaagaaagtaaatggtagcacacagcccgtcacagcgggctctgaaataatactgtacctttcccaaatcctgactcttgggtgacagggagttggcggaggtcaccccacatttgtccacggttttgccccaatttgatcacgaaattgttgttctccctgagctttccaatttgattaccattctaacggttctgtcacttgtctcaacatattggggggaggagtgtaattgagattctcattaaaaattatctgaacccacttagccagcactgtttcatctaagcttagttttatgggctgtatttaattccctgtgccccccacacattaaaatcagatcatcaaaatgtcggtaggaaagggtgaaggaaatggtccaatgctccagtttactggaagactattatctttagacatagttcaaaattttgaggaaataaaaaggatatacgctttggggggaaaatgttttaatattctagaatgggggtattactccccccattccagagaatccgcactggagttgtttatgtaaaaatgtaacatccttgaaattcacagatacgtaaggttagtgtctccccttccccaggctcccagtccaggcgatctagccctaaaggagctagtacctttgatgctacaatcttgtttacatctgcagggcagagaattgcttgctttgcttggacgctccctccacccccttctaatttgaagtaatcggaatctaaatacagtcgccaaggcccgctcttcctttactgctttgacaagggaaaaacctgaaatccacgtcttaaatcagctcggtggtttgtagccccccagcaccctgcttctacgattgcatgcctaatgtattccctggtgattctgggcattaattagttgtttaataggagtatgactaaaaatgtaaaagaaggattaggagcgtgaaacgtatgtccagctccttccacacactcgaggagggaatgagaatcattctgtatcttctatttctccaggagccatttgcatttcccaccagctgctcacttcagctgcactggcgctgggcaaggcgaggacccaaaagctcagcgcagtgtctgcggcggccgggactggggttaaccagcctctggcgggcgagactccagacagaaggggggcgagaggaacgtgagcttcccgagccccttcctctcagccctggtttgcaaacctctgaaacctgaaaggggagggagttgcacgcgcgtatctttgcgtcttttcagcgcaactcccttccctctccctgtgtctctccgcggatctctgaatctttctgtctttggttttctcattctcttccaacttttccatgagattgcctatcctcgccaccagctgaaggcaaggccgttctgctacgagcgcctcttaatctctacaaaatgaaaagaaaaaaagggaggattattagcccattactcagaggaatggggaggctgcaaaaatcgtcgatgggcagaggtgaagatgtctttctcggactgcactttccggtgtcctgtaactagagttcagttgtgggacttgttgaagaaatttgattttcttgcctcggcgagatttcaaaaaccagaaatagaaattctcagagtcagagaggaaatacaattaaacagcacgtgggcattttccccctcatttctctccccttaaataacactgctttgagtttccactgggtaaagagagaaagtttgagttttcacggatgttacgtggaggttagaaatggcttaaaatgtagatctctaatcagttttcttcgtggctgaagaggctaaccctttccataaaatgagtccatctgtcgactgttagctatttcaaagtgaagggatttagcactcaaaacaaattgagcaagtttgtttgcctgtttttactgctaactcaaatgaattcaaaacacggagtaattcaagaaaacacataacatgttccagacagcccccaaaagtagggaaagcccagcacctatatagtgactagggttagttttaagcgccaagcttttttaaacgtatctattttatgcacattctcccgagtcactatatatttctaaaattgcgagtattggtatattgatttaggaagagcaatacaacttttagagggaactttattctcaattagggaccaaagagatgtctttttaatagcgggcctgagttttgctctcaagcaggaattaatattggtgggaaaatccgaatccaggagcaatggctgtgttccggcactttccaaaaacatacattaacaggatgcccttgagattgaaaaaacattgtcccatatgcctggcagaagccttcacacctggtcctccaggcgaattatatttatagtccttccactcagaggcaggacagagccaaaatattctgctcactaccaaaatacacatctttgctcaagtcaagaaatcagaaaatcagggttcagaagtaaggcacacttttcgagtgagaatatgccctgtaatttcacatactctttgctttgcaggagcaaatgtggacttgagggaaactctctcccccacccccacttctatcccgtgcaatttaataccatcctcgccaggaaccttaacctcgtcattttaaaaaatgagatatccgtgacccagggtgaacttgttgaatgtaggtacagcagaggaaattctagactctatgagcgtctgagccttgtccagtgcaaacccttcgtgaacactgggtcagtgcgtggccgtgcccacctgtgcgccgacactctcagcatgcctggtccacccgccttgacctcgggcgcggtgtcccagctaagctgggcccagcgtcccggccttccccagctgacaagcctagctcgttcgctcccggctgtggccctcccaccctctcccactagctcactccattcttctagatttctcttcactcatcctctcccatccccaccgcgcccacctccactcccgccctctaccggtctctcactttcctccctccgcagtccctctttgctgtgacctctttcctcaactctgcaggcctgaaagaaggtcacacacgcacgctcacacccacactccacacgcctcgtcccaaacaaccccatgaacattgtcctttgttccgtctcttgggccactttccctgtcgcttcctcccagcccgtcctgatttgctccccaaaagtacgtttctgtctccccgctgccctggcgctccccctttgatttattagggctgccgggttggcgcagattgctttttcttctcttccatcccatcctcccttctggtcctcctttccacagtgggagtccgtgctcctgctcctcggttggctcctaagtgccccgccaggtcccctctcctttcgctctcccggctccggctcccgactcttcggcccgctggcatctgcttccctcccctgcctcgtttctcgtcgcccctgctcgctccccccggcgctcgcccgggcgctgtgctcgctcctggatcgccagccgcgcagccgggctcggccggccgcccgcgcgccactgtgcagtggagtttggtggaatctctgctgacgtcacgtcactccccacacggagtaggagcagagggaagagagagggatgagagggagggagaggagagagagtgcgagaccgagcgagaaagctggagaggagcagaaagaaactgccagtggcggctagatttcggaggccccagtgcacccgtggactccttcggaacttggcaccctcaggagccctgcagtcctctcaggcccggctttcgggcgcttgccgtgcagccggaggctcggctcgctggaaatcgccccgggaagcagtgggacgcggagacagcagctctctcccggtagccggtaagtggaggccatctatcccgcagggatgtgagataatgcgagtctggaaatttgttccacttcggagaatcttcaccgtaggtgatttgtggcttttggggctaagtttcgcccaaggtaacgcagtcggcaaacagaccttgcaaagccctgttcctttcgtcccccgccacagacactaacaatctacagggtgctgaagtcgagagggaagccagaccgtggctggcatttaaaacgaggtatcttcccttaaatctcggtgccaacactgcaggaacaaatcctcgggccaaggattagcattctcaagataaagggctgggtacaaagtttcagctactggaagattagcccccttcccattgttatccattgggaaaaaaaagaaaagaaaaagattccatcttaactggcagttagtgacctctcaggcccaagcgaattacctgggagccaggcctggatgccaagctctcaccatttctttggattgtaactcctttaaattgatcaccagtcaactccaatctggcac

SEQ ID NO: 3 - DNA, 4001 bp, Homo sapiens
ttttcgcccttagctcacacacaccccttctgcctgcttggactttaatggctcaagacagccttgagctcactgggaaaagaaaatgactgttaaaaattatccttgaaattggttatttggcaacattcttaattgtatggaaattcattaaggcatatttcatatataattagctcaaggttgttgattctacaggctttatggatttaaatctgattgataataaagtaaacaagagagtcgaatttaaagcgtggctctctcgggttaggacgagcttaatacagtgtacaaggaatttgaaagatctaggatatgtgtcttaatcaacgttaagtagaatggataagctttcagcattttgaaaacgctgggttagggtttctcttctattgtgtgttttctgtctggggactaataagcatcacagagaacgtgatctgaggcgactttttattcttgtataaatccagagtgaaccaccaaacagttgttcgtttaaagtcaaggtaattttcttttgacgggtccatttgcttctcgatttctaatttattagcctgccttttcagggctctgtcttctttgcaattaaagcttcttcagattagcgcagcattcacttgacaggctgtttggaaaatttaagatcggagaggtgatttgttgctgtttttcaaattttctagttttaagtaacgtgtctcctttttatatggggtgggggattggaaatggatgtagtgagacacaaagagtgggtgtcttgttgatccttgtacctttctcttcttgaccattccactctcttctcccaagccttcgactcctagcctcatctcttcacctttgggttcgtactaaaagccggatcgccttgggctgggcaggagctgaattcccgggagcttgcctgtgtagacccagtgcgcacggcgaggcagtagcccggccccgcactgctgataggtgcaggcaggacagtccctccaccgcggctcggggcgtcctgattggtgcggagccacgtcagtcgcacccggagaagggtctgggaggaggcggaggcggagagggctggggagggccgcggcggagtgacgtctcggcaccaggaagcccgcctctggttttaagatgttaggccaacagggaagcgcggagccgcagatctggtccgtcgctcgcctgggtgcctggagctgagctgcggcaaggcccggctcctgttcgaccgcccgaggggtgtgcgtgtgcgcgttgcggagggtgcgctcagagggccgcgtcgtggctgcagcggctgctgccgccgcaggggatctaatatcacctacctgtccctgtcactcttgacacttctctgtcagggctgccgcgtggggggggggcgggcagagcgcggtcggcgttagctttccttattggaggggttcttgggggagggagggagagaagaagggggtctttgcccactcttgtttcgctttggagcttggaagcctgctccctaaagacgctctgagtggtgcccttctgcccacatcccatgtcttcgtttgcccgctgactttccgtctccggactttttcgcttgagccttccggaggagacgggggcagcttggcttgagaactcggcgggggttgcgtcccctggctctccccgcagcggggaaactccgcgcctagagcgcgacccggagcgggcagcggcggctacgggggctcggcggggcagtagccaaggactagtagagcgtcgcgctccctcgtccatgaactgcatgaaaggcccgcttcacttggagcaccgagcagcggggaccaagctgtcggccgtctcctcatcttcctgtcaccatccccagccgttagccatggcttcggttctggctcccggtcagccccggtcgctggactcctccaagcacaggctggaggtgcacaccatctccgacacctccagcccggaggccgcaggtaaggcgccgcgccgccctgcagacattcccgctcagctgctctgcgccacccgctccctctcgccccaaggaagtcagcccctccggggggaggcgtggtgggagtggtcgttcgcctggctccccgcagaacttccgggagccggaattttgactaccccgcatccctttagttctccctcgaccggcccggctcctggggcgctaagggcgcgagcaattctgccgccctctctattcgtaccctggcctcccttctgtttcctgggtcacaaaaatcccagcatcttgattcgaggaccttcagaggccgccgacctctgtccctgttttcctctcggctttcagctcccgaggagctccactcgttaggaaattgcctgaaaccactcagaaatgcccttcgcgaagaggcattttttttttttttttgggaaagggccggcgaacttcggtgcccaaccgaatccccacatcttttcctagccttcccaaaccgcatggaaatctgagctttctgcgagggggaggggggtctgtaaaccacgcgcgtgtgcgcgtcccaggagatttggtgtgtctgcgcagaggtgtataaatatacttgaaagcacaggctataaaagtgaatgtgccgctgcagtgagataaacatgtaaataaaacgtgcggcgctgggggaggggaggaaatggggcgcggacacccacacttgcgcctgcacaccccacaggcgcagcgctcctcgcggcccggagccgccgcgcgcaccctcctccggcgccaggcagcccagctcttccacggcttctgccgccggtccagttggcgtccgcgttgcaggtgggcatgctgacgggaaagtgtgtgtgtttcgttttcagagaaagataaaagccagcaggggaagaatgaggacgtgggcgccgaggacccgtctaagaagaagcggcaaaggcggcagcggactcactttaccagccagcagctccaggagctggaggccactttccagaggaaccgctacccggacatgtccacacgcgaagaaatcgctgtgtggaccaaccttacggaagcccgagtccgggtaggagccagcacggagtctgggagggatggggggaggatgttgtggaggtacaggccaagtagaccaggagagaatgtggaaggcagcgccgcctgggagggcgccggtggggcgcagctttgcaaaggcagaaggcctcgcggcggcctggttgcgagattacagttccctctccgaggccgacaggactgccgccctggctcaggctcccagagcggcaccggctcactgccccgccatcccgcgatctcacgagctgggctgcatgggcaatcccctgcacaggacattgtgttcctggcttgcagttgccagagcagagctaataaaatccctaccaggccaagagccgcgaacaggctccaacctgtgagcctttaacaaggaaaacccgccagagacacggaagagttggccctccctgggaaacctttgtcccggccctggcccagctttttccctcctgggctcgcgcttcttacaccttctttacggttgtttcggccattcaggtctctcccacacaccctatttcctagttttgtgatctccgggagcaaagttttaatacacaactactagtcctcttagaaggagaaagaaaaaaagaagaaagacttttctgcttggtttatttatcttctctcaggagttgaactctggaaattgaaactcacaccccctcttctaaattataatcatagttttgtaaaaagggcttaccttaactttgtagcaaatctgtactttatggattggcaaaaatgagctcaaataaataacccaatagcaacgtcctggtttatgctggtcggtggaagattccaaatttgttaggattctggaagcagaaaacagaatcaagcaaatcaagcggcatccagaggctttgctgttaaaaaaaaaaaattaagtgctctg

SEQ ID NO: 4 - DNA, 32001 bp, Homo sapiens
tatggattgcgtgattattaaatttggtattttagggggtatattttttttgagtaatttttataaatatgtttgtttgtaggatatttagattttttggtttggtagtaaagtaatataagaataattttgaatttgatgtttatttttgttttttttttaattttaggagttttttgaggtttggattaatttattgattaggaaatagtatttggaaaggttaaataaaatattatttttagggaaatagtatttggaaaggttaaataaaatatatttttttagtttttttaaattttttagaagatatattttttaaaaaataaattaagttagtaatatttaaattaaatttttgttttgtttataatataaaagatgataaaaaaattgttgggaaggtgagaaattaattttatttataattagaagtaaagtttttatttaaaaatgtaatattatttaaatttaatttgggaaataaaaaggatttaaaaaatagtttgttaaagttaatttgtaaataagtgcgttttttttttttttaagttgtattttaggtttagagtatatgtgtaggtttgttatgtaggtaaatttgttatagggatttgttgtatagattattttgttatttaggtattaagtttcgtatttaatagttattttttttgattttttttttttttttattcgttattttttaataggttttagtgtttgttgtttttttttttgtatttatgagttttttttatttagtttttatttataagtgagaatatgcgttatttggttttttggttttgatttagtttgttaaggataatggtttttagttttatttatatttttgtaaaaggtatgattttattttttttttaattattttattttttttattatttttttttttttttttaattttgaattttattatgttagtttaattatttttttttttttttttttttttgtttatttgtatatagttaaaagatgttatgaatttttttttttaatttagtatatgtttattaaagatttaaaaatattatttatattatttagaatttagtttaagaaattattaaaaaataaagttattagaaagtaattgaattattttgttgagttataattttagatttcgattttgttttttttttattttaggtaggttattttttttttttttttaaattgttttttttgtatttaataatatatttttgtggatttagaaagggtggagtatgaggaaaaggaatatgatatatgtattttagaggaaaataataaataaatattttaggatggaaaatattatttttatttttattgagttttttagagtttatttgatttgtgtaaattagaaattagtagaatgatattaatgaattaatgaaaagtagaatgagttattagttgtaataaaaagaataaagaattttaagaatatagttttaattatgtatggttgcggggagagaaaaataataaaatgtttttagtgaatatatttttgagagaagaaaggaaatatttaaggagaggataaaaagagtaaatattaaaaataggagtaagaattttattgttttttttagttgataaataaaaattgtatatatttattgtggataatatgatattttgaggattacgattatttttgatttataaattatatttaagaaaaagaaatttttaaaaagtttgggaatatatgaagttgaaagaatattaatatttagataaggatagtatatgataaattatttttgttttaatatttttttttaggaaatttaaatattttttagtgaagtattagttttttgaaattaagtatgagaaaaaaaattaaatttatttgtggaaaaaaagatatagttaaataaaaaagcggttgttataattttaagagtggtatgaataaaatgattaatatttttttaagtgatagtataaatattaaaagttttaataagtggaagtggttttgttatgataaaaggtgtggtatttgtataatttttagataagaataaagttatgacgttaagatagtagtagtattgtttgttatacgtgatatttgaaaaatatgataattattttaatttgtttaagtagtatttatggtgagggtgaaattttattaatattggttaatttatggtgttttaaaaaattagtaaggagataaattgatggattaaaagataaattatttataggtagataaatagaaggatagatagagttataattaaatatgtattttatttaggtagaaagataataattagtttttaagaagtgatgtgtttgttagaaaagttttgaatatagaattttttgattttgtttttaatttagtttttttaggtattacgttgtataattaggtgtaattttttaaaagtttttatgatagaattttttatttgttaaattaggttaataatatttttatttttttttagggtaaagatgtgaaatatttggagaattttggaaaatatgttttttattaattagagttttttgatgtgatattattttttttagtatttggagtttagttaatagatatatagtgtagttgtgaaattatgaagtatgagaatgtattattaagggatcgtaggaggttttttattgaaaagtgtagttggttatatttttggaagtaatttaaatataggttgagggagaggagtattttttagattttttttagattttattttttatgaattttaattttttttttttatttagaaaaaataatgagatttatagcgtagagatagaaaataaggttttgtgtgtttttaaattttatttttaaaaatattatagtattttggacgagatagttttgaatttttgtaatagtataggtatgagagtttttattagaaaataggagattggattgatttttttattttttttttatgttttttaaaattgaaaagttatatatataaattatatttatttattttttttggaaaaggttaaaatgaatttaattttggattatttttaataatgggataaatttgaattgagaataatttttagaattagttttgtttttttgtgataaaatggatttgtagaaagttatttggtgtttttttttagttaatattttattataaataacgggtatgtaatttagtattgttttttataggttatgtttttggaattattatttttgtattttatttgtttgttgatatttttttatttaagatgttttttttagtataagaagttattttttttaaaattttaaatgattttattataataatagagttgttaattagatttaggtaagtaatgataataaaaatttgatttttatttagagtgtagtatggtttaatataataattagagttttaataggtttttttagattttatttttatttaatttgtatgtttttgtaatatagatgtttttattattcggtttttatttttatttttttttgtttttggaataaaattatttaaatttaatttagagattttatttttttttggaattattgggaaatagttttagtaaattatatttttgagattttatattaggtttagtttaaattgattatttaagtattaatttttttgtggtttaggaatatttttgagtttatttttttttttttaaattgtttaggataaatatcggagtttggtttttttgtttttttatttaattatttttcgtttttttttttttagtatttaaaatatttttgattttttttattttttaagaaatatatttgtttttttgtttttgtattatttttttgtttatgaaatattttataggtaagttttatattttttttttttagaggtttttggttttttggttttagttgttattggtttagtgtattagttaatattttggattttggagttatataaatttagatttaaatttttattatgttatttattgtttacgtgatttgaagtaatattttatttattgtggtttttagtagttataagtttgtgttttaattagttgggtgattttgggttagtgatataattatggtaaattttattgtttttatttgtaaaatgatagtatttattttgtagtgttggtataaggaataagtgtgattgttaatataaaagtgtttagtataatagttaaattaattaagtattttgtaaatattagtttttattattattattaatttaaatgattagatgtattttgtgtatattaggttttttgagtttattttgtttttaataaatattattatttttagtatgtggtttatattatattttattagttagaggatatgtgaagtttagagtggaaagttagggtagtaggaagtattgttatattttatatagttaaagttatttaaatatgtttgaatttgagttttgttgagtttttatttgtttttattttttttgtgtgttttagtttattaataaagtaggtttaatataaatatattaaaagtttaaatattgagattatgataatgaatatgagggttatgattataaaatattattgaattagagatttgttacgaaattatatggtgaagattataagggaggaatttgtatatatatcgagtgttttgggattttaaagtgggaagagttagtgttttaattaaagagaaattcggggtagggaattaattataatattagttattttattgaatttaggtttgttttagttgacgtagttgttaatttttaatgttttttttttttttaattgtttttaatttatttttttagaaattgaaagtttattaaagaggatatttttttagagagttgttttagttattataagtttttgttagaaattttaagaaagtttataaggtatttttataaggtggtattgagtaagttagaagtattttaagtattaattattatgtaaataagggttttatttttagattttgttgtttgtggtggtggtgatgttggtgttttttttggaatttagtttaatttttaaaaaagtaaaaggagtataaatagtaatataaattattattatttatattaattaaaatagaagttttgaatgagtaaggagttagaggaggtaaaaattgggaatttcgtatattaaaaggtttttataatttgaaaattaagattatgttggttaaataggttgttttaaaattagtatagtaattaaatttgtttgtaatgaatgtagatttaaatagtgatgttagatttgataaggatttgtaaattttaaaagagtgtaaaaagattatagaagaataatattatatttttgtatttatagaaatggttagtttaagagatgtatttagtttagggtggttgtaagttttattttttgaatttgttattagaagttaaaagaaattttgtataattgtttttgatggaaatataaattggttgatgtaaatgaaatatataaagtagttggtgttttatttatttttataattataaatgaaattaaatgattaaaaattatagattttggggattttttttttattgaggagtttatggaatttgttttttttagtattaataattgtgttgatttatttttttttgtttaattttgtatatattaaaattaggtggttacgaataaaatttagaaatataatttatattttaataaaatgattttaaaattattttattttttattgtggttttatttgttgttttataatgtaggtttttttgggtttttgtttagaatgattttgttaatgtagatgatagttagagttgaatggggaatttagaaattggggattcgggtttttgatgtaatttatatgttaatttattttattagttttttttttatttatagtttggtaaagaatatgggtggagttgttttgggtttatttgtatatatgtttaaattgttttgaaaaaggaagggtaagaaagagtggtatttaagttggaattaggtaggtattttagattaagagacgaattggaaagggaatatttgttagatattttgggtttgaaggtagtttgtgtaagtttttatatttttgagtgtgtgtatatagtggagagggtggagtttgttatttttaaatttgaaaagattgagagattttagagggtttagatgtgttaaaggttagagggattaatatataggttttattacggaaaggcggggaaaaggttcgaatagaaaattgttgtagaagggaagttattgagaggtaagggagtttttgaataattaaaaagttaagaataagtaaaaggaaggaggtcgggtgggggataaaaaaaagtagttgatgtggtaattaagaatttggtgggagtttgggtaggttatttttttttttagattagagttttattagaaatttttttaagtgtttttttgcgtcgttaaagatgataatagtaaattaataagtgtttgaaatgaaaggggatgttgattagtttttaggttatagatttttcgtcgttagttttttttgaatttttatagcgtgtttttgtatcgttttttttaagaagagttattttttatttttatttttaggacgaaggtaagtgtttagttagtatatttattaaatgttagttttggttttagtttttcgtttgcgcggaaagtttattgttatagcgcgtttagtttgtcggaggggtagatagaaaaagtaagtttggtttggcgatttgcggggttacgtatttttagggttggttcggagttttttagagtttaacgtttttgggttagaattgtaaggtttcggttcgagtaaagggtttgagttatcgtagtcgtgggagcgttttttttatttgaatgtatttatttataaataagtataaaatttttttaatagtagaggagaaagatttttgttttaaaattaaagttgggaattatcggaaatttcgttttgagtgcgagatattggtttgttatttttttaatttttatattttttttgtaatatgttttgatttaataatttttttagcgtttagtattgttcggacgttttaattgggtaatttattagtgagttaatataggtatttatatatttttttagtttaagtggttaagtattaatttcgaaatgattataaaatatcggaatcggtaacgtatagtaattttaatttatatgtaaattaattggtttattttaaatgttttttttaaaaaaataattattgtattgtagtatcggaggtatggattaaatttttagaatagataattcggaaataagatttggattaggaagataatttagaatagttaataaattaataatgtttgaggtagttaaatatcgttagttattggtatttatatattcgtttgttgttagataaggagttggggaaattgtttgttagggttgagattataatttagagtgaagaaagtaaatggtagtatatagttcgttatagcgggttttgaaataatattgtattttttttaaattttgatttttgggtgatagggagttggcggaggttattttatatttgtttacggttttgttttaatttgattacgaaattgttgttttttttgagttttttaatttgattattattttaacggttttgttatttgttttaatatattggggggaggagtgtaattgagatttttattaaaaattatttgaatttatttagttagtattgttttatttaagtttagttttatgggttgtatttaattttttgtgttttttatatattaaaattagattattaaaatgtcggtaggaaagggtgaaggaaatggtttaatgttttagtttattggaagattattatttttagatatagtttaaaattttgaggaaataaaaaggatatacgttttggggggaaaatgttttaatattttagaatgggggtattattttttttattttagagaattcgtattggagttgtttatgtaaaaatgtaatatttttgaaatttatagatacgtaaggttagtgtttttttttttttaggtttttagtttaggcgatttagttttaaaggagttagtatttttgatgttataattttgtttatatttgtagggtagagaattgtttgttttgtttggacgttttttttatttttttttaatttgaagtaatcggaatttaaatatagtcgttaaggttcgttttttttttattgttttgataagggaaaaatttgaaatttacgttttaaattagttcggtggtttgtagttttttagtattttgtttttacgattgtatgtttaatgtattttttggtgattttgggtattaattagttgtttaataggagtatgattaaaaatgtaaaagaaggattaggagcgtgaaacgtatgtttagttttttttatatattcgaggagggaatgagaattattttgtattttttatttttttaggagttatttgtattttttattagttgtttattttagttgtattggcgttgggtaaggcgaggatttaaaagtttagcgtagtgtttgcggcggtcgggattggggttaattagtttttggcgggcgagattttagatagaaggggggcgagaggaacgtgagtttttcgagttttttttttttagttttggtttgtaaatttttgaaatttgaaaggggagggagttgtacgcgcgtatttttgcgtttttttagcgtaatttttttttttttttttgtgttttttcgcggatttttgaatttttttgtttttggtttttttatttttttttaatttttttatgagattgtttattttcgttattagttgaaggtaaggtcgttttgttacgagcgttttttaatttttataaaatgaaaagaaaaaaagggaggattattagtttattatttagaggaatggggaggttgtaaaaatcgtcgatgggtagaggtgaagatgtttttttcggattgtatttttcggtgttttgtaattagagtttagttgtgggatttgttgaagaaatttgatttttttgtttcggcgagattttaaaaattagaaatagaaatttttagagttagagaggaaatataattaaatagtacgtgggtatttttttttttatttttttttttttaaataatattgttttgagtttttattgggtaaagagagaaagtttgagtttttacggatgttacgtggaggttagaaatggtttaaaatgtagatttttaattagtttttttcgtggttgaagaggttaattttttttataaaatgagtttatttgtcgattgttagttattttaaagtgaagggatttagtatttaaaataaattgagtaagtttgtttgtttgtttttattgttaatttaaatgaatttaaaatacggagtaatttaagaaaatatataatatgttttagatagtttttaaaagtagggaaagtttagtatttatatagtgattagggttagttttaagcgttaagtttttttaaacgtatttattttatgtatattttttcgagttattatatatttttaaaattgcgagtattggtatattgatttaggaagagtaatataatttttagagggaattttatttttaattagggattaaagagatgtttttttaatagcgggtttgagttttgtttttaagtaggaattaatattggtgggaaaattcgaatttaggagtaatggttgtgtttcggtattttttaaaaatatatattaataggatgtttttgagattgaaaaaatattgttttatatgtttggtagaagtttttatatttggttttttaggcgaattatatttatagtttttttatttagaggtaggatagagttaaaatattttgtttattattaaaatatatatttttgtttaagttaagaaattagaaaattagggtttagaagtaaggtatatttttcgagtgagaatatgttttgtaattttatatattttttgttttgtaggagtaaatgtggatttgagggaaatttttttttttatttttatttttatttcgtgtaatttaatattattttcgttaggaattttaatttcgttattttaaaaaatgagatattcgtgatttagggtgaatttgttgaatgtaggtatagtagaggaaattttagattttatgagcgtttgagttttgtttagtgtaaatttttcgtgaatattgggttagtgcgtggtcgtgtttatttgtgcgtcgatatttttagtatgtttggtttattcgttttgatttcgggcgcggtgttttagttaagttgggtttagcgtttcggttttttttagttgataagtttagttcgttcgttttcggttgtggtttttttatttttttttattagtttattttatttttttagatttttttttatttatttttttttatttttatcgcgtttatttttattttcgttttttatcggttttttattttttttttttcgtagtttttttttgttgtgatttttttttttaattttgtaggtttgaaagaaggttatatacgtacgtttatatttatattttatacgtttcgttttaaataattttatgaatattgttttttgtttcgttttttgggttattttttttgtcgtttttttttagttcgttttgatttgttttttaaaagtacgtttttgttttttcgttgttttggcgttttttttttgatttattagggttgtcgggttggcgtagattgttttttttttttttttattttatttttttttttggtttttttttttatagtgggagttcgtgtttttgtttttcggttggtttttaagtgtttcgttaggtttttttttttttcgttttttcggtttcggttttcgatttttcggttcgttggtatttgttttttttttttgtttcgtttttcgtcgtttttgttcgtttttttcggcgttcgttcgggcgttgtgttcgtttttggatcgttagtcgcgtagtcgggttcggtcggtcgttcgcgcgttattgtgtagtggagtttggtggaatttttgttgacgttacgttattttttatacggagtaggagtagagggaagagagagggatgagagggagggagaggagagagagtgcgagatcgagcgagaaagttggagaggagtagaaagaaattgttagtggcggttagatttcggaggttttagtgtattcgtggattttttcggaatttggtatttttaggagttttgtagtttttttaggttcggttttcgggcgtttgtcgtgtagtcggaggttcggttcgttggaaatcgtttcgggaagtagtgggacgcggagatagtagttttttttcggtagtcggtaagtggaggttatttatttcgtagggatgtgagataatgcgagtttggaaatttgttttatttcggagaatttttatcgtaggtgatttgtggtttttggggttaagtttcgtttaaggtaacgtagtcggtaaatagattttgtaaagttttgtttttttcgtttttcgttatagatattaataatttatagggtgttgaagtcgagagggaagttagatcgtggttggtatttaaaacgaggtatttttttttaaatttcggtgttaatattgtaggaataaattttcgggttaaggattagtatttttaagataaagggttgggtataaagttttagttattggaagattagttttttttttattgttatttattgggaaaaaaaagaaaagaaaaagattttattttaattggtagttagtgattttttaggtttaagcgaattatttgggagttaggtttggatgttaagtttttattatttttttggattgtaatttttttaaattgattattagttaattttaatttggtattttaggagatatattttaaatggatgtagagaattattttttagttggagattaagaaaaaaattttcgattttaaattttcgaaatatgttttttttttttagtttaattattttatttttttaagtaatttagaaattaaattattataaggtggtgtgatttttttttatttttttgtgtgagtattgttttattaaattaaacggaaaaaatttttattattataaatgtaaatattagaatttatatattttaaaatatttttatgaaaaattaatttgatttaaagaaatttttttgtatttgttttagtttattaattaaaattaaagatgtttttattatataaaatattattttggtagaaatttatttaaaatttaaatattaataatattaagaaaataaagtatataagtaaaataaattgaagatttttgttgatgtaatatgagtatataatattttaataattaaattttttttaaaaaattaaatagttattttatttgtggaatgttttattttaatttagtaaaattatatttaaattatttaggtgttttgttttttaagttaagcgtgtttgtttttaaatgtttttaaagtatttatattaattggttgtaaagaacgtatatatatggtaaaatatagaattgaattgagtagtattttaatttttttaaataattatttattataaattaatttattggttaattttataatttagtttatttaaaatatatgtttttgtgttgtttatttttaaattttttattaaagattttgttatggggtaataaagtgtatgaaaaggggggaaatgtgaaaggatttgggattattcgaattgtattttttttgtatttttagttttgcggtagttattagaaattattttttagtaaattgttttattttttagggtttgtttgtttgttttgttatggtttttcgtttttcgttagtcgtgtagtgttttttgtgtgtttataatataaaatttaagttggttaaaataagagtttttggtatatatattttaattagaatatgaattttgggggtgagaattattttttattaggaaaagttttttattttaatttgtgagattagttattgaagttagtttcgaagtttggtagttaaattttttatagaagatttgttttgatagggtaagtttaaggattagtaggcgggaattggaggtttttttttaaaaaattattttttttagttatttagatttagtttttttagtaggtttggttattaaatgaagtataaaaatgtaagttttaaggtttattttgattgtaaaataaatttttaagttataaggatatgtaggagtgagttaaggaatacgttttgattttttttttagtttttagagtggagttttatgagtttttgaagatttgttttgtattgttttgtttggtttttagtattgaagtacggggaagtggggggaagaatgtgtaataattgattgattttatattaagtaacgtaattttttttttttgtatattttattttttaaaaaaaataaataaataaaaattatttgtagttattatttgtagtgtttcggttattagttaataatgtagttagtttagatatataaaaaaaaaagattatcgaaatgatgatgatatgtaaatttttttcgaaattattataagtaaatatttgaagtttggattaataaaattttatttgtgttattttatatcgagttagtagaaagttgtgataatgaattttgtaatattttacgaatagatattttaattagggattaattttgtgattttattgtagaattattaaatttggagtcgttaaattgttatttttgggtttacgggtttataaggatcgaatcggtagagttttcgttcgcgttttcgttagcgggtgggggaatcgtttggtcgtttttattttggatttttacgttatagcgtcgggtagttttttttgtaggtagcgattttggttagaggttttttagggtttagttttttttaggagaggtcgagacgtagggaaacggtatttaggttagaggtaggttcgtagttttttgtttcgtttttgtgttttcgttaattcgataacgtttgtttttatttcgattttcgtattcgcgcgaagtgggtttttcggtcgtcggcgtattttggttagcgtggagagaggtaggcgttgagatcgaaggggtttagggagttttggattttttttttttgtttttaaagtaatcgcggtttttttatttattcggtggagtttttcgagatttatttttttcggtttgtttgtggtagagaagggggagcgcgttaaatgtttggttcgttgcgttgtggttgaaaacgtgaaaaagatttggttcgttcgggagagaaagggggagaattgggtagtagttatattagagttattttttcgtttttggcgggtagtaaattttttaagaacgtttgttttgttttttttagtttcgtttagtttatttagtgttttttttttgcgattttaaattatattttagggtaattatttgtagtaagtaaataaatggtcgggttagtatttttaggagaaagtgtggttaaatatggaaaagtggtttttgatggatgagaggttcgaatttagttcgtttttgaaatattttaggttaagagttcgttcgttttagaattatagaaaatcgagggaaattgttgtttaggataggggtacgttggcgttgatgttttataaatgtttatcgagttttaattaatggataagtattgaagggtggtttttgtatatagttttttaaagagaaaagttttttttatttatttattttcgttgttattgcgtttagatgagtttttaatttcggtatcgagatttttgaaagtaggtttatagtttttttagtatattgtggttttatagttttttaatttttgggtatttttgcggtaattttggagggagatttttttttgataaataaatgttttgggttcgaggttaggttggagatgttgttgtatagttagaggttgttaggtcggaaaaatacgtttgaagtttagtatatagtaggcgtttaatagttagtgtaacgtagttttatttgagttttgtttattcgacggtcgtcgttttttatagtttttttttttttttgttttgtagataacggggaatggagattaattgtcgtaaattggtgtcggcgtgtgtgtaattaggtaagaattttttttttttgttcgggttatcggacgggaggtcgcgttacgtgagggcggtaagagggtattggttttgcggcgaggttttagcgaggggcgttttttcgaggggttagtttgggtaggaaggaaattagaattaaatcgttagtggtttttttttgtggcggggcggtggattaggaagtagcggcgcgttgtgtatcgaagttttttagtttatttttttcggttggaatcgtcggtaatcggggaggcgtagaaagagtacgttattttgtttcgggttgttagagggttcgggggacggggatgtcgttagtttttttttttaattgggtttttgttttttgtttttttttttttttcggtttgtttcgttttttttttttttttcgttttcggtttttttcggtcgcggttcgggacgttttttttcgtacgtggggcgggcgcgcgcgtggtttaggcgtgtagtcggcggtcgttgaatgttttttttttaaagatttcgaaattaaaaaggtcgagtttacggatttttttgagagtcgaaaagaggtagttagtagtaagtttttttcgcggtagtattttggcgttaatggtaaggtcgggagggaagcgtaggtcgcgcgttgggtattcgttttcgggattttgggtttcgggcgaagcgtaagaaggcgaggtcgttagatttgacgcgtttgttgtttgaatttagatatttcgtttttgggtgggacgggaagtagtcgttttagggacgttaatttttttttttaaattatattgtatttttgagatttaatatttttttttttttttcgttcgttttttgtggtttgattttttgcgtacgttttagtaaatttcggcgtttaggttggcgtggaaaagtggtttaatagcgatttttgtcgttcgttatatttcgttgcgcgtagtattattagggtttatttagttatttaggtttttagttacgttttatttagatttgtgggtgcgcggtttatcgcgggaggtaagtaagggaaatttgagttggcgaaggtttgttttggttggttgggggaggggcggggggtcgataatatttttgaagagttggagggtagttattgtgtttagtagtttagggtagaatggaggtttgtttttgtcgacgcgaatttgtttgaagtattggttgttaggttttgggttttggcgatgtcgttgtttgattggttggttttattttggaggaatcgagggatattgttagaggaggtttataggtttatgtaaaaagttaaaaagtttttaatttacgttataggttttttttgaattgaaatttgttttatggggcggaggggggggtgtaagggatggaggagggaagatgtttttttttttaaatatatggaaaaaaattttttaaatttattgtttttttatttttttggtttcgtagtaaataagtgtttagttttaggaggttattgatttttgataatgtgagtagataaagtttttttttttttatagttttcggtttttaatttttttttttcggattaaagtgtaagaatataaatgtaatatgggatggaggggggcgatttgggatttcggttaaaaaaataaatcgtattattaagaagaaaataaaggttttgtattggagttttttcgtgaatttgagagaaaatgattatttgttgaaatgaagcgtttaaagcgatttagtgttttacgttcggatattgtattatatcgttagtcgttttgttgggttagttaaacgtttatttgttcgggattaattttatggggttaaatgggggtaatgtagagataacgtcgcgtgatttttgttatttagattgtgttaaattttttttttgtttgataatcggtagtaaaaataaattattagatcgtagtatgtttgggatatggttaaaaattaagagtagcgatgatttttggggagaatgttttgcgcgggtttagttttggtttcggttagattagaggagttttttaatttcgtttcgcgcggggcgggttcgtagtcgttaagtcgaggttgatattttttattgtgttgggagttagagagacgtaaaatgttttttttttttagtttttattttaggttttttagatatggggaatgtattttgaggataggtggagaagtttacggtaggatggggttttcgtaggtgagtaggaaacggttaagagtagaggagttttgtttgcgttagttataagtcgcgtaggcgtttttggtcgttcgtttttgataattagtatataaagaattagaaataatgaatgattgtttttttaattattatttttaggttcgtattgttttagtgtacgtgaaaggttttttttttatatttaatatgtttttttttattttttgatcgaaaagaaaaattgttgtttaaatacgtttaatgttattaattaagaaaaggtatgtaatgggaagaaatgttgaaaattttgatttaattggtttttaaggaattagtagacgataaaaaaaaattatacgagtgggtaaagttatagtattgttgaaggatagagtatttatttttttttgattttaagttaatttatggaatatttaaagttttggttatagtttgtttgtaaaataaaaggatttattttttgtgtttttttaaagtttttttttgtttttaaagagaaaaaaagtttataatgatatatgatttttttaaaaggtcgtgatagtttattacgttatttttttcgtttttgtttttaacgtcgtttaaaaatattatgttttcgttaaagattaaacgttttgtataggtagagtttatttttaagtagtttaggttttgttttttttttttagtgagttttattttttttggtatttattgggcggatgtttagtttggatagaatttcgaaacgggggtagtacgagagcgattggagatttttaaaagttagaggtttgagagagggtggacgtagttagtagaagatggtgtagaagttagttgagaacgattttttagagtaaagagatttttttttggttttttttgttttgggggttttgaaaggaatttataaaatggtttttatttttaggaggaggacggattgatttttttttgttattggtttaaaaagttttagggcggcggttttgggtttcgtgttgaaatcggattgtattgtagtttttttggatttgacgtttggttttgcgtttcgataaggggcgggtatttttttcggttttttttaggaacgtattaattgttaaatagttttggtttagtggatgggttgaaagtgttcgatttaagtcgttggtgtgtatagattttttttttttgggaggtgggttttatggttcgttgtggtatttttagtcgcgatatatatttttatacgcggtagtagttcggttttaatttttttcgaaggatttgggttaattttggcggttttggcggtcgtagattttttttcgtcgtttcgttttcgcgttttttatttaattagcgaatgtttgcggagtatatattacgtggatttttaatgtattttttgaaagtaaataatatagtttttttcgtcgttatgaagggattttaattttaatatggatattagcgagattagtttagatcgtttttagtaaaacgtaaaatggtggtgcgtggggtggtgattaaggttttgagttttgttagaaagaaggggatgtgtagagaaaggtggagaattttagttgtggttagcgcggaagggataggtgtttgtcgaagggggtatgaggtttgaggaaaaagtaacgaaataggggtaaggagagttttttattttttttttttcgttcgattttcgttattttatttttttttttttttttttatttttcgcgttaattaaatttgtagtttatttgaaaggtgtttcgtcgcgttgtggttttttatttttaggggaaattgtattagttgttcgaaagtagttagtttttgcggatttttgttcgtaaaagtggtttttataggtcgcgtttttcgttgttgattcggtatataaagttttttaaggttggttcggttgttattttttatcgttcgttgttaatatatgtagtagttgttagagcggttcgggggaaaaggaaatgtataacgaaagtttattcgtgagtaggaatatattaatggaataatttgatgtttttttaattttatgtaaaaagttttgtcgtttttttaatattgattgaatgggtaattaatggttttttatttaggcgaatattttgtaatttaagataggtaaaagataataagtttaaggtagaagataaaaggtttaattgtagcggcgtttgttcgttttttattttttagggtttttgattaggaaagtttttttttagaggagaaaaaggtaggagtgggagaatatatatttattatttcggggttagattttatcgtagtatttgattatttagtttagttttttgttattttgtttttttatttttagtttttttttttgtatttttttttttttttaatttttttaggatgattttttattattatcgttattatggttttaataatttttttttttaaattttatattttttattttagtaattaatgaggttgttttttgatttaggaggagattttttttttttagaatttaatgcgtagagtttttgagaattaaagtagttggtaggggaggaagaaattaatagaaagggagagagtatatagaattgtgtgtgtatgttaaagagcgattaggaatgatagagttaatttttttgtgaggatttgacgggaagagtgtttaagattttattagtatgtttttaataggttgatattttaatttaaatttttagaagtaatatattatttgggttattataatgaggtgggtttttttttttttgttagttgatagtttttaaaatattatttcgttagggaaataaaagttttattttagattataggtgggtatttttggatttaggtgatttatggttattatgataattaatgttgaatgttagttattagtatgtttgggagagagaaaatagaaagaagggagagtaaaagaaatagaaaagggagatggatataagttggagagggaagaaaagagaaaaagaggaagatagatgagtgtttaatttaattgttgtttaaaaaagtggcgggggggtgggattttatttagttttttgttattttttttttttttgatttggatatttatgtttaattttatattttatttttttttttttttttttaaatatatgtgttatattattttttttattttatttagttcggtaagtagttgttttttggagatttagtgatatttaggaaaattgtggtagtaatatgtaaatgtgaggaagtattaatagtatgttcgttgagtgattttagtaaatgtttttttttttaatttttttttttttttttttttaggttattgtgaggtggtaatttttattgttatttgaatattgtttttttaggtagttattttaaattttaaatggttgagtagttagagttgtgggttggaaaaatgggtattatttgtagggatttagagagggtggttgttgtttaatatatttatagatttttaatttagaaaataattttttttttttgataagttagagttttttaaattttatttaggaaatggggaaaaggatagttatagtgaagtttttaatttttgggttatttggttttatagttatgaggggtggtgggtagtggattgtttttagtttggtttgtatgtagagaaaagttagatattggagggggtggggtatttttcgggtaggatgtaaggtttttatttgatttttgcgttttattaggagtttatatatttacgtttattacgtggttttaagttgagtttaggcgggtttcgtttttgagttagtttgggtagggtaggatttttattcgtttaaggtttaatagtttagggagatgtttaattaagttattttttgggtgaattttgaagatagattttttttaaaagttagagattatttggttgagttttaggttagattgatacggagagtttggcggtatagtttaatcgtttattgttatggttagagggattttgtataattaatattgaagagtgtgaaattaaataagattttaagattggtaatcggtggtaaatattagtataaaatacggttgattttatgttatatattttttttttttagggtttttttttgaaagaataagtaagaaattttaatcgagataatttttgatgttttttagatttaaaattttacgtcggtattgggttttttttttttgttttacgtgagttatgtagtatttttagtttttttattaggattttattaatgtttttcgtattggaaatttttgtgttagaggttgaatttatagtaatttttaaaattaattaagaagaatttagttagaggttatagtaatgttggaattataaaatgtataagatttatttttttttggttttttttttatttatgttgtttatgtttgtgtatttataagttttatgtatattaaatttttaaaattaattattattatgttatagagtttttattggatagtgttttttagtttttattatatatttttttttttttatgtagatttattatgttggtgttttgttatatagggggtttgagaagaatgttatttaatcgtcgttgttgtgagtgtgtaaagtgattaggagattaggagaatgttgaaatttttgttggaaaaatgtaaagaaaatttttattttgagttagttgtttatagagttagtgtgtgtgtgcgtgtgtgtgtttgtaatataaaatggatgtgaatatatatatataaatagatatggttttgtttttattttaatttgaattatttagataattgtttttatttattatttgattttaatgggtttatataaattaggatattttatttttttaggtatttaggttgttgttgatttttagtgtttttaatatttcgtatacgttggtattatgaggagtagttacgtgtttttgggttttttaattattttggaggttgattgaggttttttatatatgtatatttgtcgtgatgaaagttttatcggtagagtggagttattagagtttttattaaaattttgtgggtttatgagagatgggtttagaaatttatatggttttgtggggtttttcggttttttaaaataaggtattaatatttaagtttttaaaaatatttgtagttttggggtttgaattttgaaaaataaggagtgaggggttgtgtatattaattatagtggagattttttttattttttaatgtgatggagtttttttatgaaatgaagttttaaggggtatggtattgtggggattatagttattttgaggtttaaaagaagaaattggaatatgattagtaaatatatttagtagaaaagagttggatttttattgatttagttataggttatcggttggtagtgtaatgggaggaaatatttattttatatatatattttatgattttgggggaattagaggaaatttaataagaaaacggttagaaatatttaaaatttttatttaaaagatttaagtaaattagagttttattagattaaaaattattataaatgtaagagtattgtttttagtgaaacgttgtggggtttgagaaggagatttttcgttaaattttcgggataaaatgcgttatttaagtattagataatgagtagaatgtaaattaatttaattttttttattaataggttgttagtgtaatgtgtataatttagtgataagattgtaggatttaatatagttggatgtatgagttttagttaatgtagatttgttatatgaggatgtgttttattttgagtaggtgtttgtatgtgtggaatggggtaaagtggaataaaaggttaaaagtagaaatgttgatttaaagtttattatgaagaaattttttttttgtagttaaattatttttaaagtgggatgatattggtgaagaaagattgaaaaataatttttatgtgcgtttttggattgtaagtttaaaatggggaggagttgtagatagggtttgggggtggttagggtaaaggagagatatataagttgtaaatatatttgtagtttgttttatttattttgttttatatcgaataagttttttaattttgtgaataaggataaggagggagtgttttaaagatattttatgttggtattgtaaattattgattgtaatgttaaataaatatatatttagagatgataatattaattttatagtaaaataatcgtttatgtagaaatttagaggagattagtttgttttttttagttgatttatgttgggggataaaaggatttttaaaaattattttgaatatgtttggatttttttttttaatttttttggaaattaaatttgtttggaaatagtgttataaagagttgatgtttttaaaggtgattttttttgttttatataaataaggttttgtttttgttagttgagcgtagttttaggtttttcgtttttagtttatatatattttttttgtttgtttggattttaatggtttaagatagttttgagtttattgggaaaagaaaatgattgttaaaaattatttttgaaattggttatttggtaatatttttaattgtatggaaatttattaaggtatattttatatataattagtttaaggttgttgattttataggttttatggatttaaatttgattgataataaagtaaataagagagtcgaatttaaagcgtggttttttcgggttaggacgagtttaatatagtgtataaggaatttgaaagatttaggatatgtgttttaattaacgttaagtagaatggataagtttttagtattttgaaaacgttgggttagggttttttttttattgtgtgttttttgtttggggattaataagtattatagagaacgtgatttgaggcgattttttatttttgtataaatttagagtgaattattaaatagttgttcgtttaaagttaaggtaatttttttttgacgggtttatttgtttttcgatttttaatttattagtttgtttttttagggttttgttttttttgtaattaaagtttttttagattagcgtagtatttatttgataggttgtttggaaaatttaagatcggagaggtgatttgttgttgttttttaaattttttagttttaagtaacgtgttttttttttatatggggtgggggattggaaatggatgtagtgagatataaagagtgggtgttttgttgatttttgtatttttttttttttgattattttattttttttttttaagttttcgatttttagttttatttttttatttttgggttcgtattaaaagtcggatcgttttgggttgggtaggagttgaattttcgggagtttgtttgtgtagatttagtgcgtacggcgaggtagtagttcggtttcgtattgttgataggtgtaggtaggatagtttttttatcgcggttcggggcgttttgattggtgcggagttacgttagtcgtattcggagaagggtttgggaggaggcggaggcggagagggttggggagggtcgcggcggagtgacgtttcggtattaggaagttcgtttttggttttaagatgttaggttaatagggaagcgcggagtcgtagatttggttcgtcgttcgtttgggtgtttggagttgagttgcggtaaggttcggtttttgttcgatcgttcgaggggtgtgcgtgtgcgcgttgcggagggtgcgtttagagggtcgcgtcgtggttgtagcggttgttgtcgtcgtaggggatttaatattatttatttgtttttgttatttttgatatttttttgttagggttgtcgcgtggggggggggcgggtagagcgcggtcggcgttagttttttttattggaggggtttttgggggagggagggagagaagaagggggtttttgtttatttttgtttcgttttggagtttggaagtttgttttttaaagacgttttgagtggtgtttttttgtttatattttatgttttcgtttgttcgttgatttttcgttttcggattttttcgtttgagtttttcggaggagacgggggtagtttggtttgagaattcggcgggggttgcgttttttggtttttttcgtagcggggaaatttcgcgtttagagcgcgattcggagcgggtagcggcggttacgggggttcggcggggtagtagttaaggattagtagagcgtcgcgttttttcgtttatgaattgtatgaaaggttcgttttatttggagtatcgagtagcggggattaagttgtcggtcgtttttttatttttttgttattatttttagtcgttagttatggtttcggttttggttttcggttagtttcggtcgttggatttttttaagtataggttggaggtgtatattattttcgatatttttagttcggaggtcgtaggtaaggcgtcgcgtcgttttgtagatattttcgtttagttgttttgcgttattcgttttttttcgttttaaggaagttagttttttcggggggaggcgtggtgggagtggtcgttcgtttggtttttcgtagaattttcgggagtcggaattttgattatttcgtatttttttagttttttttcgatcggttcggtttttggggcgttaagggcgcgagtaattttgtcgttttttttattcgtattttggttttttttttgttttttgggttataaaaattttagtattttgattcgaggatttttagaggtcgtcgatttttgtttttgtttttttttcggtttttagttttcgaggagttttattcgttaggaaattgtttgaaattatttagaaatgtttttcgcgaagaggtattttttttttttttttgggaaagggtcggcgaatttcggtgtttaatcgaatttttatatttttttttagtttttttaaatcgtatggaaatttgagttttttgcgagggggaggggggtttgtaaattacgcgcgtgtgcgcgttttaggagatttggtgtgtttgcgtagaggtgtataaatatatttgaaagtataggttataaaagtgaatgtgtcgttgtagtgagataaatatgtaaataaaacgtgcggcgttgggggaggggaggaaatggggcgcggatatttatatttgcgtttgtatattttataggcgtagcgtttttcgcggttcggagtcgtcgcgcgtattttttttcggcgttaggtagtttagtttttttacggtttttgtcgtcggtttagttggcgttcgcgttgtaggtgggtatgttgacgggaaagtgtgtgtgtttcgtttttagagaaagataaaagttagtaggggaagaatgaggacgtgggcgtcgaggattcgtttaagaagaagcggtaaaggcggtagcggatttattttattagttagtagttttaggagttggaggttattttttagaggaatcgttattcggatatgtttatacgcgaagaaatcgttgtgtggattaattttacggaagttcgagttcgggtaggagttagtacggagtttgggagggatggggggaggatgttgtggaggtataggttaagtagattaggagagaatgtggaaggtagcgtcgtttgggagggcgtcggtggggcgtagttttgtaaaggtagaaggtttcgcggcggtttggttgcgagattatagtttttttttcgaggtcgataggattgtcgttttggtttaggtttttagagcggtatcggtttattgtttcgttatttcgcgattttacgagttgggttgtatgggtaattttttgtataggatattgtgtttttggtttgtagttgttagagtagagttaataaaatttttattaggttaagagtcgcgaataggttttaatttgtgagtttttaataaggaaaattcgttagagatacggaagagttggttttttttgggaaatttttgtttcggttttggtttagtttttttttttttgggttcgcgttttttatattttttttacggttgtttcggttatttaggttttttttatatattttattttttagttttgtgattttcgggagtaaagttttaatatataattattagtttttttagaaggagaaagaaaaaaagaagaaagatttttttgtttggtttatttatttttttttaggagttgaattttggaaattgaaatttatatttttttttttaaattataattatagttttgtaaaaagggtttattttaattttgtagtaaatttgtattttatggattggtaaaaatgagtttaaataaataatttaatagtaacgttttggtttatgttggtcggtggaagattttaaatttgttaggattttggaagtagaaaatagaattaagtaaattaagcggtatttagaggttttgttgttaaaaaaaaaaaattaagtgttttgggtagaaaaaataaagttttcggttagagtagagtaaataaaaagaagaaaataacgataaaaagaataaagattaaaatgtttttttaaattagagggaatgaagatattttttgggtggtatttgtgtaaggtatgaggttatgttggtggataaaaggtcgggaagaagttgaaaatggttttagtttaattgtttagagttagagttgggttttgggcggcgtggttttgagtaaggttagttttttattagtttttttgtatattaagggaacgggttttttacgtatttttttcgtttgagtaaagtttagatggtttagggtagaaatggtaagtaattaaagatagagtttatgggttttttgggatttttcgaaaacgtttttttatttcgttcgttatttcgtagttttattttagtgttttgtagtcgcggcgttgggttttttttgtagttgtttttttttttagggcggttgtttgtcgagttaagtgggagtgaggcgtgttttttatagtagtcgggtgtaaagaggaagggggataaaaaggaaattaagaatgaaaggaaaaagagaaaaagcggattatacggttgggttcggcggagatgtgtaatgtgaaatattattggtgttagttcggatattttaggttaggtttttttttaatatataaaagtcgtcgtttggggcgatagggaggttcgatgtggattgggatcggggttgcggttgggttatcggatacgggtggaagtcggtcggtttgggtggtcgtttgtaaagttaaacgattcggttgggtttggcgcgcggataggtttgtggtgggtttagggtaaagaagaggtagagcgaaagaagggggaatttttaaaattatttttttcgggttttcggagtttaatatgttaagtttttggagttaacgagttgacgaagaggtggttttttgttttttatttggttgttttgttaggcgagaaagagtgttggcggtttagtttttgttaagggagtacgtattagggggtgggggacgatagtggaggttagggaaggaagggaggaattgcgtgggagaaagagcgattttttagtgtttttttagttttttttttttattcgtgggtttgtggttttggaatggaagtaagtttgtaaggtgtttcgggaagggttggaaaagtttgttgtttcgcgtttgttttatattaagtgtttttggatttggagaaacgtttggttgagtgattaaatcgttcgtaggtttttatgcgttcggttgaggtttgtggcgtagtttcgagttttagttcgtaggttagagtagattaggttttttgcgtttggtggagattcgggttagtaattgaaagttggttttggtattttggtgtgtagggcggtgtagtgaagcgaggttagggtgtgtgagtgcgttagcgtgtgtgtcgggggaaggcgggggttggttttcgatggaagttttagtaatttgtattgtggtatttgtttgtttttttgttttaatcgtttttaggtttggtttaagaatcgtcgggttaaatggagaaagagggagcgtaattagtaggtcgagttatgtaagaatggtttcgggtcgtagtttaatgggtttatgtagttttacgacgatatgtatttaggttatttttataataattgggtcgttaagggttttatattcgtttttttatttattaagagtttttttttttttaattttatgaacgttaattttttgttattatagagtatgttttttttatttaattttatttcgtttatgagtatgtcgtttagtatggtgtttttagtagtgataggcgtttcgggttttagttttaatagtttgaataatttgaataatttgagtagttcgtcgttgaatttcgcggtgtcgacgtttgtttgtttttacgcgtcgtcgattttttcgtatgtttatagggatacgtgtaattcgagtttggttagtttgagattgaaagtaaagtagtattttagtttcggttacgttagcgtgtagaattcggtttttaatttgagtgtttgttagtatgtagtggatcggttcgtgtgagtcgtatttatagcgtcgggattttaggattttgtcggatggggtaatttcgtttttgaaagattgggaattatgttagaaggtcgtgggtattaaagaaagggagagaaagagaagttatatagagaaaaggaaattattgaattaaagagagagtttttttgattttaaagggatgtttttagtgtttgatattttttattataagtatttttaatagttgtaaggatatatatataaataaatgtttgattggatatgatattttaatattattataagtttgttattttttaagtttagtattgttaatatttaaatgattgaaaggatgtatatatatcgaaatgttaaattaattttataaaagtagttgttagtaatattataatagtgtttttaaaggttaggttttaaaataaagtatgttatatagaagcgattaggatttttcgtttgcgagtaagggagtgtatatattaaatgttatattgtatgtttttaatatattattattattataaaaaatgtgtgaatattagttttagaatagtttttttggtggatgtaatgatgtttttgaaattgttatgtataatttattttgtgtataatatttcgtataatattattgttttattttttagtaaatatgaaataaatgtgttttattttatgggagtaaaatatattgtatataaattggtttggattttttttttttttttttgttattaatttggttaggatattttagttattgttttttaaataaattagttttttttgtttgtttagttaaatatataaggtagtagtttttatttaaatttggtagaaataaatgatagttatttattagaaattaaaaagaaaaaaaaaggtattttcgggggggaaaagggttataaaatttaattttgtttttttaatttttttttggtttaaatttagaggattttattatggttagtaaataatatgaaaaagaaaaaagaagaaagaaatttagtaagtttattagtttaaaatgatttttaagtttatttttttacggggaaatttatatttttagtaaattgttttggagaaatatttgtgtatgtatatatgtatagtttatatgtattttttttaggaggaatatatttataataaatttatagggaaatatttttagtttaaaatatttaggtttttacgtttatttttaggtttaagtagagagattttttatgttatattgtattattatttttaaattttttggagatattaaaagaaataaagatgatttttaataattatagttttttagttttttaaagaatttaggggttgagaggttagagtggagttttttgagttttgtcgagtaatatgtagttgaggtaaaggttatgttttcggtgttttgttttaaataatattgatttattaattttaaatttgtttgtttttgaaattatataggattatagtttgtaaattgtaggataatgaagtaaattaagatgaattatagttttggttttttttgttattttttgatatttaaatagggaatgagttcggtgtgagtgtttaaatgaattttaagtattcgatttttttttattcgcgatttttagttttaaaaaaatgtgaaatttgattttataataaatagaaataaatattatttagttttagagaatttatttttatggcgttaggagggtcgttgtggaggtggggggagggatgtgttgagattttttgttatgtttgttaatttttcgtataattaaagtgggcgagaataaatattacgttggggaatttagagtaaaaagtaatcgtcgattttttggagtcgataatattattgttttttcgttttagt

SEQ ID NO: 5 - DNA, 12001 bp, Homo sapiens
tatggattgcgtgattattaaatttggtattttagggggtatattttttttgagtaatttttataaatatgtttgtttgtaggatatttagattttttggtttggtagtaaagtaatataagaataattttgaatttgatgtttatttttgttttttttttaattttaggagttttttgaggtttggattaatttattgattaggaaatagtatttggaaaggttaaataaaatattatttttagggaaatagtatttggaaaggttaaataaaatatatttttttagtttttttaaattttttagaagatatattttttaaaaaataaattaagttagtaatatttaaattaaatttttgttttgtttataatataaaagatgataaaaaaattgttgggaaggtgagaaattaattttatttataattagaagtaaagtttttatttaaaaatgtaatattatttaaatttaatttgggaaataaaaaggatttaaaaaatagtttgttaaagttaatttgtaaataagtgcgttttttttttttttaagttgtattttaggtttagagtatatgtgtaggtttgttatgtaggtaaatttgttatagggatttgttgtatagattattttgttatttaggtattaagtttcgtatttaatagttattttttttgattttttttttttttttattcgttattttttaataggttttagtgtttgttgtttttttttttgtatttatgagttttttttatttagtttttatttataagtgagaatatgcgttatttggttttttggttttgatttagtttgttaaggataatggtttttagttttatttatatttttgtaaaaggtatgattttattttttttttaattattttattttttttattatttttttttttttttttaattttgaattttattatgttagtttaattatttttttttttttttttttttttgtttatttgtatatagttaaaagatgttatgaatttttttttttaatttagtatatgtttattaaagatttaaaaatattatttatattatttagaatttagtttaagaaattattaaaaaataaagttattagaaagtaattgaattattttgttgagttataattttagatttcgattttgttttttttttattttaggtaggttattttttttttttttttaaattgttttttttgtatttaataatatatttttgtggatttagaaagggtggagtatgaggaaaaggaatatgatatatgtattttagaggaaaataataaataaatattttaggatggaaaatattatttttatttttattgagttttttagagtttatttgatttgtgtaaattagaaattagtagaatgatattaatgaattaatgaaaagtagaatgagttattagttgtaataaaaagaataaagaattttaagaatatagttttaattatgtatggttgcggggagagaaaaataataaaatgtttttagtgaatatatttttgagagaagaaaggaaatatttaaggagaggataaaaagagtaaatattaaaaataggagtaagaattttattgttttttttagttgataaataaaaattgtatatatttattgtggataatatgatattttgaggattacgattatttttgatttataaattatatttaagaaaaagaaatttttaaaaagtttgggaatatatgaagttgaaagaatattaatatttagataaggatagtatatgataaattatttttgttttaatatttttttttaggaaatttaaatattttttagtgaagtattagttttttgaaattaagtatgagaaaaaaaattaaatttatttgtggaaaaaaagatatagttaaataaaaaagcggttgttataattttaagagtggtatgaataaaatgattaatatttttttaagtgatagtataaatattaaaagttttaataagtggaagtggttttgttatgataaaaggtgtggtatttgtataatttttagataagaataaagttatgacgttaagatagtagtagtattgtttgttatacgtgatatttgaaaaatatgataattattttaatttgtttaagtagtatttatggtgagggtgaaattttattaatattggttaatttatggtgttttaaaaaattagtaaggagataaattgatggattaaaagataaattatttataggtagataaatagaaggatagatagagttataattaaatatgtattttatttaggtagaaagataataattagtttttaagaagtgatgtgtttgttagaaaagttttgaatatagaattttttgattttgtttttaatttagtttttttaggtattacgttgtataattaggtgtaattttttaaaagtttttatgatagaattttttatttgttaaattaggttaataatatttttatttttttttagggtaaagatgtgaaatatttggagaattttggaaaatatgttttttattaattagagttttttgatgtgatattattttttttagtatttggagtttagttaatagatatatagtgtagttgtgaaattatgaagtatgagaatgtattattaagggatcgtaggaggttttttattgaaaagtgtagttggttatatttttggaagtaatttaaatataggttgagggagaggagtattttttagattttttttagattttattttttatgaattttaattttttttttttatttagaaaaaataatgagatttatagcgtagagatagaaaataaggttttgtgtgtttttaaattttatttttaaaaatattatagtattttggacgagatagttttgaatttttgtaatagtataggtatgagagtttttattagaaaataggagattggattgatttttttattttttttttatgttttttaaaattgaaaagttatatatataaattatatttatttattttttttggaaaaggttaaaatgaatttaattttggattatttttaataatgggataaatttgaattgagaataatttttagaattagttttgtttttttgtgataaaatggatttgtagaaagttatttggtgtttttttttagttaatattttattataaataacgggtatgtaatttagtattgttttttataggttatgtttttggaattattatttttgtattttatttgtttgttgatatttttttatttaagatgttttttttagtataagaagttattttttttaaaattttaaatgattttattataataatagagttgttaattagatttaggtaagtaatgataataaaaatttgatttttatttagagtgtagtatggtttaatataataattagagttttaataggtttttttagattttatttttatttaatttgtatgtttttgtaatatagatgtttttattattcggtttttatttttatttttttttgtttttggaataaaattatttaaatttaatttagagattttatttttttttggaattattgggaaatagttttagtaaattatatttttgagattttatattaggtttagtttaaattgattatttaagtattaatttttttgtggtttaggaatatttttgagtttatttttttttttttaaattgtttaggataaatatcggagtttggtttttttgtttttttatttaattatttttcgtttttttttttttagtatttaaaatatttttgattttttttattttttaagaaatatatttgtttttttgtttttgtattatttttttgtttatgaaatattttataggtaagttttatattttttttttttagaggtttttggttttttggttttagttgttattggtttagtgtattagttaatattttggattttggagttatataaatttagatttaaatttttattatgttatttattgtttacgtgatttgaagtaatattttatttattgtggtttttagtagttataagtttgtgttttaattagttgggtgattttgggttagtgatataattatggtaaattttattgtttttatttgtaaaatgatagtatttattttgtagtgttggtataaggaataagtgtgattgttaatataaaagtgtttagtataatagttaaattaattaagtattttgtaaatattagtttttattattattattaatttaaatgattagatgtattttgtgtatattaggttttttgagtttattttgtttttaataaatattattatttttagtatgtggtttatattatattttattagttagaggatatgtgaagtttagagtggaaagttagggtagtaggaagtattgttatattttatatagttaaagttatttaaatatgtttgaatttgagttttgttgagtttttatttgtttttattttttttgtgtgttttagtttattaataaagtaggtttaatataaatatattaaaagtttaaatattgagattatgataatgaatatgagggttatgattataaaatattattgaattagagatttgttacgaaattatatggtgaagattataagggaggaatttgtatatatatcgagtgttttgggattttaaagtgggaagagttagtgttttaattaaagagaaattcggggtagggaattaattataatattagttattttattgaatttaggtttgttttagttgacgtagttgttaatttttaatgttttttttttttttaattgtttttaatttatttttttagaaattgaaagtttattaaagaggatatttttttagagagttgttttagttattataagtttttgttagaaattttaagaaagtttataaggtatttttataaggtggtattgagtaagttagaagtattttaagtattaattattatgtaaataagggttttatttttagattttgttgtttgtggtggtggtgatgttggtgttttttttggaatttagtttaatttttaaaaaagtaaaaggagtataaatagtaatataaattattattatttatattaattaaaatagaagttttgaatgagtaaggagttagaggaggtaaaaattgggaatttcgtatattaaaaggtttttataatttgaaaattaagattatgttggttaaataggttgttttaaaattagtatagtaattaaatttgtttgtaatgaatgtagatttaaatagtgatgttagatttgataaggatttgtaaattttaaaagagtgtaaaaagattatagaagaataatattatatttttgtatttatagaaatggttagtttaagagatgtatttagtttagggtggttgtaagttttattttttgaatttgttattagaagttaaaagaaattttgtataattgtttttgatggaaatataaattggttgatgtaaatgaaatatataaagtagttggtgttttatttatttttataattataaatgaaattaaatgattaaaaattatagattttggggattttttttttattgaggagtttatggaatttgttttttttagtattaataattgtgttgatttatttttttttgtttaattttgtatatattaaaattaggtggttacgaataaaatttagaaatataatttatattttaataaaatgattttaaaattattttattttttattgtggttttatttgttgttttataatgtaggtttttttgggtttttgtttagaatgattttgttaatgtagatgatagttagagttgaatggggaatttagaaattggggattcgggtttttgatgtaatttatatgttaatttattttattagttttttttttatttatagtttggtaaagaatatgggtggagttgttttgggtttatttgtatatatgtttaaattgttttgaaaaaggaagggtaagaaagagtggtatttaagttggaattaggtaggtattttagattaagagacgaattggaaagggaatatttgttagatattttgggtttgaaggtagtttgtgtaagtttttatatttttgagtgtgtgtatatagtggagagggtggagtttgttatttttaaatttgaaaagattgagagattttagagggtttagatgtgttaaaggttagagggattaatatataggttttattacggaaaggcggggaaaaggttcgaatagaaaattgttgtagaagggaagttattgagaggtaagggagtttttgaataattaaaaagttaagaataagtaaaaggaaggaggtcgggtgggggataaaaaaaagtagttgatgtggtaattaagaatttggtgggagtttgggtaggttatttttttttttagattagagttttattagaaatttttttaagtgtttttttgcgtcgttaaagatgataatagtaaattaataagtgtttgaaatgaaaggggatgttgattagtttttaggttatagatttttcgtcgttagttttttttgaatttttatagcgtgtttttgtatcgttttttttaagaagagttattttttatttttatttttaggacgaaggtaagtgtttagttagtatatttattaaatgttagttttggttttagtttttcgtttgcgcggaaagtttattgttatagcgcgtttagtttgtcggaggggtagatagaaaaagtaagtttggtttggcgatttgcggggttacgtatttttagggttggttcggagttttttagagtttaacgtttttgggttagaattgtaaggtttcggttcgagtaaagggtttgagttatcgtagtcgtgggagcgttttttttatttgaatgtatttatttataaataagtataaaatttttttaatagtagaggagaaagatttttgttttaaaattaaagttgggaattatcggaaatttcgttttgagtgcgagatattggtttgttatttttttaatttttatattttttttgtaatatgttttgatttaataatttttttagcgtttagtattgttcggacgttttaattgggtaatttattagtgagttaatataggtatttatatatttttttagtttaagtggttaagtattaatttcgaaatgattataaaatatcggaatcggtaacgtatagtaattttaatttatatgtaaattaattggtttattttaaatgttttttttaaaaaaataattattgtattgtagtatcggaggtatggattaaatttttagaatagataattcggaaataagatttggattaggaagataatttagaatagttaataaattaataatgtttgaggtagttaaatatcgttagttattggtatttatatattcgtttgttgttagataaggagttggggaaattgtttgttagggttgagattataatttagagtgaagaaagtaaatggtagtatatagttcgttatagcgggttttgaaataatattgtattttttttaaattttgatttttgggtgatagggagttggcggaggttattttatatttgtttacggttttgttttaatttgattacgaaattgttgttttttttgagttttttaatttgattattattttaacggttttgttatttgttttaatatattggggggaggagtgtaattgagatttttattaaaaattatttgaatttatttagttagtattgttttatttaagtttagttttatgggttgtatttaattttttgtgttttttatatattaaaattagattattaaaatgtcggtaggaaagggtgaaggaaatggtttaatgttttagtttattggaagattattatttttagatatagtttaaaattttgaggaaataaaaaggatatacgttttggggggaaaatgttttaatattttagaatgggggtattattttttttattttagagaattcgtattggagttgtttatgtaaaaatgtaatatttttgaaatttatagatacgtaaggttagtgtttttttttttttaggtttttagtttaggcgatttagttttaaaggagttagtatttttgatgttataattttgtttatatttgtagggtagagaattgtttgttttgtttggacgttttttttatttttttttaatttgaagtaatcggaatttaaatatagtcgttaaggttcgttttttttttattgttttgataagggaaaaatttgaaatttacgttttaaattagttcggtggtttgtagttttttagtattttgtttttacgattgtatgtttaatgtattttttggtgattttgggtattaattagttgtttaataggagtatgattaaaaatgtaaaagaaggattaggagcgtgaaacgtatgtttagttttttttatatattcgaggagggaatgagaattattttgtattttttatttttttaggagttatttgtattttttattagttgtttattttagttgtattggcgttgggtaaggcgaggatttaaaagtttagcgtagtgtttgcggcggtcgggattggggttaattagtttttggcgggcgagattttagatagaaggggggcgagaggaacgtgagtttttcgagttttttttttttagttttggtttgtaaatttttgaaatttgaaaggggagggagttgtacgcgcgtatttttgcgtttttttagcgtaatttttttttttttttttgtgttttttcgcggatttttgaatttttttgtttttggtttttttatttttttttaatttttttatgagattgtttattttcgttattagttgaaggtaaggtcgttttgttacgagcgttttttaatttttataaaatgaaaagaaaaaaagggaggattattagtttattatttagaggaatggggaggttgtaaaaatcgtcgatgggtagaggtgaagatgtttttttcggattgtatttttcggtgttttgtaattagagtttagttgtgggatttgttgaagaaatttgatttttttgtttcggcgagattttaaaaattagaaatagaaatttttagagttagagaggaaatataattaaatagtacgtgggtatttttttttttatttttttttttttaaataatattgttttgagtttttattgggtaaagagagaaagtttgagtttttacggatgttacgtggaggttagaaatggtttaaaatgtagatttttaattagtttttttcgtggttgaagaggttaattttttttataaaatgagtttatttgtcgattgttagttattttaaagtgaagggatttagtatttaaaataaattgagtaagtttgtttgtttgtttttattgttaatttaaatgaatttaaaatacggagtaatttaagaaaatatataatatgttttagatagtttttaaaagtagggaaagtttagtatttatatagtgattagggttagttttaagcgttaagtttttttaaacgtatttattttatgtatattttttcgagttattatatatttttaaaattgcgagtattggtatattgatttaggaagagtaatataatttttagagggaattttatttttaattagggattaaagagatgtttttttaatagcgggtttgagttttgtttttaagtaggaattaatattggtgggaaaattcgaatttaggagtaatggttgtgtttcggtattttttaaaaatatatattaataggatgtttttgagattgaaaaaatattgttttatatgtttggtagaagtttttatatttggttttttaggcgaattatatttatagtttttttatttagaggtaggatagagttaaaatattttgtttattattaaaatatatatttttgtttaagttaagaaattagaaaattagggtttagaagtaaggtatatttttcgagtgagaatatgttttgtaattttatatattttttgttttgtaggagtaaatgtggatttgagggaaatttttttttttatttttatttttatttcgtgtaatttaatattattttcgttaggaattttaatttcgttattttaaaaaatgagatattcgtgatttagggtgaatttgttgaatgtaggtatagtagaggaaattttagattttatgagcgtttgagttttgtttagtgtaaatttttcgtgaatattgggttagtgcgtggtcgtgtttatttgtgcgtcgatatttttagtatgtttggtttattcgttttgatttcgggcgcggtgttttagttaagttgggtttagcgtttcggttttttttagttgataagtttagttcgttcgttttcggttgtggtttttttatttttttttattagtttattttatttttttagatttttttttatttatttttttttatttttatcgcgtttatttttattttcgttttttatcggttttttattttttttttttcgtagtttttttttgttgtgatttttttttttaattttgtaggtttgaaagaaggttatatacgtacgtttatatttatattttatacgtttcgttttaaataattttatgaatattgttttttgtttcgttttttgggttattttttttgtcgtttttttttagttcgttttgatttgttttttaaaagtacgtttttgttttttcgttgttttggcgttttttttttgatttattagggttgtcgggttggcgtagattgttttttttttttttttattttatttttttttttggtttttttttttatagtgggagttcgtgtttttgtttttcggttggtttttaagtgtttcgttaggtttttttttttttcgttttttcggtttcggttttcgatttttcggttcgttggtatttgttttttttttttgtttcgtttttcgtcgtttttgttcgtttttttcggcgttcgttcgggcgttgtgttcgtttttggatcgttagtcgcgtagtcgggttcggtcggtcgttcgcgcgttattgtgtagtggagtttggtggaatttttgttgacgttacgttattttttatacggagtaggagtagagggaagagagagggatgagagggagggagaggagagagagtgcgagatcgagcgagaaagttggagaggagtagaaagaaattgttagtggcggttagatttcggaggttttagtgtattcgtggattttttcggaatttggtatttttaggagttttgtagtttttttaggttcggttttcgggcgtttgtcgtgtagtcggaggttcggttcgttggaaatcgtttcgggaagtagtgggacgcggagatagtagttttttttcggtagtcggtaagtggaggttatttatttcgtagggatgtgagataatgcgagtttggaaatttgttttatttcggagaatttttatcgtaggtgatttgtggtttttggggttaagtttcgtttaaggtaacgtagtcggtaaatagattttgtaaagttttgtttttttcgtttttcgttatagatattaataatttatagggtgttgaagtcgagagggaagttagatcgtggttggtatttaaaacgaggtatttttttttaaatttcggtgttaatattgtaggaataaattttcgggttaaggattagtatttttaagataaagggttgggtataaagttttagttattggaagattagttttttttttattgttatttattgggaaaaaaaagaaaagaaaaagattttattttaattggtagttagtgattttttaggtttaagcgaattatttgggagttaggtttggatgttaagtttttattatttttttggattgtaatttttttaaattgattattagttaattttaatttggtat

SEQ ID NO: 6 - DNA, 4001 bp, Homo sapiens
ttttcgtttttagtttatatatattttttttgtttgtttggattttaatggtttaagatagttttgagtttattgggaaaagaaaatgattgttaaaaattatttttgaaattggttatttggtaatatttttaattgtatggaaatttattaaggtatattttatatataattagtttaaggttgttgattttataggttttatggatttaaatttgattgataataaagtaaataagagagtcgaatttaaagcgtggttttttcgggttaggacgagtttaatatagtgtataaggaatttgaaagatttaggatatgtgttttaattaacgttaagtagaatggataagtttttagtattttgaaaacgttgggttagggttttttttttattgtgtgttttttgtttggggattaataagtattatagagaacgtgatttgaggcgattttttatttttgtataaatttagagtgaattattaaatagttgttcgtttaaagttaaggtaatttttttttgacgggtttatttgtttttcgatttttaatttattagtttgtttttttagggttttgttttttttgtaattaaagtttttttagattagcgtagtatttatttgataggttgtttggaaaatttaagatcggagaggtgatttgttgttgttttttaaattttttagttttaagtaacgtgttttttttttatatggggtgggggattggaaatggatgtagtgagatataaagagtgggtgttttgttgatttttgtatttttttttttttgattattttattttttttttttaagttttcgatttttagttttatttttttatttttgggttcgtattaaaagtcggatcgttttgggttgggtaggagttgaattttcgggagtttgtttgtgtagatttagtgcgtacggcgaggtagtagttcggtttcgtattgttgataggtgtaggtaggatagtttttttatcgcggttcggggcgttttgattggtgcggagttacgttagtcgtattcggagaagggtttgggaggaggcggaggcggagagggttggggagggtcgcggcggagtgacgtttcggtattaggaagttcgtttttggttttaagatgttaggttaatagggaagcgcggagtcgtagatttggttcgtcgttcgtttgggtgtttggagttgagttgcggtaaggttcggtttttgttcgatcgttcgaggggtgtgcgtgtgcgcgttgcggagggtgcgtttagagggtcgcgtcgtggttgtagcggttgttgtcgtcgtaggggatttaatattatttatttgtttttgttatttttgatatttttttgttagggttgtcgcgtggggggggggcgggtagagcgcggtcggcgttagttttttttattggaggggtttttgggggagggagggagagaagaagggggtttttgtttatttttgtttcgttttggagtttggaagtttgttttttaaagacgttttgagtggtgtttttttgtttatattttatgttttcgtttgttcgttgatttttcgttttcggattttttcgtttgagtttttcggaggagacgggggtagtttggtttgagaattcggcgggggttgcgttttttggtttttttcgtagcggggaaatttcgcgtttagagcgcgattcggagcgggtagcggcggttacgggggttcggcggggtagtagttaaggattagtagagcgtcgcgttttttcgtttatgaattgtatgaaaggttcgttttatttggagtatcgagtagcggggattaagttgtcggtcgtttttttatttttttgttattatttttagtcgttagttatggtttcggttttggttttcggttagtttcggtcgttggatttttttaagtataggttggaggtgtatattattttcgatatttttagttcggaggtcgtaggtaaggcgtcgcgtcgttttgtagatattttcgtttagttgttttgcgttattcgttttttttcgttttaaggaagttagttttttcggggggaggcgtggtgggagtggtcgttcgtttggtttttcgtagaattttcgggagtcggaattttgattatttcgtatttttttagttttttttcgatcggttcggtttttggggcgttaagggcgcgagtaattttgtcgttttttttattcgtattttggttttttttttgttttttgggttataaaaattttagtattttgattcgaggatttttagaggtcgtcgatttttgtttttgtttttttttcggtttttagttttcgaggagttttattcgttaggaaattgtttgaaattatttagaaatgtttttcgcgaagaggtattttttttttttttttgggaaagggtcggcgaatttcggtgtttaatcgaatttttatatttttttttagtttttttaaatcgtatggaaatttgagttttttgcgagggggaggggggtttgtaaattacgcgcgtgtgcgcgttttaggagatttggtgtgtttgcgtagaggtgtataaatatatttgaaagtataggttataaaagtgaatgtgtcgttgtagtgagataaatatgtaaataaaacgtgcggcgttgggggaggggaggaaatggggcgcggatatttatatttgcgtttgtatattttataggcgtagcgtttttcgcggttcggagtcgtcgcgcgtattttttttcggcgttaggtagtttagtttttttacggtttttgtcgtcggtttagttggcgttcgcgttgtaggtgggtatgttgacgggaaagtgtgtgtgtttcgtttttagagaaagataaaagttagtaggggaagaatgaggacgtgggcgtcgaggattcgtttaagaagaagcggtaaaggcggtagcggatttattttattagttagtagttttaggagttggaggttattttttagaggaatcgttattcggatatgtttatacgcgaagaaatcgttgtgtggattaattttacggaagttcgagttcgggtaggagttagtacggagtttgggagggatggggggaggatgttgtggaggtataggttaagtagattaggagagaatgtggaaggtagcgtcgtttgggagggcgtcggtggggcgtagttttgtaaaggtagaaggtttcgcggcggtttggttgcgagattatagtttttttttcgaggtcgataggattgtcgttttggtttaggtttttagagcggtatcggtttattgtttcgttatttcgcgattttacgagttgggttgtatgggtaattttttgtataggatattgtgtttttggtttgtagttgttagagtagagttaataaaatttttattaggttaagagtcgcgaataggttttaatttgtgagtttttaataaggaaaattcgttagagatacggaagagttggttttttttgggaaatttttgtttcggttttggtttagtttttttttttttgggttcgcgttttttatattttttttacggttgtttcggttatttaggttttttttatatattttattttttagttttgtgattttcgggagtaaagttttaatatataattattagtttttttagaaggagaaagaaaaaaagaagaaagatttttttgtttggtttatttatttttttttaggagttgaattttggaaattgaaatttatatttttttttttaaattataattatagttttgtaaaaagggtttattttaattttgtagtaaatttgtattttatggattggtaaaaatgagtttaaataaataatttaatagtaacgttttggtttatgttggtcggtggaagattttaaatttgttaggattttggaagtagaaaatagaattaagtaaattaagcggtatttagaggttttgttgttaaaaaaaaaaaattaagtgttttg

SEQ ID NO: 7 - DNA, 32001 bp, Homo sapiens
attaaggcgaaaaaataatgatattgtcggttttagaaaatcggcggttattttttgttttaagttttttagcgtggtgtttgttttcgtttattttggttgtgcggggggttgataagtataataaaagattttagtatatttttttttttatttttataacgatttttttagcgttatgaggatgaattttttgggattaagtggtatttgtttttatttgttatgaaattaaattttatatttttttaaagttgaaaatcgcggataaagaaggatcgggtgtttaaagtttatttaaatatttatatcgaatttattttttgtttagatgttagaggatggtagggagggttagggttgtaatttattttgatttgttttattgttttgtagtttgtaaattataattttgtataattttaggaataagtaggtttagaattaatgggttaatattatttaaaataaaatatcgggagtatgatttttgttttaattatatattgttcgataagatttaggaaattttattttaattttttaatttttgagttttttgagaaattgaagggttgtagttattagaaattatttttgttttttttaatgtttttaaaggatttggaaatagtaatgtaatataatatgaaggatttttttatttaagtttgaagataaacgtggaagtttaaatattttgaattggagatgtttttttgtaaatttattatagatgtattttttttgagagaaatgtatataaattatatatgtatatatgtataaatatttttttagaataatttgttagaggtgtaggttttttcgtaaaggagtaaatttgagagttattttaagttgatggatttgttaaattttttttttttttttttttttttatattatttgttagttataatggaattttttaggtttaagttaaagaaaaattggagagataaaattagattttgtagtttttttttttttcgggaatgtttttttttttttttttagtttttgatgaatggttattatttatttttattaaatttaaataaggattgttgttttgtatgtttaattaggtaggtagagggaattggtttgtttaggaagtagtgattgagatgttttggttaagttagtgatagaggaggggagaaagaatttagattaatttgtatgtagtatattttatttttatgaaataaaatatatttgttttatatttgttgaaaagtaaaataataatattgtacgaaatgttatatatagggtaggttgtatatagtagttttagaaatattattgtatttattagagaaattattttaaaattgatatttatatattttttataataataataatatgttagaaatatatagtgtggtatttagtatatatatttttttgttcgtaagcgaaaaattttaatcgtttttgtataatatgttttattttaaagtttaatttttaaaaatattgttgtgatattattaataattgtttttataaaattaatttgatatttcgatatatatatatttttttagttatttaaatgttaataatgttaaatttaaaaaataataagtttatagtaatgttaaaatgttatatttagttaaatatttgtttgtgtatgtgtttttgtaattgttagaaatatttgtagtgaaagatgttagatattgaggatatttttttgaaattaaaggagttttttttttgatttagtggtttttttttttttatatagtttttttttttttttttttttttagtgtttacgattttttagtataatttttagttttttaagggcggagttgttttattcggtaaggttttaggatttcggcgttgtgggtgcggtttatacgggtcggtttattgtatattggtaagtatttaggttggaggtcgggttttgtacgttggcgtagtcgaagttggagtgttgttttgtttttagttttaggttggttaggttcgagttatacgtgtttttataaatatacggaggagtcggcggcgcgtaaggataggtaggcgtcggtatcgcggaatttagcgacgggttatttaggttgtttaagttatttaggttgttgagattggagttcgggacgtttgttattgttgagggtattatgttggacgatatgtttatggacgagatagagttgggtggggaaaatatgttttgtgatgatagggggttgacgtttatagagttgaagaaggggaagtttttggtggatagggaggcggatgtaaggtttttggcggtttagttgttgtaggaatagtttgggtatatgtcgtcgtagggttgtatgagtttattgaattgcggttcgaagttatttttgtatagttcggtttgttggttgcgttttttttttttttatttggttcgacgatttttgaattaaatttgggggcggttggggtaagggagtaaatagatgttatagtgtagattattaaaatttttatcggaggttaattttcgttttttttcgatatatacgttagcgtatttatatattttggtttcgttttattgtatcgttttgtatattaagatattagggttagtttttagttattggttcgggtttttattaagcgtaggagatttggtttgttttggtttgcgagttgggattcggagttacgttataaattttagtcgaacgtatggagatttgcggacggtttgattatttagttaggcgtttttttaggtttaaaaatatttaatgtaaaataaacgcggggtagtaggtttttttaatttttttcggggtattttgtaaatttgtttttattttaaagttatagatttacggatgaggagaaggggttggaagggtattagaggatcgtttttttttttacgtaattttttttttttttttttgatttttattgtcgttttttattttttggtacgtgtttttttaatagggattaggtcgttaatattttttttcgtttagtaaaataattaaataaagagtaaaagattattttttcgttagttcgttaattttaggagtttggtatattaaatttcgggaattcggaaagggtagttttggagatttttttttttttcgttttgttttttttttattttaagtttattataggtttgttcgcgcgttaggtttagtcgggtcgtttggttttgtaggcggttatttaggtcggtcggtttttattcgtgttcggtggtttagtcgtaatttcgattttaatttatatcgggtttttttgtcgttttagacggcggtttttgtgtattggagagaggtttggtttgagatattcgagttgatattagtgatgttttatattatatattttcgtcgggtttagtcgtgtaattcgttttttttttttttttttttatttttgattttttttttatttttttttttttttgtattcgattgttataaaaagtacgttttatttttatttggttcgataagtagtcgttttggaaggagaggtagttgtaaggagagtttagcgtcgcggttataaagtattagggtggagttgcggaatagcgggcggggtgggagggcgttttcgaaggattttagaaaatttatagattttgtttttaattatttgttatttttattttaggttatttaaattttgtttaggcgagaagagtacgtgagaggttcgtttttttgatgtgtaagagagttaatgaaagattgattttgtttaaaattacgtcgtttaggatttagttttggttttggatagttaaattaaaattatttttaattttttttcggttttttatttattagtatagttttatgttttgtataaatgttatttagagagtgtttttattttttttgatttgggagagtattttggtttttattttttttatcgttgtttttttttttttgtttgttttgttttaatcgggggttttattttttttatttagagtatttaattttttttttttaatagtaaagtttttggatgtcgtttgatttgtttgattttgttttttgtttttagaattttaataaatttggaattttttatcgattagtataaattaggacgttgttattgggttatttatttgagtttatttttgttaatttataaagtatagatttgttataaagttaaggtaagttttttttataaaattatgattataatttagaagagggggtgtgagttttaatttttagagtttaatttttgagagaagataaataaattaagtagaaaagttttttttttttttttttttttttttttaagaggattagtagttgtgtattaaaattttgttttcggagattataaaattaggaaatagggtgtgtgggagagatttgaatggtcgaaataatcgtaaagaaggtgtaagaagcgcgagtttaggagggaaaaagttgggttagggtcgggataaaggttttttagggagggttaattttttcgtgtttttggcgggttttttttgttaaaggtttataggttggagtttgttcgcggtttttggtttggtagggattttattagttttgttttggtaattgtaagttaggaatataatgttttgtgtaggggattgtttatgtagtttagttcgtgagatcgcgggatggcggggtagtgagtcggtgtcgttttgggagtttgagttagggcggtagttttgtcggtttcggagagggaattgtaatttcgtaattaggtcgtcgcgaggttttttgtttttgtaaagttgcgttttatcggcgtttttttaggcggcgttgttttttatatttttttttggtttatttggtttgtatttttataatattttttttttattttttttagatttcgtgttggtttttattcggattcgggttttcgtaaggttggtttatatagcgattttttcgcgtgtggatatgttcgggtagcggtttttttggaaagtggtttttagtttttggagttgttggttggtaaagtgagttcgttgtcgtttttgtcgtttttttttagacgggttttcggcgtttacgtttttattttttttttgttggtttttatttttttttgaaaacgaaatatatatattttttcgttagtatgtttatttgtaacgcggacgttaattggatcggcggtagaagtcgtggaagagttgggttgtttggcgtcggaggagggtgcgcgcggcggtttcgggtcgcgaggagcgttgcgtttgtggggtgtgtaggcgtaagtgtgggtgttcgcgttttattttttttttttttttagcgtcgtacgttttatttatatgtttattttattgtagcggtatatttatttttatagtttgtgtttttaagtatatttatatatttttgcgtagatatattaaattttttgggacgcgtatacgcgcgtggtttatagatttttttttttttcgtagaaagtttagatttttatgcggtttgggaaggttaggaaaagatgtggggattcggttgggtatcgaagttcgtcggtttttttttaaaaaaaaaaaaaaaatgttttttcgcgaagggtatttttgagtggttttaggtaattttttaacgagtggagtttttcgggagttgaaagtcgagaggaaaatagggatagaggtcggcggtttttgaaggttttcgaattaagatgttgggatttttgtgatttaggaaatagaagggaggttagggtacgaatagagagggcggtagaattgttcgcgtttttagcgttttaggagtcgggtcggtcgagggagaattaaagggatgcggggtagttaaaatttcggttttcggaagttttgcggggagttaggcgaacgattatttttattacgttttttttcggaggggttgatttttttggggcgagagggagcgggtggcgtagagtagttgagcgggaatgtttgtagggcggcgcggcgttttatttgcggttttcgggttggaggtgtcggagatggtgtgtatttttagtttgtgtttggaggagtttagcgatcggggttgatcgggagttagaatcgaagttatggttaacggttggggatggtgataggaagatgaggagacggtcgatagtttggttttcgttgttcggtgttttaagtgaagcgggttttttatgtagtttatggacgagggagcgcgacgttttattagtttttggttattgtttcgtcgagttttcgtagtcgtcgttgttcgtttcgggtcgcgttttaggcgcggagttttttcgttgcggggagagttaggggacgtaattttcgtcgagtttttaagttaagttgttttcgtttttttcggaaggtttaagcgaaaaagttcggagacggaaagttagcgggtaaacgaagatatgggatgtgggtagaagggtattatttagagcgtttttagggagtaggtttttaagttttaaagcgaaataagagtgggtaaagatttttttttttttttttttttttttttaagaatttttttaataaggaaagttaacgtcgatcgcgttttgttcgttttttttttacgcggtagttttgatagagaagtgttaagagtgatagggataggtaggtgatattagattttttgcggcggtagtagtcgttgtagttacgacgcggttttttgagcgtatttttcgtaacgcgtatacgtatatttttcgggcggtcgaataggagtcgggttttgtcgtagtttagttttaggtatttaggcgagcgacggattagatttgcggtttcgcgtttttttgttggtttaatattttaaaattagaggcgggttttttggtgtcgagacgttatttcgtcgcggttttttttagtttttttcgttttcgtttttttttagattttttttcgggtgcgattgacgtggtttcgtattaattaggacgtttcgagtcgcggtggagggattgttttgtttgtatttattagtagtgcggggtcgggttattgtttcgtcgtgcgtattgggtttatataggtaagttttcgggaatttagtttttgtttagtttaaggcgattcggtttttagtacgaatttaaaggtgaagagatgaggttaggagtcgaaggtttgggagaagagagtggaatggttaagaagagaaaggtataaggattaataagatatttattttttgtgttttattatatttatttttaattttttattttatataaaaaggagatacgttatttaaaattagaaaatttgaaaaatagtaataaattattttttcgattttaaattttttaaatagtttgttaagtgaatgttgcgttaatttgaagaagttttaattgtaaagaagatagagttttgaaaaggtaggttaataaattagaaatcgagaagtaaatggattcgttaaaagaaaattattttgattttaaacgaataattgtttggtggtttattttggatttatataagaataaaaagtcgttttagattacgttttttgtgatgtttattagtttttagatagaaaatatataatagaagagaaattttaatttagcgtttttaaaatgttgaaagtttatttattttatttaacgttgattaagatatatattttagattttttaaattttttgtatattgtattaagttcgttttaattcgagagagttacgttttaaattcgatttttttgtttattttattattaattagatttaaatttataaagtttgtagaattaataattttgagttaattatatatgaaatatgttttaatgaatttttatataattaagaatgttgttaaataattaattttaaggataatttttaatagttattttttttttttagtgagtttaaggttgttttgagttattaaagtttaagtaggtagaaggggtgtgtgtgagttaagggcgaaaagtttagaattgcgtttaattagtaaaagtaaaattttatttatataaaataaaaaaaattatttttggagatattaattttttatagtattgtttttaagtaaatttaatttttaaagaaattaaagaaagaaatttaaatatatttaaaataatttttgaaagtttttttgttttttagtataggttagttggagaggataaattaattttttttgggtttttgtatgggcgattgttttattatggagttagtgttattatttttgaatgtgtatttgtttgatattatagttaatgatttgtaatgttagtatgaagtatttttaaaatattttttttttgtttttgtttataagattgggaaatttattcgatgtggaataaagtggatgaagtagattataaatatatttgtaatttatgtgttttttttttgttttgattatttttaaattttatttgtaatttttttttattttaaatttgtagtttaaagacgtatatgagaattgttttttagtttttttttattagtattattttattttaagaataatttagttgtaagggaggaatttttttatagtaagttttaaattagtatttttgtttttaattttttattttattttattttattttatatatatagatatttgtttagagtaaaatatatttttatgtgataggtttgtattagttgaggtttatatatttagttatattaggttttgtaattttattattaaattatatatattatattagtagtttgttggtaaagaaggttaaattaatttatattttgtttattatttggtgtttaaatgacgtattttatttcggagatttggcggagaattttttttttagattttatagcgttttattgaagataatgtttttatatttgtagtggtttttaatttgataagattttaatttgtttaagttttttaaataagggttttaaatgtttttagtcgtttttttattgaattttttttaatttttttaagattataaagtatatgtgtaaagtaaatatttttttttattgtattgttagtcgatgatttataattaagttaataagaatttagtttttttttgttgaatgtgtttattaattatattttagtttttttttttaaattttagaatagttgtggtttttataatattatgttttttaaagttttattttatgaagggattttattatattaaagaatgaaaaaaatttttattgtagttagtatatatagttttttattttttgttttttaagatttaaattttagagttgtaaatatttttggaagtttgggtgttaatgttttattttagaaagtcgagaagttttatagagttatatagatttttaaatttattttttataaatttatagaattttgataaaagttttggtggttttattttatcgatggaatttttattacgataaatatatatgtatgaaggattttaattagtttttaaagtggttgaaaaatttaagggtacgtgattgttttttatagtgttaacgtgtgcgagatgttggaagtattggggattagtagtagtttagatgtttaaaaagataaggtgttttaatttgtgtggatttattgaagttaagtggtgaataaagataattatttagataatttagattaaagtaaaagtaaaattatatttatttgtatatatatatttatatttattttatattatagatatatatacgtatatatatattggttttgtaaataattgatttaaagtgaggattttttttgtatttttttagtaggagttttaatatttttttaattttttaattattttatatatttatagtagcggcgattgggtgatattttttttaggttttttgtgtggtaggatattaatatgataagtttgtatggggaaaaggaggtatgtggtgggaattaagaaatattgtttagtgaaaattttgtggtatggtggtggttgattttggagatttaatgtatataagatttgtgggtgtataggtataggtagtatggatgagaaaggggttagaagaaaataaattttatgtattttgtgattttagtattattgtgatttttggttaagttttttttaattggttttagaaattattatgagtttagtttttaatatagaaatttttaatacggagaatattggtgggattttggtagggaaattagaggtgttgtatggtttacgtggggtaaagaaggaaagtttagtgtcggcgtgaggttttgagtttgggagatattaggggttgtttcgattggggttttttgtttatttttttaaagaaagattttagaggagggaaatgtgtgatatggggttagtcgtgttttgtgttggtatttgttatcgattattagttttaaagttttatttaattttatattttttagtgttagttgtgtaaagtttttttggttatggtagtgagcggttgggttgtgtcgttaaatttttcgtattaatttggtttgggatttaattaagtgatttttgatttttggaaagagtttgtttttagagtttatttagaagatggtttaattagatatttttttgagttgttaggttttagacgggtgggagttttgttttgtttaagttagtttaaggacgaggttcgtttggatttagtttggagttacgtgatgggcgtgagtgtgtgagtttttggtaaggcgtagaggttagatggagattttgtattttgttcgagaagtgttttattttttttaatatttggtttttttttgtatataaattaagttgaaaatagtttattatttattattttttatagttatggaattaaataatttagaaattaaaagttttattgtagttgtttttttttttattttttaaatggaatttaaaaagttttggtttgttaaaaggggaagattattttttgaattggaagtttgtagatatattgagtaatagttattttttttgggtttttgtaaatggtatttatttttttaatttatagttttagttgtttaattatttgagatttggggtaattatttgggggaatagtgtttagatggtagtgggagttattattttatagtggtttggggaagagaagagaaagagattagaggagggggtatttgttaaaattatttaacgaatatgttgttaatgtttttttatatttgtatgttattgttatagtttttttaggtgttattgagtttttagaaagtaattatttgtcgaattaagtaaaataaggagaatggtatagtatatgtgtttggagaaggggaaggaagggtggaatatgaaattgagtatagatatttaggttaggaaagaaggaagtggtaaggggttaaatgaagttttattttttcgttatttttttaaataatagttggattaaatatttatttgtttttttttttttttttttttttttttttttagtttatgtttattttttttttttattttttttgtttttttttttttttgtttttttttttttagatatgttggtagttaatatttagtattagttgttatggtgattataaattatttaaatttaaaaatatttatttataatttgagatgaagtttttatttttttagcgaaataatattttaaaagttgttagttgataaaaaaaaaggaatttattttattgtagtaatttaagtaatatattatttttaaaggtttaaattaaaatgttagtttgttaaaaatatgttggtagagttttggatatttttttcgttagatttttataaagaagttgattttgttatttttggtcgttttttaatatatatatataattttgtatgttttttttttttttattaattttttttttttttattaattattttagtttttaaagattttacgtattgggttttaaaagaaaagaatttttttttggattagaaaatagttttattggttgttgaagtgaaagatgtggggtttagggggaaaggttattaggattataatggcggtggtggtaggaggttattttagaggagttaagaagaaaaaaaaatgtagggagaaggattggaggtggaaagatagagtaatagaaaattgagttgggtggttaggtgttgcggtgaagtttagtttcgaaatgataggtatatatttttttatttttgttttttttttttttgagagaaaatttttttagttagagattttggggggtaggaggcgggtaaacgtcgttgtagttgggttttttgttttttattttgggtttgttgttttttgtttattttggattatagggtattcgtttagatgaagagttattaattatttatttagttaatattaggaagacgataaagttttttatataggattaagaagatattagattgttttattagtatatttttgtttacgaataagttttcgttatatatttttttttttttcgagtcgttttaataattgttgtatatattagtagcgggcggtgaggaataatagtcgaattagttttaagaaattttgtgtatcgagttagtagcgaggaacgcgatttgtgaagattatttttgcgggtagggattcgtagggattgattattttcggataattggtataattttttttgggggtgaaaaattataacgcggcggggtattttttaagtgagttgtagatttgattggcgcggggggtgggggaggggaggggagaatgggatggcggaggtcgggcggaggaaagaaaatggaaaattttttttatttttatttcgttgttttttttttaagttttatgtttttttcggtaagtatttgtttttttcgcgttagttatagttagagttttttatttttttttatatatttttttttttttgataaggtttaggattttggttattattttacgtattattattttgcgttttgttagagacggtttgggttgatttcgttggtgtttatgttaggattaaaatttttttatgacggcgaggaaaattgtattatttgtttttagggggtatattaggagtttacgtagtatatgtttcgtaaatattcgttgattgaatgagaggcgcgggggcggggcggcggagaggggtttgcggtcgttaaggtcgttagggttaatttaggtttttcgaagaaggttgggatcgagttgttgtcgcgtgtgaaggtgtgtgtcgcggttgggggtgttataacgggttatggagtttattttttagagggaggaagtttgtgtatattagcgatttgggtcgaatatttttagtttatttattgggttaaagttatttaataattaatgcgtttttgggggaggtcgggggaagtattcgttttttgtcgggacgtaaagttaggcgttaggtttaaaggggttgtagtgtagttcgattttagtacggaatttagagtcgtcgttttgaaattttttaagttagtgatagaggagggttagttcgttttttttttgagggtgaagattattttatgagttttttttaggatttttaaagtaagaaaagttaaagaaaggtttttttgttttagggggtcgtttttagttggtttttatattattttttgttagttgcgtttatttttttttaaatttttggtttttaggggtttttagtcgttttcgtgttattttcgtttcggggttttatttaggttgggtattcgtttaatggatattaaggagaatgggatttattagggaaggaaggtagagtttggattgtttagaggtggattttgtttatatagaacgtttagtttttaacgaggatatggtatttttgggcggcgttgggggtagaggcggagagggtagcgtaatagattattacggttttttgaagaagttatatgttattgtgaattttttttttttttaaaagtaaagaaaaattttaaaaaaatataagaaataaatttttttgttttataagtaggttgtggttaggattttggatattttataagttaatttaaaattagggaaggataggtgttttattttttagtagtgttatagttttgtttattcgtgtgatttttttttgtcgtttattagttttttaaaagttaattaaattaagatttttagtatttttttttattatatgtttttttttaattaatggtattaaacgtgtttaggtagtaattttttttttcggttaaaaagtagaaaaagatatattgagtgtaggggaagagttttttacgtgtattaaaataatgcgggtttgaaagtaatggttaagaaagtaattatttattatttttagttttttatgtgttagttattaaaagcgaacgattaggggcgtttgcgcggtttgtgattggcgtaagtagaatttttttgtttttagtcgttttttgtttatttacgaggattttattttatcgtaggtttttttatttgtttttagaatgtattttttatgtttaggaaatttggggtagggattgggggaaggagatattttgcgtttttttggtttttagtataataagaaatgttagtttcggtttggcgattgcgagttcgtttcgcgcgaagcgagattggggagtttttttagtttggtcggagttagggttgagttcgcgtaaagtattttttttagaagttatcgttgtttttgatttttaattatattttaaatatattacggtttaataatttatttttattatcgattattaaatagaagaagaatttaatataatttaaatgatagaaattacgcgacgttatttttgtattgtttttatttaattttatggggttaatttcggataagtgagcgtttaattggtttagtagggcgattggcggtgtagtgtagtgttcgggcgtgaagtattggatcgttttagacgttttattttaataaatgattatttttttttagatttacggggaaattttaatgtaagatttttgttttttttttagtaatacggtttgtttttttgatcggggttttaaatcgtttttttttattttatattatatttgtatttttatattttaattcggaaagagggggttaggggtcgagggttgtgggggggggggggttttatttgtttatattattaaaggttaatagttttttaaggttaggtatttatttattacggagttaggaaaatagaggaatagtaaatttgaggggtttttttttatgtatttgaaaagaaaggtatttttttttttttattttttatattttttttttcgttttatagaataagttttaatttaggaaaggtttgtggcgtaggttggagattttttaattttttatataagtttgtagattttttttggtaatgtttttcgatttttttagagtgaaattagttaattaagtaacgatatcgttaaaatttaaggtttggtaattagtattttaggtaggttcgcgtcgataggggtaaatttttattttattttgggttgttaagtatagtggttgttttttagttttttagggatgttgtcggtttttcgttttttttttaattagttaaagtaaattttcgttaatttaagttttttttgtttgtttttcgcgatgaatcgcgtatttataagtttgggtggggcgtggttgagagtttgagtgattgagtgggttttggtggtgttgcgcgtagcgggatataacgagcgatagaggtcgttgttggattatttttttacgttagtttagacgtcgaggtttgttggagcgtgcgtaggggattagattatagggagcgagcgagagggagagagaggtgttgggttttaggagtgtagtataatttggggaaaggaattaacgtttttgggacggttgtttttcgttttatttagaggcggagtgtttaagtttaagtagtaggcgcgttaggtttggcggtttcgtttttttgcgtttcgttcgaggtttagagtttcggaggcgggtgtttagcgcgcggtttgcgtttttttttcggttttattattggcgttaggatgttgtcgcgggaagaatttgttgttggttgttttttttcggtttttaggagagttcgtgaattcgatttttttgatttcggagtttttggagaagagatatttaacggtcgtcggttgtacgtttgggttacgcgcgcgttcgttttacgtgcggagagaggcgtttcggatcgcggtcgaaaggagtcggggacgggaggagggggaggggcgaggtaggtcggaggagaaagagggataaagagtaaagatttagttagaggaaagagttgacggtattttcgtttttcggattttttggtaattcggggtaggatggcgtattttttttgcgttttttcggttgtcggcggttttagtcgggaggagtaggttggggggtttcggtatatagcgcgtcgttgttttttagtttatcgtttcgttatagggagaggttattggcgatttggttttgattttttttttgtttaggttggtttttcggggaagcgtttttcgttggggtttcgtcgtagggttagtgtttttttgtcgtttttacgtggcgcggtttttcgttcgatgattcgggtaggagaagggggtttttatttaattgtatatacgtcgatattagtttgcggtagttggtttttatttttcgttatttgtaaaatagaagagaaggaaggttgtaagaagcggcggtcgtcgagtgagtagggtttagatgagattacgttatattagttgttaggcgtttattgtgtgttaggttttaggcgtgttttttcgatttgatagtttttggttgtgtagtagtatttttagtttagtttcgggtttaggatatttatttattaagaggggatttttttttagagttgtcgtaaaagtgtttagaggttagaggattataaagttatagtgtgttggggaggttgtggatttatttttaagaatttcggtgtcggggttaagaatttatttgaacgtaatggtagcgggagtgggtgggtggagaggatttttttttttgggaagttgtatgtaaagattattttttagtgtttgtttattagttggagttcggtaaatatttgtagaatattagcgttaacgtgtttttgttttagatagtagtttttttcggttttttgtaattttgaaacgaacgggtttttggtttagggtgttttaggagcgagttgagttcgggttttttatttattaggagttatttttttatatttagttatatttttttttagagatattaattcggttatttatttatttattataaataattattttaaagtatgatttaagatcgtagaggagagatattgggtggattgagcgagattgaggagagtagggtaaacgtttttggagggtttattgttcgttaaggacggagaaatagttttggtataattgttatttagttttttttttttttttttcgggcgagttaaattttttttacgtttttaattataacgtagcgagttaagtatttaacgcgtttttttttttttgttataggtaagtcgggagaggtgggtttcgaggggttttatcgggtgggtagaagagtcgcggttgttttaaagataagaaaagaaggtttagggttttttaggttttttcgattttagcgtttgtttttttttacgttaattagggtacgtcgacgatcggagggtttatttcgcgcgggtgcggggatcggggtgggagtaagcgttgtcgggttggcggaggtatagaggcggggtagggagttgcgggtttgtttttggtttgagtatcgtttttttgcgtttcggttttttttgaagggagttgggttttggggagtttttggttaaggtcgttgtttataggaggggttgttcggcgttgtggcgtggggatttagggtggggacggttaggcggtttttttattcgttagcgagaacgcgggcggggattttgtcgattcgatttttgtgggttcgtgggtttagaagtagtagtttggcggttttagatttagtgattttgtagtaaaattataggattagtttttgattgagatgtttgttcgtgagatattataaaatttattattatagttttttattaattcgatatgaagtaatatagatgggattttattagtttagattttaaatgtttatttatgataatttcggaggaaatttgtatgttattattatttcgataattttttttttttatatgtttgaattggttgtattattagttggtagtcggagtattgtagatggtaattgtaaatagtttttatttatttattttttttaaagaatgaaatatataaaagaaaaagattgcgttgtttggtgtaaagttagttaattattatatatttttttttttattttttcgtgttttagtgttgaagattaaataaagtaatataaaataaatttttaagaatttatagagttttattttaaggattgaaaagaaggttaaggcgtgttttttagtttatttttatatgtttttgtgatttggagatttattttgtagttaaaatgagttttgagatttgtatttttatgttttatttaatgattaggtttattagaagaattgagtttaaataattggggaagataattttttaaaaagagatttttaattttcgtttgttgatttttaaatttgttttattaagataagttttttgtgagaaatttggttgttagatttcggaattggttttaatggttaattttataaattgagatgggagattttttttgatgggaggtagtttttatttttaaagtttatgttttagttggaatgtatatgttaaggatttttgttttggttaatttgggttttatattgtgagtatataaaaagtattatacggttaacggaggacgaggaattatggtaaagtaggtaggtaagttttaagaaataaaataatttgttaaaaaataatttttgatgattatcgtaagattgaaagtgtaggaaaaatatagttcgaataattttagatttttttatattttttttttttttatatattttgttattttataataaaatttttaatggaaagtttaaaaataaatagtataggaatatgtgttttaaatgaattaaattgtgaaattagttagtaaattaatttgtagtaagtaattatttaaggaaattaaaatattgtttagtttagttttgtattttattatgtgtatgcgttttttataattaattaatataagtgttttaggaatatttgaagataaatacgtttaatttaaggaataaagtatttaaataatttaagtgtaattttgttgagttaaagtaaaatattttataaatgaagtggttatttaattttttagggaaagtttggttattgaaatgttgtatgtttatgttatattaataaaaatttttaatttattttgtttatgtgttttgtttttttgatattattggtatttgaattttagatggatttttgttaaaatgatattttgtgtgataaaagtatttttagttttgattgatagattaaaataaatgtaaggaaatttttttaaattagattaattttttataaaaatattttagaatgtatgaattttgatatttatatttataatggtaaaagtttttttcgtttagtttagtaagataatatttatataaaagagtaaaaaaaaattatattattttatgatagtttgatttttaaattgtttaagaaagtaaagtggttaaattggaaaagaggaatatatttcggaggtttagaatcgaaaattttttttttaatttttagttggaaaataattttttgtatttatttaaagtgtattttttgaagtgttagattggagttgattggtgattaatttaaaggagttataatttaaagaaatggtgagagtttggtatttaggtttggtttttaggtaattcgtttgggtttgagaggttattaattgttagttaagatggaattttttttttttttttttttttttaatggataataatgggaagggggttaattttttagtagttgaaattttgtatttagttttttattttgagaatgttaatttttggttcgaggatttgtttttgtagtgttggtatcgagatttaagggaagatatttcgttttaaatgttagttacggtttggtttttttttcgattttagtattttgtagattgttagtgtttgtggcgggggacgaaaggaatagggttttgtaaggtttgtttgtcgattgcgttattttgggcgaaatttagttttaaaagttataaattatttacggtgaagatttttcgaagtggaataaatttttagattcgtattattttatatttttgcgggatagatggtttttatttatcggttatcgggagagagttgttgttttcgcgttttattgtttttcggggcgatttttagcgagtcgagttttcggttgtacggtaagcgttcgaaagtcgggtttgagaggattgtagggtttttgagggtgttaagtttcgaaggagtttacgggtgtattggggttttcgaaatttagtcgttattggtagtttttttttgtttttttttagttttttcgttcggtttcgtattttttttttttttttttttttttattttttttttttttttttgtttttatttcgtgtggggagtgacgtgacgttagtagagattttattaaattttattgtatagtggcgcgcgggcggtcggtcgagttcggttgcgcggttggcgatttaggagcgagtatagcgttcgggcgagcgtcggggggagcgagtaggggcgacgagaaacgaggtaggggagggaagtagatgttagcgggtcgaagagtcgggagtcggagtcgggagagcgaaaggagaggggatttggcggggtatttaggagttaatcgaggagtaggagtacggatttttattgtggaaaggaggattagaagggaggatgggatggaagagaagaaaaagtaatttgcgttaattcggtagttttaataaattaaagggggagcgttagggtagcggggagatagaaacgtatttttggggagtaaattaggacgggttgggaggaagcgatagggaaagtggtttaagagacggaataaaggataatgtttatggggttgtttgggacgaggcgtgtggagtgtgggtgtgagcgtgcgtgtgtgatttttttttaggtttgtagagttgaggaaagaggttatagtaaagagggattgcggagggaggaaagtgagagatcggtagagggcgggagtggaggtgggcgcggtggggatgggagaggatgagtgaagagaaatttagaagaatggagtgagttagtgggagagggtgggagggttatagtcgggagcgaacgagttaggtttgttagttggggaaggtcgggacgttgggtttagtttagttgggatatcgcgttcgaggttaaggcgggtggattaggtatgttgagagtgtcggcgtataggtgggtacggttacgtattgatttagtgtttacgaagggtttgtattggataaggtttagacgtttatagagtttagaattttttttgttgtatttatatttaataagtttattttgggttacggatattttattttttaaaatgacgaggttaaggtttttggcgaggatggtattaaattgtacgggatagaagtgggggtgggggagagagttttttttaagtttatatttgtttttgtaaagtaaagagtatgtgaaattatagggtatatttttattcgaaaagtgtgttttatttttgaattttgattttttgattttttgatttgagtaaagatgtgtattttggtagtgagtagaatattttggttttgttttgtttttgagtggaaggattataaatataattcgtttggaggattaggtgtgaaggtttttgttaggtatatgggataatgtttttttaattttaagggtattttgttaatgtatgtttttggaaagtgtcggaatatagttattgtttttggattcggatttttttattaatattaatttttgtttgagagtaaaatttaggttcgttattaaaaagatatttttttggtttttaattgagaataaagttttttttaaaagttgtattgttttttttaaattaatatattaatattcgtaattttagaaatatatagtgattcgggagaatgtgtataaaatagatacgtttaaaaaagtttggcgtttaaaattaattttagttattatataggtgttgggttttttttatttttgggggttgtttggaatatgttatgtgtttttttgaattatttcgtgttttgaatttatttgagttagtagtaaaaataggtaaataaatttgtttaatttgttttgagtgttaaatttttttattttgaaatagttaatagtcgatagatggatttattttatggaaagggttagtttttttagttacgaagaaaattgattagagatttatattttaagttatttttaatttttacgtaatattcgtgaaaatttaaattttttttttttatttagtggaaatttaaagtagtgttatttaaggggagagaaatgagggggaaaatgtttacgtgttgtttaattgtattttttttttgattttgagaatttttatttttggtttttgaaatttcgtcgaggtaagaaaattaaatttttttaataagttttataattgaattttagttataggatatcggaaagtgtagttcgagaaagatatttttatttttgtttatcgacgatttttgtagtttttttatttttttgagtaatgggttaataattttttttttttttttttttattttgtagagattaagaggcgttcgtagtagaacggttttgtttttagttggtggcgaggataggtaattttatggaaaagttggaagagaatgagaaaattaaagatagaaagatttagagattcgcggagagatatagggagagggaagggagttgcgttgaaaagacgtaaagatacgcgcgtgtaattttttttttttttaggttttagaggtttgtaaattagggttgagaggaaggggttcgggaagtttacgtttttttcgttttttttttgtttggagtttcgttcgttagaggttggttaattttagtttcggtcgtcgtagatattgcgttgagtttttgggttttcgttttgtttagcgttagtgtagttgaagtgagtagttggtgggaaatgtaaatggtttttggagaaatagaagatatagaatgatttttatttttttttcgagtgtgtggaaggagttggatatacgttttacgtttttaattttttttttatatttttagttatatttttattaaataattaattaatgtttagaattattagggaatatattaggtatgtaatcgtagaagtagggtgttggggggttataaattatcgagttgatttaagacgtggattttaggttttttttttgttaaagtagtaaaggaagagcgggttttggcgattgtatttagatttcgattattttaaattagaagggggtggagggagcgtttaagtaaagtaagtaattttttgttttgtagatgtaaataagattgtagtattaaaggtattagtttttttagggttagatcgtttggattgggagtttggggaaggggagatattaattttacgtatttgtgaattttaaggatgttatatttttatataaataattttagtgcggattttttggaatggggggagtaatatttttattttagaatattaaaatattttttttttaaagcgtatattttttttatttttttaaaattttgaattatgtttaaagataatagttttttagtaaattggagtattggattattttttttatttttttttatcgatattttgatgatttgattttaatgtgtggggggtatagggaattaaatatagtttataaaattaagtttagatgaaatagtgttggttaagtgggtttagataatttttaatgagaattttaattatatttttttttttaatatgttgagataagtgatagaatcgttagaatggtaattaaattggaaagtttagggagaataataatttcgtgattaaattggggtaaaatcgtggataaatgtggggtgattttcgttaattttttgttatttaagagttaggatttgggaaaggtatagtattattttagagttcgttgtgacgggttgtgtgttattatttattttttttattttggattatgattttaattttggtaagtaatttttttagttttttatttgataataagcgagtatgtaaatattaatggttagcgatgtttaattgttttaaatattattgatttgttggttgttttaaattgtttttttagtttaggttttgttttcgaattgtttattttagaggtttgatttatgttttcgatgttataatataataattgtttttttaaaaaaggtatttaagatgaattaattgatttgtatataaattaaaattattatgcgttgtcgatttcggtgttttataattatttcgaaattagtatttaattatttgagttaaaagaatatataaatgtttgtattgatttattaatgaattatttaattaaaacgttcgggtaatgttgggcgttggaaagattgttaaattaagatatattataggagggatatgaagattagaaaggtaatagattaatatttcgtatttaaaacggagttttcggtgatttttagttttaattttggagtaggggttttttttttttgttgttaaaaagattttgtgtttgtttgtgagtgagtgtatttaagtggaaggaacgtttttacggttacggtggtttaggttttttgttcggatcgggattttatagttttaatttaggagcgttaaattttggaagatttcgggttagttttggaggtgcgtggtttcgtaagtcgttaggttaagtttgttttttttgtttgttttttcggtaggttgggcgcgttatggtagtgagtttttcgcgtaaacggagagttggaattaaagttgatatttaatagatatgttaattgagtatttattttcgttttgagaataggaataaaaggtagttttttttaagagaggcggtgtaaaggtacgttataggagtttagaaaaggttggcggcgggaaatttgtagtttgggggttagttaatatttttttttattttaagtatttattgatttgttgttgttatttttggcgacgtagaaggatatttgaaagaatttttgatggggttttgatttgagaaaggaggtgatttgtttaggtttttattaaatttttaattattatattaattgtttttttttattttttattcgatttttttttttttgtttatttttaattttttaattatttagaaatttttttattttttagtggttttttttttgtagtagttttttattcgaatttttttttcgttttttcgtggtagggtttgtatattgatttttttgatttttggtatatttgggttttttgaaattttttaatttttttagatttgaggatggtaggttttattttttttattgtgtgtatatatttagagatatgaaaatttatatagattgtttttaaatttagggtatttaatagatgttttttttttagttcgttttttgatttgaaatgtttgtttgattttaatttggatattatttttttttgtttttttttttttaaagtagtttggatatgtgtgtaagtgagtttagaatagttttatttatattttttattaaattgtaaataaaagaagaattaatgaagtagattggtatatagattgtattaagagttcgaatttttagtttttggattttttatttaattttggttgttatttatattgatagagttattttaagtagaggtttagagaaatttgtattgtgggataataggtaaagttatagtaaaaagtggaataattttaaagttattttattagaatgtaaattgtatttttgggttttgttcgtaattatttagttttaatatatatagagttagataggaaaaaataggttaatatagttattggtattagagaagataaattttatgggttttttagtgaaaagaagatttttaaagtttataatttttgattatttaattttatttataattgtgggaatgaataagatattaattgttttatgtattttatttatattaattaatttgtgtttttattaaaagtagttatatagaattttttttaatttttggtagtaagtttagaaaatgaagtttatagttattttgaattggatatattttttgagttgattatttttgtaagtgtaggaatataatattgtttttttatggtttttttgtatttttttagggtttgtaagtttttattaggtttgatattattgtttgggtttatatttattataagtaaatttgattattatgttgattttaaaatagtttatttggttagtataattttagtttttaaattataaaaattttttaatatacgaagtttttagtttttattttttttagttttttgtttatttaaaatttttattttaattggtgtaagtaataataatttgtattattatttgtattttttttatttttttggagattgggttggattttagagagaatattagtattattattattataaataataaaatttaaaagtaaagtttttatttgtatgataattggtatttggaatgtttttgatttatttaatgttattttataaaggtattttgtaaatttttttggaatttttagtaagagtttgtagtaattggaataattttttgggaagatattttttttgatgggtttttagtttttggaggaatagattgagagtaattagggagggaggggatattggaaattggtagttacgttagttgaaataagtttgggtttagtaaggtgattgatgttgtggttgattttttatttcgagtttttttttaattggggtattgattttttttattttgggattttaaggtattcggtgtgtatgtagattttttttttgtggtttttattatgtggtttcgtagtaggtttttggtttaatgatattttatagttatagtttttatatttattattatgattttaatgtttaggtttttagtgtatttatattaaatttgttttattagtaagttggagtatataggagagatgggggtaagtaaggatttagtagagtttaaatttagatatgtttaaatggttttgattgtgtaaagtgtggtaatgttttttgttgttttagttttttattttaagttttatatgttttttggttaatgaagtgtgatataggttatatgttaggaataatagtatttgttgagaataaagtgaatttaggaaatttggtatatataaaatgtatttagttatttgaattagtaataatggtaaaaattaatatttatagagtgtttagttaatttagttattgtattaaatatttttgtattgataattatatttattttttatgttaatattataaggtaggtattgttattttataaatgaagatagtgaggtttgttatgattgtgttattggtttaaggttatttagttggttagagtataagtttataattgttggaggttatagtggataggatattgttttaggttacgtaggtagtaagtggtatagtgggaatttgaatttaggtttgtgtaattttaaagtttaaaatgttaattagtatattgaattaatggtaattggaattagaagattaggggtttttgggggaaggaaatatagaatttatttatggaatattttataaataaaagaataatgtagagataggaaagtaaatatattttttgagggatggagaaagttagaaatgttttaaatgttaaagaggaggaaacgagaaatgattggatgagaaagtagaaaagttaaatttcggtatttgttttgggtagtttaggaagagaaaggtaagtttagggatatttttgagttataggaaaattaatgtttagatggttagtttggattaagtttaatataggattttaggaatatggtttattagaattgttttttagtaattttaagggagaataaaatttttgaattgggtttaagtagttttattttagaagtaaagagagatggaagtaaggatcgagtaataagaatatttatattgtaagaatatgtaagttgagtaggagtgaaatttagaaaaatttgttaggattttggttgttgtgttaaattatgttatattttaagtagaaattagatttttattattattatttgtttaggtttagttagtaattttattattgtagtaaagttatttgaaattttaagagaaatgattttttgtgttgaagaagatattttgggtggaaggatgttagtagataaatggagtgtaaagatagtgattttaaggatatagtttgtggggagtaatattggattatatattcgttgtttgtggtagaatgttagttaggggagaatattaggtagttttttataagtttattttattataaaaagataggattgattttaaaggttatttttaatttaggtttgttttattattgaaaatgatttaaaattggatttattttggttttttttaggagggatagataaatataatttgtatatatggttttttagttttaggaagtataggaggagaatgaaagaattaatttagttttttgttttttggtaaaaatttttatatttgtgttgttgtaagaatttaagattatttcgtttagaatgttgtggtatttttgaaagtaaggtttgagggtatatagagttttattttttatttttacgttgtggattttattgttttttttaaatgggaaagagaaattagaatttatagaaagtaaggtttggaaaggatttagagggtattttttttttttagtttatgtttaaattatttttagaaatatagttagttatattttttagtaaagagttttttacggttttttggtaatgtatttttatgttttataattttatagttatattgtatatttattgattaaattttaagtattgaagaaaatgatgttatattaaaaagttttaattagtagggggtatgttttttagagttttttaaatattttatatttttattttaaaaaaagatgaaaatattattagtttaatttaatagatggaaaattttgttatagagatttttagagagttatatttggttatgtagcgtgatgtttgaaagaattaaattaaaaataaagttaggaaattttatgtttagggtttttttagtagatatattattttttgggggttggttattatttttttgtttgagtaaagtatatgtttgattgtaattttatttgtttttttgtttgtttgtttgtgagtagtttattttttaatttattaatttatttttttgttagttttttaaaatattataagttaattaatgttgataaaattttatttttattatgagtgttatttgagtagattgagatggttgttatattttttaaatattacgtgtaataaatagtgttgttattgttttagcgttatgattttgtttttatttggaaattgtataaatattatattttttgttatgataggattatttttatttattaggatttttgatatttgtgttgttatttgggagaatgttgattattttgtttatgttatttttgaggttataataatcgtttttttgtttagttgtgtttttttttttataggtgaatttagtttttttttttatgtttgattttaagaaattggtgttttattgaaagatgtttaaattttttgagagaaaatgttggagtaagaataatttgttatgtattgtttttatttgagtattaatgtttttttaattttatatgtttttaaattttttgagaattttttttttttgaatgtaatttatgaattaaaagtgatcgtaatttttaaaatattatgttgtttatagtaaatatatataatttttatttgttaattaaaaaaagtaatagggtttttatttttatttttgatatttgttttttttattttttttttaagtattttttttttttttttagagatgtatttattgagagtattttgttattttttttttttcgtagttatgtatgattaaagttgtgtttttgaaattttttattttttttgttataattgataatttattttgttttttattaatttattaatgttattttattggtttttgatttatataaattaaatagattttagaaaatttaataaaaataaaaataatgttttttattttgaaatatttatttattgtttttttttagggtatatatattatattttttttttttatattttattttttttgaatttataagaatgtgttattgaatatagagaaaataatttaagaaaggaaaaggaatgatttgtttaaaatgaggaaaaagtagagtcgaggtttaggattgtggtttaataagatgatttagttattttttggtagttttattttttggtaattttttaagttgagttttggatgatgtaaataatatttttagatttttaatgggtatatgttgaattaaaaagaaaaatttatggtattttttaattatgtgtaaatgagtaaagaaaaaggaaagaaaaggagtggttaaattgatatggtagggtttaggattgggggaagaagaaagagtaatagagagagtggaatagttaaaaaaagaatgagattatgttttttgtagaaatatggatggagttggaggttattatttttagtaaattaaattaggattagaaaattaaataacgtatgtttttatttataagtgggagttaaatgaggagaatttatagatataaagagaggaataatagatattggggtttattggaaggtggcggatgggagaggggagaggattagaaaaaataattattgggtacgaggtttagtatttgggtgataaaataatttgtataataaatttttgtgataggtttatttatataataaatttgtatatgtgttttgaatttgagatataatttaaagaaaaagagagcgtatttgtttgtaaattggttttagtagattgttttttgagttttttttgttttttaaattgaatttaagtggtattatatttttaaatgaaaattttatttttaattataggtgaagttaattttttatttttttaataatttttttattattttttgtattgtaagtaaggtaaagatttagtttaaatgttgttagtttagtttattttttaaaaaatatattttttgagaggtttgagaaaattaagaaagtatattttgtttagtttttttaaatattatttttttggaaatagtattttgtttagtttttttaaatattattttttaattagtgagttagtttagattttagagggtttttggaattagaaagaaggtaaggatgaatattaggtttaagattatttttatgttgttttattattaaattagaaaatttggatgttttgtaggtaggtatgtttatgagagttatttaaaaaagatatgttttttgaagtgttaagtttagtgattacgtagtttatg

SEQ ID NO: 8 - DNA, 12001 bp, Homo sapiens
gtgttagattggagttgattggtgattaatttaaaggagttataatttaaagaaatggtgagagtttggtatttaggtttggtttttaggtaattcgtttgggtttgagaggttattaattgttagttaagatggaattttttttttttttttttttttttaatggataataatgggaagggggttaattttttagtagttgaaattttgtatttagttttttattttgagaatgttaatttttggttcgaggatttgtttttgtagtgttggtatcgagatttaagggaagatatttcgttttaaatgttagttacggtttggtttttttttcgattttagtattttgtagattgttagtgtttgtggcgggggacgaaaggaatagggttttgtaaggtttgtttgtcgattgcgttattttgggcgaaatttagttttaaaagttataaattatttacggtgaagatttttcgaagtggaataaatttttagattcgtattattttatatttttgcgggatagatggtttttatttatcggttatcgggagagagttgttgttttcgcgttttattgtttttcggggcgatttttagcgagtcgagttttcggttgtacggtaagcgttcgaaagtcgggtttgagaggattgtagggtttttgagggtgttaagtttcgaaggagtttacgggtgtattggggttttcgaaatttagtcgttattggtagtttttttttgtttttttttagttttttcgttcggtttcgtattttttttttttttttttttttttattttttttttttttttttgtttttatttcgtgtggggagtgacgtgacgttagtagagattttattaaattttattgtatagtggcgcgcgggcggtcggtcgagttcggttgcgcggttggcgatttaggagcgagtatagcgttcgggcgagcgtcggggggagcgagtaggggcgacgagaaacgaggtaggggagggaagtagatgttagcgggtcgaagagtcgggagtcggagtcgggagagcgaaaggagaggggatttggcggggtatttaggagttaatcgaggagtaggagtacggatttttattgtggaaaggaggattagaagggaggatgggatggaagagaagaaaaagtaatttgcgttaattcggtagttttaataaattaaagggggagcgttagggtagcggggagatagaaacgtatttttggggagtaaattaggacgggttgggaggaagcgatagggaaagtggtttaagagacggaataaaggataatgtttatggggttgtttgggacgaggcgtgtggagtgtgggtgtgagcgtgcgtgtgtgatttttttttaggtttgtagagttgaggaaagaggttatagtaaagagggattgcggagggaggaaagtgagagatcggtagagggcgggagtggaggtgggcgcggtggggatgggagaggatgagtgaagagaaatttagaagaatggagtgagttagtgggagagggtgggagggttatagtcgggagcgaacgagttaggtttgttagttggggaaggtcgggacgttgggtttagtttagttgggatatcgcgttcgaggttaaggcgggtggattaggtatgttgagagtgtcggcgtataggtgggtacggttacgtattgatttagtgtttacgaagggtttgtattggataaggtttagacgtttatagagtttagaattttttttgttgtatttatatttaataagtttattttgggttacggatattttattttttaaaatgacgaggttaaggtttttggcgaggatggtattaaattgtacgggatagaagtgggggtgggggagagagttttttttaagtttatatttgtttttgtaaagtaaagagtatgtgaaattatagggtatatttttattcgaaaagtgtgttttatttttgaattttgattttttgattttttgatttgagtaaagatgtgtattttggtagtgagtagaatattttggttttgttttgtttttgagtggaaggattataaatataattcgtttggaggattaggtgtgaaggtttttgttaggtatatgggataatgtttttttaattttaagggtattttgttaatgtatgtttttggaaagtgtcggaatatagttattgtttttggattcggatttttttattaatattaatttttgtttgagagtaaaatttaggttcgttattaaaaagatatttttttggtttttaattgagaataaagttttttttaaaagttgtattgttttttttaaattaatatattaatattcgtaattttagaaatatatagtgattcgggagaatgtgtataaaatagatacgtttaaaaaagtttggcgtttaaaattaattttagttattatataggtgttgggttttttttatttttgggggttgtttggaatatgttatgtgtttttttgaattatttcgtgttttgaatttatttgagttagtagtaaaaataggtaaataaatttgtttaatttgttttgagtgttaaatttttttattttgaaatagttaatagtcgatagatggatttattttatggaaagggttagtttttttagttacgaagaaaattgattagagatttatattttaagttatttttaatttttacgtaatattcgtgaaaatttaaattttttttttttatttagtggaaatttaaagtagtgttatttaaggggagagaaatgagggggaaaatgtttacgtgttgtttaattgtattttttttttgattttgagaatttttatttttggtttttgaaatttcgtcgaggtaagaaaattaaatttttttaataagttttataattgaattttagttataggatatcggaaagtgtagttcgagaaagatatttttatttttgtttatcgacgatttttgtagtttttttatttttttgagtaatgggttaataattttttttttttttttttttattttgtagagattaagaggcgttcgtagtagaacggttttgtttttagttggtggcgaggataggtaattttatggaaaagttggaagagaatgagaaaattaaagatagaaagatttagagattcgcggagagatatagggagagggaagggagttgcgttgaaaagacgtaaagatacgcgcgtgtaattttttttttttttaggttttagaggtttgtaaattagggttgagaggaaggggttcgggaagtttacgtttttttcgttttttttttgtttggagtttcgttcgttagaggttggttaattttagtttcggtcgtcgtagatattgcgttgagtttttgggttttcgttttgtttagcgttagtgtagttgaagtgagtagttggtgggaaatgtaaatggtttttggagaaatagaagatatagaatgatttttatttttttttcgagtgtgtggaaggagttggatatacgttttacgtttttaattttttttttatatttttagttatatttttattaaataattaattaatgtttagaattattagggaatatattaggtatgtaatcgtagaagtagggtgttggggggttataaattatcgagttgatttaagacgtggattttaggttttttttttgttaaagtagtaaaggaagagcgggttttggcgattgtatttagatttcgattattttaaattagaagggggtggagggagcgtttaagtaaagtaagtaattttttgttttgtagatgtaaataagattgtagtattaaaggtattagtttttttagggttagatcgtttggattgggagtttggggaaggggagatattaattttacgtatttgtgaattttaaggatgttatatttttatataaataattttagtgcggattttttggaatggggggagtaatatttttattttagaatattaaaatattttttttttaaagcgtatattttttttatttttttaaaattttgaattatgtttaaagataatagttttttagtaaattggagtattggattattttttttatttttttttatcgatattttgatgatttgattttaatgtgtggggggtatagggaattaaatatagtttataaaattaagtttagatgaaatagtgttggttaagtgggtttagataatttttaatgagaattttaattatatttttttttttaatatgttgagataagtgatagaatcgttagaatggtaattaaattggaaagtttagggagaataataatttcgtgattaaattggggtaaaatcgtggataaatgtggggtgattttcgttaattttttgttatttaagagttaggatttgggaaaggtatagtattattttagagttcgttgtgacgggttgtgtgttattatttattttttttattttggattatgattttaattttggtaagtaatttttttagttttttatttgataataagcgagtatgtaaatattaatggttagcgatgtttaattgttttaaatattattgatttgttggttgttttaaattgtttttttagtttaggttttgttttcgaattgtttattttagaggtttgatttatgttttcgatgttataatataataattgtttttttaaaaaaggtatttaagatgaattaattgatttgtatataaattaaaattattatgcgttgtcgatttcggtgttttataattatttcgaaattagtatttaattatttgagttaaaagaatatataaatgtttgtattgatttattaatgaattatttaattaaaacgttcgggtaatgttgggcgttggaaagattgttaaattaagatatattataggagggatatgaagattagaaaggtaatagattaatatttcgtatttaaaacggagttttcggtgatttttagttttaattttggagtaggggttttttttttttgttgttaaaaagattttgtgtttgtttgtgagtgagtgtatttaagtggaaggaacgtttttacggttacggtggtttaggttttttgttcggatcgggattttatagttttaatttaggagcgttaaattttggaagatttcgggttagttttggaggtgcgtggtttcgtaagtcgttaggttaagtttgttttttttgtttgttttttcggtaggttgggcgcgttatggtagtgagtttttcgcgtaaacggagagttggaattaaagttgatatttaatagatatgttaattgagtatttattttcgttttgagaataggaataaaaggtagttttttttaagagaggcggtgtaaaggtacgttataggagtttagaaaaggttggcggcgggaaatttgtagtttgggggttagttaatatttttttttattttaagtatttattgatttgttgttgttatttttggcgacgtagaaggatatttgaaagaatttttgatggggttttgatttgagaaaggaggtgatttgtttaggtttttattaaatttttaattattatattaattgtttttttttattttttattcgatttttttttttttgtttatttttaattttttaattatttagaaatttttttattttttagtggttttttttttgtagtagttttttattcgaatttttttttcgttttttcgtggtagggtttgtatattgatttttttgatttttggtatatttgggttttttgaaattttttaatttttttagatttgaggatggtaggttttattttttttattgtgtgtatatatttagagatatgaaaatttatatagattgtttttaaatttagggtatttaatagatgttttttttttagttcgttttttgatttgaaatgtttgtttgattttaatttggatattatttttttttgtttttttttttttaaagtagtttggatatgtgtgtaagtgagtttagaatagttttatttatattttttattaaattgtaaataaaagaagaattaatgaagtagattggtatatagattgtattaagagttcgaatttttagtttttggattttttatttaattttggttgttatttatattgatagagttattttaagtagaggtttagagaaatttgtattgtgggataataggtaaagttatagtaaaaagtggaataattttaaagttattttattagaatgtaaattgtatttttgggttttgttcgtaattatttagttttaatatatatagagttagataggaaaaaataggttaatatagttattggtattagagaagataaattttatgggttttttagtgaaaagaagatttttaaagtttataatttttgattatttaattttatttataattgtgggaatgaataagatattaattgttttatgtattttatttatattaattaatttgtgtttttattaaaagtagttatatagaattttttttaatttttggtagtaagtttagaaaatgaagtttatagttattttgaattggatatattttttgagttgattatttttgtaagtgtaggaatataatattgtttttttatggtttttttgtatttttttagggtttgtaagtttttattaggtttgatattattgtttgggtttatatttattataagtaaatttgattattatgttgattttaaaatagtttatttggttagtataattttagtttttaaattataaaaattttttaatatacgaagtttttagtttttattttttttagttttttgtttatttaaaatttttattttaattggtgtaagtaataataatttgtattattatttgtattttttttatttttttggagattgggttggattttagagagaatattagtattattattattataaataataaaatttaaaagtaaagtttttatttgtatgataattggtatttggaatgtttttgatttatttaatgttattttataaaggtattttgtaaatttttttggaatttttagtaagagtttgtagtaattggaataattttttgggaagatattttttttgatgggtttttagtttttggaggaatagattgagagtaattagggagggaggggatattggaaattggtagttacgttagttgaaataagtttgggtttagtaaggtgattgatgttgtggttgattttttatttcgagtttttttttaattggggtattgattttttttattttgggattttaaggtattcggtgtgtatgtagattttttttttgtggtttttattatgtggtttcgtagtaggtttttggtttaatgatattttatagttatagtttttatatttattattatgattttaatgtttaggtttttagtgtatttatattaaatttgttttattagtaagttggagtatataggagagatgggggtaagtaaggatttagtagagtttaaatttagatatgtttaaatggttttgattgtgtaaagtgtggtaatgttttttgttgttttagttttttattttaagttttatatgttttttggttaatgaagtgtgatataggttatatgttaggaataatagtatttgttgagaataaagtgaatttaggaaatttggtatatataaaatgtatttagttatttgaattagtaataatggtaaaaattaatatttatagagtgtttagttaatttagttattgtattaaatatttttgtattgataattatatttattttttatgttaatattataaggtaggtattgttattttataaatgaagatagtgaggtttgttatgattgtgttattggtttaaggttatttagttggttagagtataagtttataattgttggaggttatagtggataggatattgttttaggttacgtaggtagtaagtggtatagtgggaatttgaatttaggtttgtgtaattttaaagtttaaaatgttaattagtatattgaattaatggtaattggaattagaagattaggggtttttgggggaaggaaatatagaatttatttatggaatattttataaataaaagaataatgtagagataggaaagtaaatatattttttgagggatggagaaagttagaaatgttttaaatgttaaagaggaggaaacgagaaatgattggatgagaaagtagaaaagttaaatttcggtatttgttttgggtagtttaggaagagaaaggtaagtttagggatatttttgagttataggaaaattaatgtttagatggttagtttggattaagtttaatataggattttaggaatatggtttattagaattgttttttagtaattttaagggagaataaaatttttgaattgggtttaagtagttttattttagaagtaaagagagatggaagtaaggatcgagtaataagaatatttatattgtaagaatatgtaagttgagtaggagtgaaatttagaaaaatttgttaggattttggttgttgtgttaaattatgttatattttaagtagaaattagatttttattattattatttgtttaggtttagttagtaattttattattgtagtaaagttatttgaaattttaagagaaatgattttttgtgttgaagaagatattttgggtggaaggatgttagtagataaatggagtgtaaagatagtgattttaaggatatagtttgtggggagtaatattggattatatattcgttgtttgtggtagaatgttagttaggggagaatattaggtagttttttataagtttattttattataaaaagataggattgattttaaaggttatttttaatttaggtttgttttattattgaaaatgatttaaaattggatttattttggttttttttaggagggatagataaatataatttgtatatatggttttttagttttaggaagtataggaggagaatgaaagaattaatttagttttttgttttttggtaaaaatttttatatttgtgttgttgtaagaatttaagattatttcgtttagaatgttgtggtatttttgaaagtaaggtttgagggtatatagagttttattttttatttttacgttgtggattttattgttttttttaaatgggaaagagaaattagaatttatagaaagtaaggtttggaaaggatttagagggtattttttttttttagtttatgtttaaattatttttagaaatatagttagttatattttttagtaaagagttttttacggttttttggtaatgtatttttatgttttataattttatagttatattgtatatttattgattaaattttaagtattgaagaaaatgatgttatattaaaaagttttaattagtagggggtatgttttttagagttttttaaatattttatatttttattttaaaaaaagatgaaaatattattagtttaatttaatagatggaaaattttgttatagagatttttagagagttatatttggttatgtagcgtgatgtttgaaagaattaaattaaaaataaagttaggaaattttatgtttagggtttttttagtagatatattattttttgggggttggttattatttttttgtttgagtaaagtatatgtttgattgtaattttatttgtttttttgtttgtttgtttgtgagtagtttattttttaatttattaatttatttttttgttagttttttaaaatattataagttaattaatgttgataaaattttatttttattatgagtgttatttgagtagattgagatggttgttatattttttaaatattacgtgtaataaatagtgttgttattgttttagcgttatgattttgtttttatttggaaattgtataaatattatattttttgttatgataggattatttttatttattaggatttttgatatttgtgttgttatttgggagaatgttgattattttgtttatgttatttttgaggttataataatcgtttttttgtttagttgtgtttttttttttataggtgaatttagtttttttttttatgtttgattttaagaaattggtgttttattgaaagatgtttaaattttttgagagaaaatgttggagtaagaataatttgttatgtattgtttttatttgagtattaatgtttttttaattttatatgtttttaaattttttgagaattttttttttttgaatgtaatttatgaattaaaagtgatcgtaatttttaaaatattatgttgtttatagtaaatatatataatttttatttgttaattaaaaaaagtaatagggtttttatttttatttttgatatttgttttttttattttttttttaagtattttttttttttttttagagatgtatttattgagagtattttgttattttttttttttcgtagttatgtatgattaaagttgtgtttttgaaattttttattttttttgttataattgataatttattttgttttttattaatttattaatgttattttattggtttttgatttatataaattaaatagattttagaaaatttaataaaaataaaaataatgttttttattttgaaatatttatttattgtttttttttagggtatatatattatattttttttttttatattttattttttttgaatttataagaatgtgttattgaatatagagaaaataatttaagaaaggaaaaggaatgatttgtttaaaatgaggaaaaagtagagtcgaggtttaggattgtggtttaataagatgatttagttattttttggtagttttattttttggtaattttttaagttgagttttggatgatgtaaataatatttttagatttttaatgggtatatgttgaattaaaaagaaaaatttatggtattttttaattatgtgtaaatgagtaaagaaaaaggaaagaaaaggagtggttaaattgatatggtagggtttaggattgggggaagaagaaagagtaatagagagagtggaatagttaaaaaaagaatgagattatgttttttgtagaaatatggatggagttggaggttattatttttagtaaattaaattaggattagaaaattaaataacgtatgtttttatttataagtgggagttaaatgaggagaatttatagatataaagagaggaataatagatattggggtttattggaaggtggcggatgggagaggggagaggattagaaaaaataattattgggtacgaggtttagtatttgggtgataaaataatttgtataataaatttttgtgataggtttatttatataataaatttgtatatgtgttttgaatttgagatataatttaaagaaaaagagagcgtatttgtttgtaaattggttttagtagattgttttttgagttttttttgttttttaaattgaatttaagtggtattatatttttaaatgaaaattttatttttaattataggtgaagttaattttttatttttttaataatttttttattattttttgtattgtaagtaaggtaaagatttagtttaaatgttgttagtttagtttattttttaaaaaatatattttttgagaggtttgagaaaattaagaaagtatattttgtttagtttttttaaatattatttttttggaaatagtattttgtttagtttttttaaatattattttttaattagtgagttagtttagattttagagggtttttggaattagaaagaaggtaaggatgaatattaggtttaagattatttttatgttgttttattattaaattagaaaatttggatgttttgtaggtaggtatgtttatgagagttatttaaaaaagatatgttttttgaagtgttaagtttagtgattacgtagtttatg

SEQ ID NO: 9 - DNA, 4001 bp, Homo sapiens
tagagtatttaattttttttttttaatagtaaagtttttggatgtcgtttgatttgtttgattttgttttttgtttttagaattttaataaatttggaattttttatcgattagtataaattaggacgttgttattgggttatttatttgagtttatttttgttaatttataaagtatagatttgttataaagttaaggtaagttttttttataaaattatgattataatttagaagagggggtgtgagttttaatttttagagtttaatttttgagagaagataaataaattaagtagaaaagttttttttttttttttttttttttttttaagaggattagtagttgtgtattaaaattttgttttcggagattataaaattaggaaatagggtgtgtgggagagatttgaatggtcgaaataatcgtaaagaaggtgtaagaagcgcgagtttaggagggaaaaagttgggttagggtcgggataaaggttttttagggagggttaattttttcgtgtttttggcgggttttttttgttaaaggtttataggttggagtttgttcgcggtttttggtttggtagggattttattagttttgttttggtaattgtaagttaggaatataatgttttgtgtaggggattgtttatgtagtttagttcgtgagatcgcgggatggcggggtagtgagtcggtgtcgttttgggagtttgagttagggcggtagttttgtcggtttcggagagggaattgtaatttcgtaattaggtcgtcgcgaggttttttgtttttgtaaagttgcgttttatcggcgtttttttaggcggcgttgttttttatatttttttttggtttatttggtttgtatttttataatattttttttttattttttttagatttcgtgttggtttttattcggattcgggttttcgtaaggttggtttatatagcgattttttcgcgtgtggatatgttcgggtagcggtttttttggaaagtggtttttagtttttggagttgttggttggtaaagtgagttcgttgtcgtttttgtcgtttttttttagacgggttttcggcgtttacgtttttattttttttttgttggtttttatttttttttgaaaacgaaatatatatattttttcgttagtatgtttatttgtaacgcggacgttaattggatcggcggtagaagtcgtggaagagttgggttgtttggcgtcggaggagggtgcgcgcggcggtttcgggtcgcgaggagcgttgcgtttgtggggtgtgtaggcgtaagtgtgggtgttcgcgttttattttttttttttttttagcgtcgtacgttttatttatatgtttattttattgtagcggtatatttatttttatagtttgtgtttttaagtatatttatatatttttgcgtagatatattaaattttttgggacgcgtatacgcgcgtggtttatagatttttttttttttcgtagaaagtttagatttttatgcggtttgggaaggttaggaaaagatgtggggattcggttgggtatcgaagttcgtcggtttttttttaaaaaaaaaaaaaaaatgttttttcgcgaagggtatttttgagtggttttaggtaattttttaacgagtggagtttttcgggagttgaaagtcgagaggaaaatagggatagaggtcggcggtttttgaaggttttcgaattaagatgttgggatttttgtgatttaggaaatagaagggaggttagggtacgaatagagagggcggtagaattgttcgcgtttttagcgttttaggagtcgggtcggtcgagggagaattaaagggatgcggggtagttaaaatttcggttttcggaagttttgcggggagttaggcgaacgattatttttattacgttttttttcggaggggttgatttttttggggcgagagggagcgggtggcgtagagtagttgagcgggaatgtttgtagggcggcgcggcgttttatttgcggttttcgggttggaggtgtcggagatggtgtgtatttttagtttgtgtttggaggagtttagcgatcggggttgatcgggagttagaatcgaagttatggttaacggttggggatggtgataggaagatgaggagacggtcgatagtttggttttcgttgttcggtgttttaagtgaagcgggttttttatgtagtttatggacgagggagcgcgacgttttattagtttttggttattgtttcgtcgagttttcgtagtcgtcgttgttcgtttcgggtcgcgttttaggcgcggagttttttcgttgcggggagagttaggggacgtaattttcgtcgagtttttaagttaagttgttttcgtttttttcggaaggtttaagcgaaaaagttcggagacggaaagttagcgggtaaacgaagatatgggatgtgggtagaagggtattatttagagcgtttttagggagtaggtttttaagttttaaagcgaaataagagtgggtaaagatttttttttttttttttttttttttttaagaatttttttaataaggaaagttaacgtcgatcgcgttttgttcgttttttttttacgcggtagttttgatagagaagtgttaagagtgatagggataggtaggtgatattagattttttgcggcggtagtagtcgttgtagttacgacgcggttttttgagcgtatttttcgtaacgcgtatacgtatatttttcgggcggtcgaataggagtcgggttttgtcgtagtttagttttaggtatttaggcgagcgacggattagatttgcggtttcgcgtttttttgttggtttaatattttaaaattagaggcgggttttttggtgtcgagacgttatttcgtcgcggttttttttagtttttttcgttttcgtttttttttagattttttttcgggtgcgattgacgtggtttcgtattaattaggacgtttcgagtcgcggtggagggattgttttgtttgtatttattagtagtgcggggtcgggttattgtttcgtcgtgcgtattgggtttatataggtaagttttcgggaatttagtttttgtttagtttaaggcgattcggtttttagtacgaatttaaaggtgaagagatgaggttaggagtcgaaggtttgggagaagagagtggaatggttaagaagagaaaggtataaggattaataagatatttattttttgtgttttattatatttatttttaattttttattttatataaaaaggagatacgttatttaaaattagaaaatttgaaaaatagtaataaattattttttcgattttaaattttttaaatagtttgttaagtgaatgttgcgttaatttgaagaagttttaattgtaaagaagatagagttttgaaaaggtaggttaataaattagaaatcgagaagtaaatggattcgttaaaagaaaattattttgattttaaacgaataattgtttggtggtttattttggatttatataagaataaaaagtcgttttagattacgttttttgtgatgtttattagtttttagatagaaaatatataatagaagagaaattttaatttagcgtttttaaaatgttgaaagtttatttattttatttaacgttgattaagatatatattttagattttttaaattttttgtatattgtattaagttcgttttaattcgagagagttacgttttaaattcgatttttttgtttattttattattaattagatttaaatttataaagtttgtagaattaataattttgagttaattatatatgaaatatgttttaatgaatttttatataattaagaatgttgttaaataattaattttaaggataatttttaatagttattttttttttttagtgagtttaaggttgttttgagttattaaagtttaagtaggtagaaggggtgtgtgtgagttaagggcgaaaa

SEQ ID NO: 10 - DNA, 32001 bp, Homo sapiens
tatggattgtgtgattattaaatttggtattttagggggtatattttttttgagtaatttttataaatatgtttgtttgtaggatatttagattttttggtttggtagtaaagtaatataagaataattttgaatttgatgtttatttttgttttttttttaattttaggagttttttgaggtttggattaatttattgattaggaaatagtatttggaaaggttaaataaaatattatttttagggaaatagtatttggaaaggttaaataaaatatatttttttagtttttttaaattttttagaagatatattttttaaaaaataaattaagttagtaatatttaaattaaatttttgttttgtttataatataaaagatgataaaaaaattgttgggaaggtgagaaattaattttatttataattagaagtaaagtttttatttaaaaatgtaatattatttaaatttaatttgggaaataaaaaggatttaaaaaatagtttgttaaagttaatttgtaaataagtgtgttttttttttttttaagttgtattttaggtttagagtatatgtgtaggtttgttatgtaggtaaatttgttatagggatttgttgtatagattattttgttatttaggtattaagttttgtatttaatagttattttttttgattttttttttttttttatttgttattttttaataggttttagtgtttgttgtttttttttttgtatttatgagttttttttatttagtttttatttataagtgagaatatgtgttatttggttttttggttttgatttagtttgttaaggataatggtttttagttttatttatatttttgtaaaaggtatgattttattttttttttaattattttattttttttattatttttttttttttttttaattttgaattttattatgttagtttaattatttttttttttttttttttttttgtttatttgtatatagttaaaagatgttatgaatttttttttttaatttagtatatgtttattaaagatttaaaaatattatttatattatttagaatttagtttaagaaattattaaaaaataaagttattagaaagtaattgaattattttgttgagttataattttagattttgattttgttttttttttattttaggtaggttattttttttttttttttaaattgttttttttgtatttaataatatatttttgtggatttagaaagggtggagtatgaggaaaaggaatatgatatatgtattttagaggaaaataataaataaatattttaggatggaaaatattatttttatttttattgagttttttagagtttatttgatttgtgtaaattagaaattagtagaatgatattaatgaattaatgaaaagtagaatgagttattagttgtaataaaaagaataaagaattttaagaatatagttttaattatgtatggttgtggggagagaaaaataataaaatgtttttagtgaatatatttttgagagaagaaaggaaatatttaaggagaggataaaaagagtaaatattaaaaataggagtaagaattttattgttttttttagttgataaataaaaattgtatatatttattgtggataatatgatattttgaggattatgattatttttgatttataaattatatttaagaaaaagaaatttttaaaaagtttgggaatatatgaagttgaaagaatattaatatttagataaggatagtatatgataaattatttttgttttaatatttttttttaggaaatttaaatattttttagtgaagtattagttttttgaaattaagtatgagaaaaaaaattaaatttatttgtggaaaaaaagatatagttaaataaaaaagtggttgttataattttaagagtggtatgaataaaatgattaatatttttttaagtgatagtataaatattaaaagttttaataagtggaagtggttttgttatgataaaaggtgtggtatttgtataatttttagataagaataaagttatgatgttaagatagtagtagtattgtttgttatatgtgatatttgaaaaatatgataattattttaatttgtttaagtagtatttatggtgagggtgaaattttattaatattggttaatttatggtgttttaaaaaattagtaaggagataaattgatggattaaaagataaattatttataggtagataaatagaaggatagatagagttataattaaatatgtattttatttaggtagaaagataataattagtttttaagaagtgatgtgtttgttagaaaagttttgaatatagaattttttgattttgtttttaatttagtttttttaggtattatgttgtataattaggtgtaattttttaaaagtttttatgatagaattttttatttgttaaattaggttaataatatttttatttttttttagggtaaagatgtgaaatatttggagaattttggaaaatatgttttttattaattagagttttttgatgtgatattattttttttagtatttggagtttagttaatagatatatagtgtagttgtgaaattatgaagtatgagaatgtattattaagggattgtaggaggttttttattgaaaagtgtagttggttatatttttggaagtaatttaaatataggttgagggagaggagtattttttagattttttttagattttattttttatgaattttaattttttttttttatttagaaaaaataatgagatttatagtgtagagatagaaaataaggttttgtgtgtttttaaattttatttttaaaaatattatagtattttggatgagatagttttgaatttttgtaatagtataggtatgagagtttttattagaaaataggagattggattgatttttttattttttttttatgttttttaaaattgaaaagttatatatataaattatatttatttattttttttggaaaaggttaaaatgaatttaattttggattatttttaataatgggataaatttgaattgagaataatttttagaattagttttgtttttttgtgataaaatggatttgtagaaagttatttggtgtttttttttagttaatattttattataaataatgggtatgtaatttagtattgttttttataggttatgtttttggaattattatttttgtattttatttgtttgttgatatttttttatttaagatgttttttttagtataagaagttattttttttaaaattttaaatgattttattataataatagagttgttaattagatttaggtaagtaatgataataaaaatttgatttttatttagagtgtagtatggtttaatataataattagagttttaataggtttttttagattttatttttatttaatttgtatgtttttgtaatatagatgtttttattatttggtttttatttttatttttttttgtttttggaataaaattatttaaatttaatttagagattttatttttttttggaattattgggaaatagttttagtaaattatatttttgagattttatattaggtttagtttaaattgattatttaagtattaatttttttgtggtttaggaatatttttgagtttatttttttttttttaaattgtttaggataaatattggagtttggtttttttgtttttttatttaattattttttgtttttttttttttagtatttaaaatatttttgattttttttattttttaagaaatatatttgtttttttgtttttgtattatttttttgtttatgaaatattttataggtaagttttatattttttttttttagaggtttttggttttttggttttagttgttattggtttagtgtattagttaatattttggattttggagttatataaatttagatttaaatttttattatgttatttattgtttatgtgatttgaagtaatattttatttattgtggtttttagtagttataagtttgtgttttaattagttgggtgattttgggttagtgatataattatggtaaattttattgtttttatttgtaaaatgatagtatttattttgtagtgttggtataaggaataagtgtgattgttaatataaaagtgtttagtataatagttaaattaattaagtattttgtaaatattagtttttattattattattaatttaaatgattagatgtattttgtgtatattaggttttttgagtttattttgtttttaataaatattattatttttagtatgtggtttatattatattttattagttagaggatatgtgaagtttagagtggaaagttagggtagtaggaagtattgttatattttatatagttaaagttatttaaatatgtttgaatttgagttttgttgagtttttatttgtttttattttttttgtgtgttttagtttattaataaagtaggtttaatataaatatattaaaagtttaaatattgagattatgataatgaatatgagggttatgattataaaatattattgaattagagatttgttatgaaattatatggtgaagattataagggaggaatttgtatatatattgagtgttttgggattttaaagtgggaagagttagtgttttaattaaagagaaatttggggtagggaattaattataatattagttattttattgaatttaggtttgttttagttgatgtagttgttaatttttaatgttttttttttttttaattgtttttaatttatttttttagaaattgaaagtttattaaagaggatatttttttagagagttgttttagttattataagtttttgttagaaattttaagaaagtttataaggtatttttataaggtggtattgagtaagttagaagtattttaagtattaattattatgtaaataagggttttatttttagattttgttgtttgtggtggtggtgatgttggtgttttttttggaatttagtttaatttttaaaaaagtaaaaggagtataaatagtaatataaattattattatttatattaattaaaatagaagttttgaatgagtaaggagttagaggaggtaaaaattgggaattttgtatattaaaaggtttttataatttgaaaattaagattatgttggttaaataggttgttttaaaattagtatagtaattaaatttgtttgtaatgaatgtagatttaaatagtgatgttagatttgataaggatttgtaaattttaaaagagtgtaaaaagattatagaagaataatattatatttttgtatttatagaaatggttagtttaagagatgtatttagtttagggtggttgtaagttttattttttgaatttgttattagaagttaaaagaaattttgtataattgtttttgatggaaatataaattggttgatgtaaatgaaatatataaagtagttggtgttttatttatttttataattataaatgaaattaaatgattaaaaattatagattttggggattttttttttattgaggagtttatggaatttgttttttttagtattaataattgtgttgatttatttttttttgtttaattttgtatatattaaaattaggtggttatgaataaaatttagaaatataatttatattttaataaaatgattttaaaattattttattttttattgtggttttatttgttgttttataatgtaggtttttttgggtttttgtttagaatgattttgttaatgtagatgatagttagagttgaatggggaatttagaaattggggatttgggtttttgatgtaatttatatgttaatttattttattagttttttttttatttatagtttggtaaagaatatgggtggagttgttttgggtttatttgtatatatgtttaaattgttttgaaaaaggaagggtaagaaagagtggtatttaagttggaattaggtaggtattttagattaagagatgaattggaaagggaatatttgttagatattttgggtttgaaggtagtttgtgtaagtttttatatttttgagtgtgtgtatatagtggagagggtggagtttgttatttttaaatttgaaaagattgagagattttagagggtttagatgtgttaaaggttagagggattaatatataggttttattatggaaaggtggggaaaaggtttgaatagaaaattgttgtagaagggaagttattgagaggtaagggagtttttgaataattaaaaagttaagaataagtaaaaggaaggaggttgggtgggggataaaaaaaagtagttgatgtggtaattaagaatttggtgggagtttgggtaggttatttttttttttagattagagttttattagaaatttttttaagtgtttttttgtgttgttaaagatgataatagtaaattaataagtgtttgaaatgaaaggggatgttgattagtttttaggttatagattttttgttgttagttttttttgaatttttatagtgtgtttttgtattgttttttttaagaagagttattttttatttttatttttaggatgaaggtaagtgtttagttagtatatttattaaatgttagttttggttttagttttttgtttgtgtggaaagtttattgttatagtgtgtttagtttgttggaggggtagatagaaaaagtaagtttggtttggtgatttgtggggttatgtatttttagggttggtttggagttttttagagtttaatgtttttgggttagaattgtaaggttttggtttgagtaaagggtttgagttattgtagttgtgggagtgttttttttatttgaatgtatttatttataaataagtataaaatttttttaatagtagaggagaaagatttttgttttaaaattaaagttgggaattattggaaattttgttttgagtgtgagatattggtttgttatttttttaatttttatattttttttgtaatatgttttgatttaataatttttttagtgtttagtattgtttggatgttttaattgggtaatttattagtgagttaatataggtatttatatatttttttagtttaagtggttaagtattaattttgaaatgattataaaatattggaattggtaatgtatagtaattttaatttatatgtaaattaattggtttattttaaatgttttttttaaaaaaataattattgtattgtagtattggaggtatggattaaatttttagaatagataatttggaaataagatttggattaggaagataatttagaatagttaataaattaataatgtttgaggtagttaaatattgttagttattggtatttatatatttgtttgttgttagataaggagttggggaaattgtttgttagggttgagattataatttagagtgaagaaagtaaatggtagtatatagtttgttatagtgggttttgaaataatattgtattttttttaaattttgatttttgggtgatagggagttggtggaggttattttatatttgtttatggttttgttttaatttgattatgaaattgttgttttttttgagttttttaatttgattattattttaatggttttgttatttgttttaatatattggggggaggagtgtaattgagatttttattaaaaattatttgaatttatttagttagtattgttttatttaagtttagttttatgggttgtatttaattttttgtgttttttatatattaaaattagattattaaaatgttggtaggaaagggtgaaggaaatggtttaatgttttagtttattggaagattattatttttagatatagtttaaaattttgaggaaataaaaaggatatatgttttggggggaaaatgttttaatattttagaatgggggtattattttttttattttagagaatttgtattggagttgtttatgtaaaaatgtaatatttttgaaatttatagatatgtaaggttagtgtttttttttttttaggtttttagtttaggtgatttagttttaaaggagttagtatttttgatgttataattttgtttatatttgtagggtagagaattgtttgttttgtttggatgttttttttatttttttttaatttgaagtaattggaatttaaatatagttgttaaggtttgttttttttttattgttttgataagggaaaaatttgaaatttatgttttaaattagtttggtggtttgtagttttttagtattttgtttttatgattgtatgtttaatgtattttttggtgattttgggtattaattagttgtttaataggagtatgattaaaaatgtaaaagaaggattaggagtgtgaaatgtatgtttagttttttttatatatttgaggagggaatgagaattattttgtattttttatttttttaggagttatttgtattttttattagttgtttattttagttgtattggtgttgggtaaggtgaggatttaaaagtttagtgtagtgtttgtggtggttgggattggggttaattagtttttggtgggtgagattttagatagaaggggggtgagaggaatgtgagttttttgagttttttttttttagttttggtttgtaaatttttgaaatttgaaaggggagggagttgtatgtgtgtatttttgtgtttttttagtgtaatttttttttttttttttgtgtttttttgtggatttttgaatttttttgtttttggtttttttatttttttttaatttttttatgagattgtttatttttgttattagttgaaggtaaggttgttttgttatgagtgttttttaatttttataaaatgaaaagaaaaaaagggaggattattagtttattatttagaggaatggggaggttgtaaaaattgttgatgggtagaggtgaagatgttttttttggattgtattttttggtgttttgtaattagagtttagttgtgggatttgttgaagaaatttgatttttttgttttggtgagattttaaaaattagaaatagaaatttttagagttagagaggaaatataattaaatagtatgtgggtatttttttttttatttttttttttttaaataatattgttttgagtttttattgggtaaagagagaaagtttgagtttttatggatgttatgtggaggttagaaatggtttaaaatgtagatttttaattagttttttttgtggttgaagaggttaattttttttataaaatgagtttatttgttgattgttagttattttaaagtgaagggatttagtatttaaaataaattgagtaagtttgtttgtttgtttttattgttaatttaaatgaatttaaaatatggagtaatttaagaaaatatataatatgttttagatagtttttaaaagtagggaaagtttagtatttatatagtgattagggttagttttaagtgttaagtttttttaaatgtatttattttatgtatatttttttgagttattatatatttttaaaattgtgagtattggtatattgatttaggaagagtaatataatttttagagggaattttatttttaattagggattaaagagatgtttttttaatagtgggtttgagttttgtttttaagtaggaattaatattggtgggaaaatttgaatttaggagtaatggttgtgttttggtattttttaaaaatatatattaataggatgtttttgagattgaaaaaatattgttttatatgtttggtagaagtttttatatttggttttttaggtgaattatatttatagtttttttatttagaggtaggatagagttaaaatattttgtttattattaaaatatatatttttgtttaagttaagaaattagaaaattagggtttagaagtaaggtatattttttgagtgagaatatgttttgtaattttatatattttttgttttgtaggagtaaatgtggatttgagggaaatttttttttttatttttatttttattttgtgtaatttaatattatttttgttaggaattttaattttgttattttaaaaaatgagatatttgtgatttagggtgaatttgttgaatgtaggtatagtagaggaaattttagattttatgagtgtttgagttttgtttagtgtaaattttttgtgaatattgggttagtgtgtggttgtgtttatttgtgtgttgatatttttagtatgtttggtttatttgttttgattttgggtgtggtgttttagttaagttgggtttagtgttttggttttttttagttgataagtttagtttgtttgtttttggttgtggtttttttatttttttttattagtttattttatttttttagatttttttttatttatttttttttatttttattgtgtttatttttatttttgttttttattggttttttatttttttttttttgtagtttttttttgttgtgatttttttttttaattttgtaggtttgaaagaaggttatatatgtatgtttatatttatattttatatgttttgttttaaataattttatgaatattgttttttgttttgttttttgggttattttttttgttgtttttttttagtttgttttgatttgttttttaaaagtatgtttttgtttttttgttgttttggtgttttttttttgatttattagggttgttgggttggtgtagattgttttttttttttttttattttatttttttttttggtttttttttttatagtgggagtttgtgtttttgttttttggttggtttttaagtgttttgttaggttttttttttttttgtttttttggttttggtttttgattttttggtttgttggtatttgttttttttttttgttttgttttttgttgtttttgtttgttttttttggtgtttgtttgggtgttgtgtttgtttttggattgttagttgtgtagttgggtttggttggttgtttgtgtgttattgtgtagtggagtttggtggaatttttgttgatgttatgttattttttatatggagtaggagtagagggaagagagagggatgagagggagggagaggagagagagtgtgagattgagtgagaaagttggagaggagtagaaagaaattgttagtggtggttagattttggaggttttagtgtatttgtggatttttttggaatttggtatttttaggagttttgtagtttttttaggtttggtttttgggtgtttgttgtgtagttggaggtttggtttgttggaaattgttttgggaagtagtgggatgtggagatagtagtttttttttggtagttggtaagtggaggttatttattttgtagggatgtgagataatgtgagtttggaaatttgttttattttggagaatttttattgtaggtgatttgtggtttttggggttaagttttgtttaaggtaatgtagttggtaaatagattttgtaaagttttgttttttttgttttttgttatagatattaataatttatagggtgttgaagttgagagggaagttagattgtggttggtatttaaaatgaggtatttttttttaaattttggtgttaatattgtaggaataaatttttgggttaaggattagtatttttaagataaagggttgggtataaagttttagttattggaagattagttttttttttattgttatttattgggaaaaaaaagaaaagaaaaagattttattttaattggtagttagtgattttttaggtttaagtgaattatttgggagttaggtttggatgttaagtttttattatttttttggattgtaatttttttaaattgattattagttaattttaatttggtattttaggagatatattttaaatggatgtagagaattattttttagttggagattaagaaaaaaatttttgattttaaatttttgaaatatgttttttttttttagtttaattattttatttttttaagtaatttagaaattaaattattataaggtggtgtgatttttttttatttttttgtgtgagtattgttttattaaattaaatggaaaaaatttttattattataaatgtaaatattagaatttatatattttaaaatatttttatgaaaaattaatttgatttaaagaaatttttttgtatttgttttagtttattaattaaaattaaagatgtttttattatataaaatattattttggtagaaatttatttaaaatttaaatattaataatattaagaaaataaagtatataagtaaaataaattgaagatttttgttgatgtaatatgagtatataatattttaataattaaattttttttaaaaaattaaatagttattttatttgtggaatgttttattttaatttagtaaaattatatttaaattatttaggtgttttgttttttaagttaagtgtgtttgtttttaaatgtttttaaagtatttatattaattggttgtaaagaatgtatatatatggtaaaatatagaattgaattgagtagtattttaatttttttaaataattatttattataaattaatttattggttaattttataatttagtttatttaaaatatatgtttttgtgttgtttatttttaaattttttattaaagattttgttatggggtaataaagtgtatgaaaaggggggaaatgtgaaaggatttgggattatttgaattgtattttttttgtatttttagttttgtggtagttattagaaattattttttagtaaattgttttattttttagggtttgtttgtttgttttgttatggttttttgttttttgttagttgtgtagtgttttttgtgtgtttataatataaaatttaagttggttaaaataagagtttttggtatatatattttaattagaatatgaattttgggggtgagaattattttttattaggaaaagttttttattttaatttgtgagattagttattgaagttagttttgaagtttggtagttaaattttttatagaagatttgttttgatagggtaagtttaaggattagtaggtgggaattggaggtttttttttaaaaaattattttttttagttatttagatttagtttttttagtaggtttggttattaaatgaagtataaaaatgtaagttttaaggtttattttgattgtaaaataaatttttaagttataaggatatgtaggagtgagttaaggaatatgttttgattttttttttagtttttagagtggagttttatgagtttttgaagatttgttttgtattgttttgtttggtttttagtattgaagtatggggaagtggggggaagaatgtgtaataattgattgattttatattaagtaatgtaattttttttttttgtatattttattttttaaaaaaaataaataaataaaaattatttgtagttattatttgtagtgttttggttattagttaataatgtagttagtttagatatataaaaaaaaaagattattgaaatgatgatgatatgtaaattttttttgaaattattataagtaaatatttgaagtttggattaataaaattttatttgtgttattttatattgagttagtagaaagttgtgataatgaattttgtaatattttatgaatagatattttaattagggattaattttgtgattttattgtagaattattaaatttggagttgttaaattgttatttttgggtttatgggtttataaggattgaattggtagagtttttgtttgtgtttttgttagtgggtgggggaattgtttggttgtttttattttggatttttatgttatagtgttgggtagttttttttgtaggtagtgattttggttagaggttttttagggtttagttttttttaggagaggttgagatgtagggaaatggtatttaggttagaggtaggtttgtagttttttgttttgtttttgtgtttttgttaatttgataatgtttgtttttattttgatttttgtatttgtgtgaagtgggttttttggttgttggtgtattttggttagtgtggagagaggtaggtgttgagattgaaggggtttagggagttttggattttttttttttgtttttaaagtaattgtggtttttttatttatttggtggagttttttgagatttattttttttggtttgtttgtggtagagaagggggagtgtgttaaatgtttggtttgttgtgttgtggttgaaaatgtgaaaaagatttggtttgtttgggagagaaagggggagaattgggtagtagttatattagagttatttttttgtttttggtgggtagtaaattttttaagaatgtttgttttgttttttttagttttgtttagtttatttagtgttttttttttgtgattttaaattatattttagggtaattatttgtagtaagtaaataaatggttgggttagtatttttaggagaaagtgtggttaaatatggaaaagtggtttttgatggatgagaggtttgaatttagtttgtttttgaaatattttaggttaagagtttgtttgttttagaattatagaaaattgagggaaattgttgtttaggataggggtatgttggtgttgatgttttataaatgtttattgagttttaattaatggataagtattgaagggtggtttttgtatatagttttttaaagagaaaagttttttttatttatttatttttgttgttattgtgtttagatgagtttttaattttggtattgagatttttgaaagtaggtttatagtttttttagtatattgtggttttatagttttttaatttttgggtatttttgtggtaattttggagggagatttttttttgataaataaatgttttgggtttgaggttaggttggagatgttgttgtatagttagaggttgttaggttggaaaaatatgtttgaagtttagtatatagtaggtgtttaatagttagtgtaatgtagttttatttgagttttgtttatttgatggttgttgttttttatagtttttttttttttttgttttgtagataatggggaatggagattaattgttgtaaattggtgttggtgtgtgtgtaattaggtaagaattttttttttttgtttgggttattggatgggaggttgtgttatgtgagggtggtaagagggtattggttttgtggtgaggttttagtgaggggtgtttttttgaggggttagtttgggtaggaaggaaattagaattaaattgttagtggtttttttttgtggtggggtggtggattaggaagtagtggtgtgttgtgtattgaagttttttagtttattttttttggttggaattgttggtaattggggaggtgtagaaagagtatgttattttgttttgggttgttagagggtttgggggatggggatgttgttagtttttttttttaattgggtttttgttttttgttttttttttttttttggtttgttttgtttttttttttttttttgtttttggttttttttggttgtggtttgggatgtttttttttgtatgtggggtgggtgtgtgtgtggtttaggtgtgtagttggtggttgttgaatgttttttttttaaagattttgaaattaaaaaggttgagtttatggatttttttgagagttgaaaagaggtagttagtagtaagttttttttgtggtagtattttggtgttaatggtaaggttgggagggaagtgtaggttgtgtgttgggtatttgtttttgggattttgggttttgggtgaagtgtaagaaggtgaggttgttagatttgatgtgtttgttgtttgaatttagatattttgtttttgggtgggatgggaagtagttgttttagggatgttaatttttttttttaaattatattgtatttttgagatttaatattttttttttttttttgtttgttttttgtggtttgattttttgtgtatgttttagtaaattttggtgtttaggttggtgtggaaaagtggtttaatagtgatttttgttgtttgttatattttgttgtgtgtagtattattagggtttatttagttatttaggtttttagttatgttttatttagatttgtgggtgtgtggtttattgtgggaggtaagtaagggaaatttgagttggtgaaggtttgttttggttggttgggggaggggtggggggttgataatatttttgaagagttggagggtagttattgtgtttagtagtttagggtagaatggaggtttgtttttgttgatgtgaatttgtttgaagtattggttgttaggttttgggttttggtgatgttgttgtttgattggttggttttattttggaggaattgagggatattgttagaggaggtttataggtttatgtaaaaagttaaaaagtttttaatttatgttataggttttttttgaattgaaatttgttttatggggtggaggggggggtgtaagggatggaggagggaagatgtttttttttttaaatatatggaaaaaaattttttaaatttattgtttttttatttttttggttttgtagtaaataagtgtttagttttaggaggttattgatttttgataatgtgagtagataaagtttttttttttttatagtttttggtttttaattttttttttttggattaaagtgtaagaatataaatgtaatatgggatggaggggggtgatttgggattttggttaaaaaaataaattgtattattaagaagaaaataaaggttttgtattggagtttttttgtgaatttgagagaaaatgattatttgttgaaatgaagtgtttaaagtgatttagtgttttatgtttggatattgtattatattgttagttgttttgttgggttagttaaatgtttatttgtttgggattaattttatggggttaaatgggggtaatgtagagataatgttgtgtgatttttgttatttagattgtgttaaattttttttttgtttgataattggtagtaaaaataaattattagattgtagtatgtttgggatatggttaaaaattaagagtagtgatgatttttggggagaatgttttgtgtgggtttagttttggttttggttagattagaggagttttttaattttgttttgtgtggggtgggtttgtagttgttaagttgaggttgatattttttattgtgttgggagttagagagatgtaaaatgttttttttttttagtttttattttaggttttttagatatggggaatgtattttgaggataggtggagaagtttatggtaggatggggtttttgtaggtgagtaggaaatggttaagagtagaggagttttgtttgtgttagttataagttgtgtaggtgtttttggttgtttgtttttgataattagtatataaagaattagaaataatgaatgattgtttttttaattattatttttaggtttgtattgttttagtgtatgtgaaaggttttttttttatatttaatatgtttttttttattttttgattgaaaagaaaaattgttgtttaaatatgtttaatgttattaattaagaaaaggtatgtaatgggaagaaatgttgaaaattttgatttaattggtttttaaggaattagtagatgataaaaaaaaattatatgagtgggtaaagttatagtattgttgaaggatagagtatttatttttttttgattttaagttaatttatggaatatttaaagttttggttatagtttgtttgtaaaataaaaggatttattttttgtgtttttttaaagtttttttttgtttttaaagagaaaaaaagtttataatgatatatgatttttttaaaaggttgtgatagtttattatgttattttttttgtttttgtttttaatgttgtttaaaaatattatgtttttgttaaagattaaatgttttgtataggtagagtttatttttaagtagtttaggttttgttttttttttttagtgagttttattttttttggtatttattgggtggatgtttagtttggatagaattttgaaatgggggtagtatgagagtgattggagatttttaaaagttagaggtttgagagagggtggatgtagttagtagaagatggtgtagaagttagttgagaatgattttttagagtaaagagatttttttttggttttttttgttttgggggttttgaaaggaatttataaaatggtttttatttttaggaggaggatggattgatttttttttgttattggtttaaaaagttttagggtggtggttttgggttttgtgttgaaattggattgtattgtagtttttttggatttgatgtttggttttgtgttttgataaggggtgggtattttttttggttttttttaggaatgtattaattgttaaatagttttggtttagtggatgggttgaaagtgtttgatttaagttgttggtgtgtatagattttttttttttgggaggtgggttttatggtttgttgtggtatttttagttgtgatatatatttttatatgtggtagtagtttggttttaattttttttgaaggatttgggttaattttggtggttttggtggttgtagatttttttttgttgttttgtttttgtgttttttatttaattagtgaatgtttgtggagtatatattatgtggatttttaatgtattttttgaaagtaaataatatagttttttttgttgttatgaagggattttaattttaatatggatattagtgagattagtttagattgtttttagtaaaatgtaaaatggtggtgtgtggggtggtgattaaggttttgagttttgttagaaagaaggggatgtgtagagaaaggtggagaattttagttgtggttagtgtggaagggataggtgtttgttgaagggggtatgaggtttgaggaaaaagtaatgaaataggggtaaggagagttttttatttttttttttttgtttgatttttgttattttatttttttttttttttttttattttttgtgttaattaaatttgtagtttatttgaaaggtgttttgttgtgttgtggttttttatttttaggggaaattgtattagttgtttgaaagtagttagtttttgtggatttttgtttgtaaaagtggtttttataggttgtgttttttgttgttgatttggtatataaagttttttaaggttggtttggttgttattttttattgtttgttgttaatatatgtagtagttgttagagtggtttgggggaaaaggaaatgtataatgaaagtttatttgtgagtaggaatatattaatggaataatttgatgtttttttaattttatgtaaaaagttttgttgtttttttaatattgattgaatgggtaattaatggttttttatttaggtgaatattttgtaatttaagataggtaaaagataataagtttaaggtagaagataaaaggtttaattgtagtggtgtttgtttgttttttattttttagggtttttgattaggaaagtttttttttagaggagaaaaaggtaggagtgggagaatatatatttattattttggggttagattttattgtagtatttgattatttagtttagttttttgttattttgtttttttatttttagtttttttttttgtatttttttttttttttaatttttttaggatgattttttattattattgttattatggttttaataatttttttttttaaattttatattttttattttagtaattaatgaggttgttttttgatttaggaggagattttttttttttagaatttaatgtgtagagtttttgagaattaaagtagttggtaggggaggaagaaattaatagaaagggagagagtatatagaattgtgtgtgtatgttaaagagtgattaggaatgatagagttaatttttttgtgaggatttgatgggaagagtgtttaagattttattagtatgtttttaataggttgatattttaatttaaatttttagaagtaatatattatttgggttattataatgaggtgggtttttttttttttgttagttgatagtttttaaaatattattttgttagggaaataaaagttttattttagattataggtgggtatttttggatttaggtgatttatggttattatgataattaatgttgaatgttagttattagtatgtttgggagagagaaaatagaaagaagggagagtaaaagaaatagaaaagggagatggatataagttggagagggaagaaaagagaaaaagaggaagatagatgagtgtttaatttaattgttgtttaaaaaagtggtgggggggtgggattttatttagttttttgttattttttttttttttgatttggatatttatgtttaattttatattttatttttttttttttttttttaaatatatgtgttatattattttttttattttatttagtttggtaagtagttgttttttggagatttagtgatatttaggaaaattgtggtagtaatatgtaaatgtgaggaagtattaatagtatgtttgttgagtgattttagtaaatgtttttttttttaatttttttttttttttttttttaggttattgtgaggtggtaatttttattgttatttgaatattgtttttttaggtagttattttaaattttaaatggttgagtagttagagttgtgggttggaaaaatgggtattatttgtagggatttagagagggtggttgttgtttaatatatttatagatttttaatttagaaaataattttttttttttgataagttagagttttttaaattttatttaggaaatggggaaaaggatagttatagtgaagtttttaatttttgggttatttggttttatagttatgaggggtggtgggtagtggattgtttttagtttggtttgtatgtagagaaaagttagatattggagggggtggggtattttttgggtaggatgtaaggtttttatttgatttttgtgttttattaggagtttatatatttatgtttattatgtggttttaagttgagtttaggtgggttttgtttttgagttagtttgggtagggtaggatttttatttgtttaaggtttaatagtttagggagatgtttaattaagttattttttgggtgaattttgaagatagattttttttaaaagttagagattatttggttgagttttaggttagattgatatggagagtttggtggtatagtttaattgtttattgttatggttagagggattttgtataattaatattgaagagtgtgaaattaaataagattttaagattggtaattggtggtaaatattagtataaaatatggttgattttatgttatatattttttttttttagggtttttttttgaaagaataagtaagaaattttaattgagataatttttgatgttttttagatttaaaattttatgttggtattgggttttttttttttgttttatgtgagttatgtagtatttttagtttttttattaggattttattaatgttttttgtattggaaatttttgtgttagaggttgaatttatagtaatttttaaaattaattaagaagaatttagttagaggttatagtaatgttggaattataaaatgtataagatttatttttttttggttttttttttatttatgttgtttatgtttgtgtatttataagttttatgtatattaaatttttaaaattaattattattatgttatagagtttttattggatagtgttttttagtttttattatatatttttttttttttatgtagatttattatgttggtgttttgttatatagggggtttgagaagaatgttatttaattgttgttgttgtgagtgtgtaaagtgattaggagattaggagaatgttgaaatttttgttggaaaaatgtaaagaaaatttttattttgagttagttgtttatagagttagtgtgtgtgtgtgtgtgtgtgtttgtaatataaaatggatgtgaatatatatatataaatagatatggttttgtttttattttaatttgaattatttagataattgtttttatttattatttgattttaatgggtttatataaattaggatattttatttttttaggtatttaggttgttgttgatttttagtgtttttaatattttgtatatgttggtattatgaggagtagttatgtgtttttgggttttttaattattttggaggttgattgaggttttttatatatgtatatttgttgtgatgaaagttttattggtagagtggagttattagagtttttattaaaattttgtgggtttatgagagatgggtttagaaatttatatggttttgtggggttttttggttttttaaaataaggtattaatatttaagtttttaaaaatatttgtagttttggggtttgaattttgaaaaataaggagtgaggggttgtgtatattaattatagtggagattttttttattttttaatgtgatggagtttttttatgaaatgaagttttaaggggtatggtattgtggggattatagttattttgaggtttaaaagaagaaattggaatatgattagtaaatatatttagtagaaaagagttggatttttattgatttagttataggttattggttggtagtgtaatgggaggaaatatttattttatatatatattttatgattttgggggaattagaggaaatttaataagaaaatggttagaaatatttaaaatttttatttaaaagatttaagtaaattagagttttattagattaaaaattattataaatgtaagagtattgtttttagtgaaatgttgtggggtttgagaaggagattttttgttaaatttttgggataaaatgtgttatttaagtattagataatgagtagaatgtaaattaatttaattttttttattaataggttgttagtgtaatgtgtataatttagtgataagattgtaggatttaatatagttggatgtatgagttttagttaatgtagatttgttatatgaggatgtgttttattttgagtaggtgtttgtatgtgtggaatggggtaaagtggaataaaaggttaaaagtagaaatgttgatttaaagtttattatgaagaaattttttttttgtagttaaattatttttaaagtgggatgatattggtgaagaaagattgaaaaataatttttatgtgtgtttttggattgtaagtttaaaatggggaggagttgtagatagggtttgggggtggttagggtaaaggagagatatataagttgtaaatatatttgtagtttgttttatttattttgttttatattgaataagttttttaattttgtgaataaggataaggagggagtgttttaaagatattttatgttggtattgtaaattattgattgtaatgttaaataaatatatatttagagatgataatattaattttatagtaaaataattgtttatgtagaaatttagaggagattagtttgttttttttagttgatttatgttgggggataaaaggatttttaaaaattattttgaatatgtttggatttttttttttaatttttttggaaattaaatttgtttggaaatagtgttataaagagttgatgtttttaaaggtgattttttttgttttatataaataaggttttgtttttgttagttgagtgtagttttaggttttttgtttttagtttatatatattttttttgtttgtttggattttaatggtttaagatagttttgagtttattgggaaaagaaaatgattgttaaaaattatttttgaaattggttatttggtaatatttttaattgtatggaaatttattaaggtatattttatatataattagtttaaggttgttgattttataggttttatggatttaaatttgattgataataaagtaaataagagagttgaatttaaagtgtggtttttttgggttaggatgagtttaatatagtgtataaggaatttgaaagatttaggatatgtgttttaattaatgttaagtagaatggataagtttttagtattttgaaaatgttgggttagggttttttttttattgtgtgttttttgtttggggattaataagtattatagagaatgtgatttgaggtgattttttatttttgtataaatttagagtgaattattaaatagttgtttgtttaaagttaaggtaatttttttttgatgggtttatttgttttttgatttttaatttattagtttgtttttttagggttttgttttttttgtaattaaagtttttttagattagtgtagtatttatttgataggttgtttggaaaatttaagattggagaggtgatttgttgttgttttttaaattttttagttttaagtaatgtgttttttttttatatggggtgggggattggaaatggatgtagtgagatataaagagtgggtgttttgttgatttttgtatttttttttttttgattattttattttttttttttaagtttttgatttttagttttatttttttatttttgggtttgtattaaaagttggattgttttgggttgggtaggagttgaatttttgggagtttgtttgtgtagatttagtgtgtatggtgaggtagtagtttggttttgtattgttgataggtgtaggtaggatagtttttttattgtggtttggggtgttttgattggtgtggagttatgttagttgtatttggagaagggtttgggaggaggtggaggtggagagggttggggagggttgtggtggagtgatgttttggtattaggaagtttgtttttggttttaagatgttaggttaatagggaagtgtggagttgtagatttggtttgttgtttgtttgggtgtttggagttgagttgtggtaaggtttggtttttgtttgattgtttgaggggtgtgtgtgtgtgtgttgtggagggtgtgtttagagggttgtgttgtggttgtagtggttgttgttgttgtaggggatttaatattatttatttgtttttgttatttttgatatttttttgttagggttgttgtgtggggggggggtgggtagagtgtggttggtgttagttttttttattggaggggtttttgggggagggagggagagaagaagggggtttttgtttatttttgttttgttttggagtttggaagtttgttttttaaagatgttttgagtggtgtttttttgtttatattttatgtttttgtttgtttgttgattttttgtttttggatttttttgtttgagttttttggaggagatgggggtagtttggtttgagaatttggtgggggttgtgttttttggttttttttgtagtggggaaattttgtgtttagagtgtgatttggagtgggtagtggtggttatgggggtttggtggggtagtagttaaggattagtagagtgttgtgtttttttgtttatgaattgtatgaaaggtttgttttatttggagtattgagtagtggggattaagttgttggttgtttttttatttttttgttattatttttagttgttagttatggttttggttttggtttttggttagttttggttgttggatttttttaagtataggttggaggtgtatattatttttgatatttttagtttggaggttgtaggtaaggtgttgtgttgttttgtagatatttttgtttagttgttttgtgttatttgtttttttttgttttaaggaagttagtttttttggggggaggtgtggtgggagtggttgtttgtttggttttttgtagaatttttgggagttggaattttgattattttgtatttttttagtttttttttgattggtttggtttttggggtgttaagggtgtgagtaattttgttgttttttttatttgtattttggttttttttttgttttttgggttataaaaattttagtattttgatttgaggatttttagaggttgttgatttttgtttttgttttttttttggtttttagtttttgaggagttttatttgttaggaaattgtttgaaattatttagaaatgttttttgtgaagaggtattttttttttttttttgggaaagggttggtgaattttggtgtttaattgaatttttatatttttttttagtttttttaaattgtatggaaatttgagttttttgtgagggggaggggggtttgtaaattatgtgtgtgtgtgtgttttaggagatttggtgtgtttgtgtagaggtgtataaatatatttgaaagtataggttataaaagtgaatgtgttgttgtagtgagataaatatgtaaataaaatgtgtggtgttgggggaggggaggaaatggggtgtggatatttatatttgtgtttgtatattttataggtgtagtgttttttgtggtttggagttgttgtgtgtatttttttttggtgttaggtagtttagtttttttatggtttttgttgttggtttagttggtgtttgtgttgtaggtgggtatgttgatgggaaagtgtgtgtgttttgtttttagagaaagataaaagttagtaggggaagaatgaggatgtgggtgttgaggatttgtttaagaagaagtggtaaaggtggtagtggatttattttattagttagtagttttaggagttggaggttattttttagaggaattgttatttggatatgtttatatgtgaagaaattgttgtgtggattaattttatggaagtttgagtttgggtaggagttagtatggagtttgggagggatggggggaggatgttgtggaggtataggttaagtagattaggagagaatgtggaaggtagtgttgtttgggagggtgttggtggggtgtagttttgtaaaggtagaaggttttgtggtggtttggttgtgagattatagttttttttttgaggttgataggattgttgttttggtttaggtttttagagtggtattggtttattgttttgttattttgtgattttatgagttgggttgtatgggtaattttttgtataggatattgtgtttttggtttgtagttgttagagtagagttaataaaatttttattaggttaagagttgtgaataggttttaatttgtgagtttttaataaggaaaatttgttagagatatggaagagttggttttttttgggaaatttttgttttggttttggtttagtttttttttttttgggtttgtgttttttatattttttttatggttgttttggttatttaggttttttttatatattttattttttagttttgtgatttttgggagtaaagttttaatatataattattagtttttttagaaggagaaagaaaaaaagaagaaagatttttttgtttggtttatttatttttttttaggagttgaattttggaaattgaaatttatatttttttttttaaattataattatagttttgtaaaaagggtttattttaattttgtagtaaatttgtattttatggattggtaaaaatgagtttaaataaataatttaatagtaatgttttggtttatgttggttggtggaagattttaaatttgttaggattttggaagtagaaaatagaattaagtaaattaagtggtatttagaggttttgttgttaaaaaaaaaaaattaagtgttttgggtagaaaaaataaagtttttggttagagtagagtaaataaaaagaagaaaataatgataaaaagaataaagattaaaatgtttttttaaattagagggaatgaagatattttttgggtggtatttgtgtaaggtatgaggttatgttggtggataaaaggttgggaagaagttgaaaatggttttagtttaattgtttagagttagagttgggttttgggtggtgtggttttgagtaaggttagttttttattagtttttttgtatattaagggaatgggttttttatgtattttttttgtttgagtaaagtttagatggtttagggtagaaatggtaagtaattaaagatagagtttatgggttttttgggattttttgaaaatgtttttttattttgtttgttattttgtagttttattttagtgttttgtagttgtggtgttgggttttttttgtagttgtttttttttttagggtggttgtttgttgagttaagtgggagtgaggtgtgttttttatagtagttgggtgtaaagaggaagggggataaaaaggaaattaagaatgaaaggaaaaagagaaaaagtggattatatggttgggtttggtggagatgtgtaatgtgaaatattattggtgttagtttggatattttaggttaggtttttttttaatatataaaagttgttgtttggggtgatagggaggtttgatgtggattgggattggggttgtggttgggttattggatatgggtggaagttggttggtttgggtggttgtttgtaaagttaaatgatttggttgggtttggtgtgtggataggtttgtggtgggtttagggtaaagaagaggtagagtgaaagaagggggaatttttaaaattattttttttgggtttttggagtttaatatgttaagtttttggagttaatgagttgatgaagaggtggttttttgttttttatttggttgttttgttaggtgagaaagagtgttggtggtttagtttttgttaagggagtatgtattagggggtgggggatgatagtggaggttagggaaggaagggaggaattgtgtgggagaaagagtgattttttagtgtttttttagttttttttttttatttgtgggtttgtggttttggaatggaagtaagtttgtaaggtgttttgggaagggttggaaaagtttgttgttttgtgtttgttttatattaagtgtttttggatttggagaaatgtttggttgagtgattaaattgtttgtaggtttttatgtgtttggttgaggtttgtggtgtagttttgagttttagtttgtaggttagagtagattaggttttttgtgtttggtggagatttgggttagtaattgaaagttggttttggtattttggtgtgtagggtggtgtagtgaagtgaggttagggtgtgtgagtgtgttagtgtgtgtgttgggggaaggtgggggttggtttttgatggaagttttagtaatttgtattgtggtatttgtttgtttttttgttttaattgtttttaggtttggtttaagaattgttgggttaaatggagaaagagggagtgtaattagtaggttgagttatgtaagaatggttttgggttgtagtttaatgggtttatgtagttttatgatgatatgtatttaggttatttttataataattgggttgttaagggttttatatttgtttttttatttattaagagtttttttttttttaattttatgaatgttaattttttgttattatagagtatgttttttttatttaattttattttgtttatgagtatgttgtttagtatggtgtttttagtagtgataggtgttttgggttttagttttaatagtttgaataatttgaataatttgagtagtttgttgttgaattttgtggtgttgatgtttgtttgtttttatgtgttgttgatttttttgtatgtttatagggatatgtgtaatttgagtttggttagtttgagattgaaagtaaagtagtattttagttttggttatgttagtgtgtagaatttggtttttaatttgagtgtttgttagtatgtagtggattggtttgtgtgagttgtatttatagtgttgggattttaggattttgttggatggggtaattttgtttttgaaagattgggaattatgttagaaggttgtgggtattaaagaaagggagagaaagagaagttatatagagaaaaggaaattattgaattaaagagagagtttttttgattttaaagggatgtttttagtgtttgatattttttattataagtatttttaatagttgtaaggatatatatataaataaatgtttgattggatatgatattttaatattattataagtttgttattttttaagtttagtattgttaatatttaaatgattgaaaggatgtatatatattgaaatgttaaattaattttataaaagtagttgttagtaatattataatagtgtttttaaaggttaggttttaaaataaagtatgttatatagaagtgattaggattttttgtttgtgagtaagggagtgtatatattaaatgttatattgtatgtttttaatatattattattattataaaaaatgtgtgaatattagttttagaatagtttttttggtggatgtaatgatgtttttgaaattgttatgtataatttattttgtgtataatattttgtataatattattgttttattttttagtaaatatgaaataaatgtgttttattttatgggagtaaaatatattgtatataaattggtttggattttttttttttttttttgttattaatttggttaggatattttagttattgttttttaaataaattagttttttttgtttgtttagttaaatatataaggtagtagtttttatttaaatttggtagaaataaatgatagttatttattagaaattaaaaagaaaaaaaaaggtatttttgggggggaaaagggttataaaatttaattttgtttttttaatttttttttggtttaaatttagaggattttattatggttagtaaataatatgaaaaagaaaaaagaagaaagaaatttagtaagtttattagtttaaaatgatttttaagtttatttttttatggggaaatttatatttttagtaaattgttttggagaaatatttgtgtatgtatatatgtatagtttatatgtattttttttaggaggaatatatttataataaatttatagggaaatatttttagtttaaaatatttaggtttttatgtttatttttaggtttaagtagagagattttttatgttatattgtattattatttttaaattttttggagatattaaaagaaataaagatgatttttaataattatagttttttagttttttaaagaatttaggggttgagaggttagagtggagttttttgagttttgttgagtaatatgtagttgaggtaaaggttatgtttttggtgttttgttttaaataatattgatttattaattttaaatttgtttgtttttgaaattatataggattatagtttgtaaattgtaggataatgaagtaaattaagatgaattatagttttggttttttttgttattttttgatatttaaatagggaatgagtttggtgtgagtgtttaaatgaattttaagtatttgatttttttttatttgtgatttttagttttaaaaaaatgtgaaatttgattttataataaatagaaataaatattatttagttttagagaatttatttttatggtgttaggagggttgttgtggaggtggggggagggatgtgttgagattttttgttatgtttgttaattttttgtataattaaagtgggtgagaataaatattatgttggggaatttagagtaaaaagtaattgttgattttttggagttgataatattattgtttttttgttttagt

SEQ ID NO: 11 - DNA, 12001 bp, Homo sapiens
tatggattgtgtgattattaaatttggtattttagggggtatattttttttgagtaatttttataaatatgtttgtttgtaggatatttagattttttggtttggtagtaaagtaatataagaataattttgaatttgatgtttatttttgttttttttttaattttaggagttttttgaggtttggattaatttattgattaggaaatagtatttggaaaggttaaataaaatattatttttagggaaatagtatttggaaaggttaaataaaatatatttttttagtttttttaaattttttagaagatatattttttaaaaaataaattaagttagtaatatttaaattaaatttttgttttgtttataatataaaagatgataaaaaaattgttgggaaggtgagaaattaattttatttataattagaagtaaagtttttatttaaaaatgtaatattatttaaatttaatttgggaaataaaaaggatttaaaaaatagtttgttaaagttaatttgtaaataagtgtgttttttttttttttaagttgtattttaggtttagagtatatgtgtaggtttgttatgtaggtaaatttgttatagggatttgttgtatagattattttgttatttaggtattaagttttgtatttaatagttattttttttgattttttttttttttttatttgttattttttaataggttttagtgtttgttgtttttttttttgtatttatgagttttttttatttagtttttatttataagtgagaatatgtgttatttggttttttggttttgatttagtttgttaaggataatggtttttagttttatttatatttttgtaaaaggtatgattttattttttttttaattattttattttttttattatttttttttttttttttaattttgaattttattatgttagtttaattatttttttttttttttttttttttgtttatttgtatatagttaaaagatgttatgaatttttttttttaatttagtatatgtttattaaagatttaaaaatattatttatattatttagaatttagtttaagaaattattaaaaaataaagttattagaaagtaattgaattattttgttgagttataattttagattttgattttgttttttttttattttaggtaggttattttttttttttttttaaattgttttttttgtatttaataatatatttttgtggatttagaaagggtggagtatgaggaaaaggaatatgatatatgtattttagaggaaaataataaataaatattttaggatggaaaatattatttttatttttattgagttttttagagtttatttgatttgtgtaaattagaaattagtagaatgatattaatgaattaatgaaaagtagaatgagttattagttgtaataaaaagaataaagaattttaagaatatagttttaattatgtatggttgtggggagagaaaaataataaaatgtttttagtgaatatatttttgagagaagaaaggaaatatttaaggagaggataaaaagagtaaatattaaaaataggagtaagaattttattgttttttttagttgataaataaaaattgtatatatttattgtggataatatgatattttgaggattatgattatttttgatttataaattatatttaagaaaaagaaatttttaaaaagtttgggaatatatgaagttgaaagaatattaatatttagataaggatagtatatgataaattatttttgttttaatatttttttttaggaaatttaaatattttttagtgaagtattagttttttgaaattaagtatgagaaaaaaaattaaatttatttgtggaaaaaaagatatagttaaataaaaaagtggttgttataattttaagagtggtatgaataaaatgattaatatttttttaagtgatagtataaatattaaaagttttaataagtggaagtggttttgttatgataaaaggtgtggtatttgtataatttttagataagaataaagttatgatgttaagatagtagtagtattgtttgttatatgtgatatttgaaaaatatgataattattttaatttgtttaagtagtatttatggtgagggtgaaattttattaatattggttaatttatggtgttttaaaaaattagtaaggagataaattgatggattaaaagataaattatttataggtagataaatagaaggatagatagagttataattaaatatgtattttatttaggtagaaagataataattagtttttaagaagtgatgtgtttgttagaaaagttttgaatatagaattttttgattttgtttttaatttagtttttttaggtattatgttgtataattaggtgtaattttttaaaagtttttatgatagaattttttatttgttaaattaggttaataatatttttatttttttttagggtaaagatgtgaaatatttggagaattttggaaaatatgttttttattaattagagttttttgatgtgatattattttttttagtatttggagtttagttaatagatatatagtgtagttgtgaaattatgaagtatgagaatgtattattaagggattgtaggaggttttttattgaaaagtgtagttggttatatttttggaagtaatttaaatataggttgagggagaggagtattttttagattttttttagattttattttttatgaattttaattttttttttttatttagaaaaaataatgagatttatagtgtagagatagaaaataaggttttgtgtgtttttaaattttatttttaaaaatattatagtattttggatgagatagttttgaatttttgtaatagtataggtatgagagtttttattagaaaataggagattggattgatttttttattttttttttatgttttttaaaattgaaaagttatatatataaattatatttatttattttttttggaaaaggttaaaatgaatttaattttggattatttttaataatgggataaatttgaattgagaataatttttagaattagttttgtttttttgtgataaaatggatttgtagaaagttatttggtgtttttttttagttaatattttattataaataatgggtatgtaatttagtattgttttttataggttatgtttttggaattattatttttgtattttatttgtttgttgatatttttttatttaagatgttttttttagtataagaagttattttttttaaaattttaaatgattttattataataatagagttgttaattagatttaggtaagtaatgataataaaaatttgatttttatttagagtgtagtatggtttaatataataattagagttttaataggtttttttagattttatttttatttaatttgtatgtttttgtaatatagatgtttttattatttggtttttatttttatttttttttgtttttggaataaaattatttaaatttaatttagagattttatttttttttggaattattgggaaatagttttagtaaattatatttttgagattttatattaggtttagtttaaattgattatttaagtattaatttttttgtggtttaggaatatttttgagtttatttttttttttttaaattgtttaggataaatattggagtttggtttttttgtttttttatttaattattttttgtttttttttttttagtatttaaaatatttttgattttttttattttttaagaaatatatttgtttttttgtttttgtattatttttttgtttatgaaatattttataggtaagttttatattttttttttttagaggtttttggttttttggttttagttgttattggtttagtgtattagttaatattttggattttggagttatataaatttagatttaaatttttattatgttatttattgtttatgtgatttgaagtaatattttatttattgtggtttttagtagttataagtttgtgttttaattagttgggtgattttgggttagtgatataattatggtaaattttattgtttttatttgtaaaatgatagtatttattttgtagtgttggtataaggaataagtgtgattgttaatataaaagtgtttagtataatagttaaattaattaagtattttgtaaatattagtttttattattattattaatttaaatgattagatgtattttgtgtatattaggttttttgagtttattttgtttttaataaatattattatttttagtatgtggtttatattatattttattagttagaggatatgtgaagtttagagtggaaagttagggtagtaggaagtattgttatattttatatagttaaagttatttaaatatgtttgaatttgagttttgttgagtttttatttgtttttattttttttgtgtgttttagtttattaataaagtaggtttaatataaatatattaaaagtttaaatattgagattatgataatgaatatgagggttatgattataaaatattattgaattagagatttgttatgaaattatatggtgaagattataagggaggaatttgtatatatattgagtgttttgggattttaaagtgggaagagttagtgttttaattaaagagaaatttggggtagggaattaattataatattagttattttattgaatttaggtttgttttagttgatgtagttgttaatttttaatgttttttttttttttaattgtttttaatttatttttttagaaattgaaagtttattaaagaggatatttttttagagagttgttttagttattataagtttttgttagaaattttaagaaagtttataaggtatttttataaggtggtattgagtaagttagaagtattttaagtattaattattatgtaaataagggttttatttttagattttgttgtttgtggtggtggtgatgttggtgttttttttggaatttagtttaatttttaaaaaagtaaaaggagtataaatagtaatataaattattattatttatattaattaaaatagaagttttgaatgagtaaggagttagaggaggtaaaaattgggaattttgtatattaaaaggtttttataatttgaaaattaagattatgttggttaaataggttgttttaaaattagtatagtaattaaatttgtttgtaatgaatgtagatttaaatagtgatgttagatttgataaggatttgtaaattttaaaagagtgtaaaaagattatagaagaataatattatatttttgtatttatagaaatggttagtttaagagatgtatttagtttagggtggttgtaagttttattttttgaatttgttattagaagttaaaagaaattttgtataattgtttttgatggaaatataaattggttgatgtaaatgaaatatataaagtagttggtgttttatttatttttataattataaatgaaattaaatgattaaaaattatagattttggggattttttttttattgaggagtttatggaatttgttttttttagtattaataattgtgttgatttatttttttttgtttaattttgtatatattaaaattaggtggttatgaataaaatttagaaatataatttatattttaataaaatgattttaaaattattttattttttattgtggttttatttgttgttttataatgtaggtttttttgggtttttgtttagaatgattttgttaatgtagatgatagttagagttgaatggggaatttagaaattggggatttgggtttttgatgtaatttatatgttaatttattttattagttttttttttatttatagtttggtaaagaatatgggtggagttgttttgggtttatttgtatatatgtttaaattgttttgaaaaaggaagggtaagaaagagtggtatttaagttggaattaggtaggtattttagattaagagatgaattggaaagggaatatttgttagatattttgggtttgaaggtagtttgtgtaagtttttatatttttgagtgtgtgtatatagtggagagggtggagtttgttatttttaaatttgaaaagattgagagattttagagggtttagatgtgttaaaggttagagggattaatatataggttttattatggaaaggtggggaaaaggtttgaatagaaaattgttgtagaagggaagttattgagaggtaagggagtttttgaataattaaaaagttaagaataagtaaaaggaaggaggttgggtgggggataaaaaaaagtagttgatgtggtaattaagaatttggtgggagtttgggtaggttatttttttttttagattagagttttattagaaatttttttaagtgtttttttgtgttgttaaagatgataatagtaaattaataagtgtttgaaatgaaaggggatgttgattagtttttaggttatagattttttgttgttagttttttttgaatttttatagtgtgtttttgtattgttttttttaagaagagttattttttatttttatttttaggatgaaggtaagtgtttagttagtatatttattaaatgttagttttggttttagttttttgtttgtgtggaaagtttattgttatagtgtgtttagtttgttggaggggtagatagaaaaagtaagtttggtttggtgatttgtggggttatgtatttttagggttggtttggagttttttagagtttaatgtttttgggttagaattgtaaggttttggtttgagtaaagggtttgagttattgtagttgtgggagtgttttttttatttgaatgtatttatttataaataagtataaaatttttttaatagtagaggagaaagatttttgttttaaaattaaagttgggaattattggaaattttgttttgagtgtgagatattggtttgttatttttttaatttttatattttttttgtaatatgttttgatttaataatttttttagtgtttagtattgtttggatgttttaattgggtaatttattagtgagttaatataggtatttatatatttttttagtttaagtggttaagtattaattttgaaatgattataaaatattggaattggtaatgtatagtaattttaatttatatgtaaattaattggtttattttaaatgttttttttaaaaaaataattattgtattgtagtattggaggtatggattaaatttttagaatagataatttggaaataagatttggattaggaagataatttagaatagttaataaattaataatgtttgaggtagttaaatattgttagttattggtatttatatatttgtttgttgttagataaggagttggggaaattgtttgttagggttgagattataatttagagtgaagaaagtaaatggtagtatatagtttgttatagtgggttttgaaataatattgtattttttttaaattttgatttttgggtgatagggagttggtggaggttattttatatttgtttatggttttgttttaatttgattatgaaattgttgttttttttgagttttttaatttgattattattttaatggttttgttatttgttttaatatattggggggaggagtgtaattgagatttttattaaaaattatttgaatttatttagttagtattgttttatttaagtttagttttatgggttgtatttaattttttgtgttttttatatattaaaattagattattaaaatgttggtaggaaagggtgaaggaaatggtttaatgttttagtttattggaagattattatttttagatatagtttaaaattttgaggaaataaaaaggatatatgttttggggggaaaatgttttaatattttagaatgggggtattattttttttattttagagaatttgtattggagttgtttatgtaaaaatgtaatatttttgaaatttatagatatgtaaggttagtgtttttttttttttaggtttttagtttaggtgatttagttttaaaggagttagtatttttgatgttataattttgtttatatttgtagggtagagaattgtttgttttgtttggatgttttttttatttttttttaatttgaagtaattggaatttaaatatagttgttaaggtttgttttttttttattgttttgataagggaaaaatttgaaatttatgttttaaattagtttggtggtttgtagttttttagtattttgtttttatgattgtatgtttaatgtattttttggtgattttgggtattaattagttgtttaataggagtatgattaaaaatgtaaaagaaggattaggagtgtgaaatgtatgtttagttttttttatatatttgaggagggaatgagaattattttgtattttttatttttttaggagttatttgtattttttattagttgtttattttagttgtattggtgttgggtaaggtgaggatttaaaagtttagtgtagtgtttgtggtggttgggattggggttaattagtttttggtgggtgagattttagatagaaggggggtgagaggaatgtgagttttttgagttttttttttttagttttggtttgtaaatttttgaaatttgaaaggggagggagttgtatgtgtgtatttttgtgtttttttagtgtaatttttttttttttttttgtgtttttttgtggatttttgaatttttttgtttttggtttttttatttttttttaatttttttatgagattgtttatttttgttattagttgaaggtaaggttgttttgttatgagtgttttttaatttttataaaatgaaaagaaaaaaagggaggattattagtttattatttagaggaatggggaggttgtaaaaattgttgatgggtagaggtgaagatgttttttttggattgtattttttggtgttttgtaattagagtttagttgtgggatttgttgaagaaatttgatttttttgttttggtgagattttaaaaattagaaatagaaatttttagagttagagaggaaatataattaaatagtatgtgggtatttttttttttatttttttttttttaaataatattgttttgagtttttattgggtaaagagagaaagtttgagtttttatggatgttatgtggaggttagaaatggtttaaaatgtagatttttaattagttttttttgtggttgaagaggttaattttttttataaaatgagtttatttgttgattgttagttattttaaagtgaagggatttagtatttaaaataaattgagtaagtttgtttgtttgtttttattgttaatttaaatgaatttaaaatatggagtaatttaagaaaatatataatatgttttagatagtttttaaaagtagggaaagtttagtatttatatagtgattagggttagttttaagtgttaagtttttttaaatgtatttattttatgtatatttttttgagttattatatatttttaaaattgtgagtattggtatattgatttaggaagagtaatataatttttagagggaattttatttttaattagggattaaagagatgtttttttaatagtgggtttgagttttgtttttaagtaggaattaatattggtgggaaaatttgaatttaggagtaatggttgtgttttggtattttttaaaaatatatattaataggatgtttttgagattgaaaaaatattgttttatatgtttggtagaagtttttatatttggttttttaggtgaattatatttatagtttttttatttagaggtaggatagagttaaaatattttgtttattattaaaatatatatttttgtttaagttaagaaattagaaaattagggtttagaagtaaggtatattttttgagtgagaatatgttttgtaattttatatattttttgttttgtaggagtaaatgtggatttgagggaaatttttttttttatttttatttttattttgtgtaatttaatattatttttgttaggaattttaattttgttattttaaaaaatgagatatttgtgatttagggtgaatttgttgaatgtaggtatagtagaggaaattttagattttatgagtgtttgagttttgtttagtgtaaattttttgtgaatattgggttagtgtgtggttgtgtttatttgtgtgttgatatttttagtatgtttggtttatttgttttgattttgggtgtggtgttttagttaagttgggtttagtgttttggttttttttagttgataagtttagtttgtttgtttttggttgtggtttttttatttttttttattagtttattttatttttttagatttttttttatttatttttttttatttttattgtgtttatttttatttttgttttttattggttttttatttttttttttttgtagtttttttttgttgtgatttttttttttaattttgtaggtttgaaagaaggttatatatgtatgtttatatttatattttatatgttttgttttaaataattttatgaatattgttttttgttttgttttttgggttattttttttgttgtttttttttagtttgttttgatttgttttttaaaagtatgtttttgtttttttgttgttttggtgttttttttttgatttattagggttgttgggttggtgtagattgttttttttttttttttattttatttttttttttggtttttttttttatagtgggagtttgtgtttttgttttttggttggtttttaagtgttttgttaggttttttttttttttgtttttttggttttggtttttgattttttggtttgttggtatttgttttttttttttgttttgttttttgttgtttttgtttgttttttttggtgtttgtttgggtgttgtgtttgtttttggattgttagttgtgtagttgggtttggttggttgtttgtgtgttattgtgtagtggagtttggtggaatttttgttgatgttatgttattttttatatggagtaggagtagagggaagagagagggatgagagggagggagaggagagagagtgtgagattgagtgagaaagttggagaggagtagaaagaaattgttagtggtggttagattttggaggttttagtgtatttgtggatttttttggaatttggtatttttaggagttttgtagtttttttaggtttggtttttgggtgtttgttgtgtagttggaggtttggtttgttggaaattgttttgggaagtagtgggatgtggagatagtagtttttttttggtagttggtaagtggaggttatttattttgtagggatgtgagataatgtgagtttggaaatttgttttattttggagaatttttattgtaggtgatttgtggtttttggggttaagttttgtttaaggtaatgtagttggtaaatagattttgtaaagttttgttttttttgttttttgttatagatattaataatttatagggtgttgaagttgagagggaagttagattgtggttggtatttaaaatgaggtatttttttttaaattttggtgttaatattgtaggaataaatttttgggttaaggattagtatttttaagataaagggttgggtataaagttttagttattggaagattagttttttttttattgttatttattgggaaaaaaaagaaaagaaaaagattttattttaattggtagttagtgattttttaggtttaagtgaattatttgggagttaggtttggatgttaagtttttattatttttttggattgtaatttttttaaattgattattagttaattttaatttggtat

SEQ ID NO: 12 - DNA, 4001 bp, Homo sapiens
tttttgtttttagtttatatatattttttttgtttgtttggattttaatggtttaagatagttttgagtttattgggaaaagaaaatgattgttaaaaattatttttgaaattggttatttggtaatatttttaattgtatggaaatttattaaggtatattttatatataattagtttaaggttgttgattttataggttttatggatttaaatttgattgataataaagtaaataagagagttgaatttaaagtgtggtttttttgggttaggatgagtttaatatagtgtataaggaatttgaaagatttaggatatgtgttttaattaatgttaagtagaatggataagtttttagtattttgaaaatgttgggttagggttttttttttattgtgtgttttttgtttggggattaataagtattatagagaatgtgatttgaggtgattttttatttttgtataaatttagagtgaattattaaatagttgtttgtttaaagttaaggtaatttttttttgatgggtttatttgttttttgatttttaatttattagtttgtttttttagggttttgttttttttgtaattaaagtttttttagattagtgtagtatttatttgataggttgtttggaaaatttaagattggagaggtgatttgttgttgttttttaaattttttagttttaagtaatgtgttttttttttatatggggtgggggattggaaatggatgtagtgagatataaagagtgggtgttttgttgatttttgtatttttttttttttgattattttattttttttttttaagtttttgatttttagttttatttttttatttttgggtttgtattaaaagttggattgttttgggttgggtaggagttgaatttttgggagtttgtttgtgtagatttagtgtgtatggtgaggtagtagtttggttttgtattgttgataggtgtaggtaggatagtttttttattgtggtttggggtgttttgattggtgtggagttatgttagttgtatttggagaagggtttgggaggaggtggaggtggagagggttggggagggttgtggtggagtgatgttttggtattaggaagtttgtttttggttttaagatgttaggttaatagggaagtgtggagttgtagatttggtttgttgtttgtttgggtgtttggagttgagttgtggtaaggtttggtttttgtttgattgtttgaggggtgtgtgtgtgtgtgttgtggagggtgtgtttagagggttgtgttgtggttgtagtggttgttgttgttgtaggggatttaatattatttatttgtttttgttatttttgatatttttttgttagggttgttgtgtggggggggggtgggtagagtgtggttggtgttagttttttttattggaggggtttttgggggagggagggagagaagaagggggtttttgtttatttttgttttgttttggagtttggaagtttgttttttaaagatgttttgagtggtgtttttttgtttatattttatgtttttgtttgtttgttgattttttgtttttggatttttttgtttgagttttttggaggagatgggggtagtttggtttgagaatttggtgggggttgtgttttttggttttttttgtagtggggaaattttgtgtttagagtgtgatttggagtgggtagtggtggttatgggggtttggtggggtagtagttaaggattagtagagtgttgtgtttttttgtttatgaattgtatgaaaggtttgttttatttggagtattgagtagtggggattaagttgttggttgtttttttatttttttgttattatttttagttgttagttatggttttggttttggtttttggttagttttggttgttggatttttttaagtataggttggaggtgtatattatttttgatatttttagtttggaggttgtaggtaaggtgttgtgttgttttgtagatatttttgtttagttgttttgtgttatttgtttttttttgttttaaggaagttagtttttttggggggaggtgtggtgggagtggttgtttgtttggttttttgtagaatttttgggagttggaattttgattattttgtatttttttagtttttttttgattggtttggtttttggggtgttaagggtgtgagtaattttgttgttttttttatttgtattttggttttttttttgttttttgggttataaaaattttagtattttgatttgaggatttttagaggttgttgatttttgtttttgttttttttttggtttttagtttttgaggagttttatttgttaggaaattgtttgaaattatttagaaatgttttttgtgaagaggtattttttttttttttttgggaaagggttggtgaattttggtgtttaattgaatttttatatttttttttagtttttttaaattgtatggaaatttgagttttttgtgagggggaggggggtttgtaaattatgtgtgtgtgtgtgttttaggagatttggtgtgtttgtgtagaggtgtataaatatatttgaaagtataggttataaaagtgaatgtgttgttgtagtgagataaatatgtaaataaaatgtgtggtgttgggggaggggaggaaatggggtgtggatatttatatttgtgtttgtatattttataggtgtagtgttttttgtggtttggagttgttgtgtgtatttttttttggtgttaggtagtttagtttttttatggtttttgttgttggtttagttggtgtttgtgttgtaggtgggtatgttgatgggaaagtgtgtgtgttttgtttttagagaaagataaaagttagtaggggaagaatgaggatgtgggtgttgaggatttgtttaagaagaagtggtaaaggtggtagtggatttattttattagttagtagttttaggagttggaggttattttttagaggaattgttatttggatatgtttatatgtgaagaaattgttgtgtggattaattttatggaagtttgagtttgggtaggagttagtatggagtttgggagggatggggggaggatgttgtggaggtataggttaagtagattaggagagaatgtggaaggtagtgttgtttgggagggtgttggtggggtgtagttttgtaaaggtagaaggttttgtggtggtttggttgtgagattatagttttttttttgaggttgataggattgttgttttggtttaggtttttagagtggtattggtttattgttttgttattttgtgattttatgagttgggttgtatgggtaattttttgtataggatattgtgtttttggtttgtagttgttagagtagagttaataaaatttttattaggttaagagttgtgaataggttttaatttgtgagtttttaataaggaaaatttgttagagatatggaagagttggttttttttgggaaatttttgttttggttttggtttagtttttttttttttgggtttgtgttttttatattttttttatggttgttttggttatttaggttttttttatatattttattttttagttttgtgatttttgggagtaaagttttaatatataattattagtttttttagaaggagaaagaaaaaaagaagaaagatttttttgtttggtttatttatttttttttaggagttgaattttggaaattgaaatttatatttttttttttaaattataattatagttttgtaaaaagggtttattttaattttgtagtaaatttgtattttatggattggtaaaaatgagtttaaataaataatttaatagtaatgttttggtttatgttggttggtggaagattttaaatttgttaggattttggaagtagaaaatagaattaagtaaattaagtggtatttagaggttttgttgttaaaaaaaaaaaattaagtgttttg

SEQ ID NO: 13 - DNA, 32001 bp, Homo sapiens
attaaggtgaaaaaataatgatattgttggttttagaaaattggtggttattttttgttttaagttttttagtgtggtgtttgtttttgtttattttggttgtgtggggggttgataagtataataaaagattttagtatatttttttttttatttttataatgatttttttagtgttatgaggatgaattttttgggattaagtggtatttgtttttatttgttatgaaattaaattttatatttttttaaagttgaaaattgtggataaagaaggattgggtgtttaaagtttatttaaatatttatattgaatttattttttgtttagatgttagaggatggtagggagggttagggttgtaatttattttgatttgttttattgttttgtagtttgtaaattataattttgtataattttaggaataagtaggtttagaattaatgggttaatattatttaaaataaaatattgggagtatgatttttgttttaattatatattgtttgataagatttaggaaattttattttaattttttaatttttgagttttttgagaaattgaagggttgtagttattagaaattatttttgttttttttaatgtttttaaaggatttggaaatagtaatgtaatataatatgaaggatttttttatttaagtttgaagataaatgtggaagtttaaatattttgaattggagatgtttttttgtaaatttattatagatgtattttttttgagagaaatgtatataaattatatatgtatatatgtataaatatttttttagaataatttgttagaggtgtaggtttttttgtaaaggagtaaatttgagagttattttaagttgatggatttgttaaattttttttttttttttttttttttatattatttgttagttataatggaattttttaggtttaagttaaagaaaaattggagagataaaattagattttgtagttttttttttttttgggaatgtttttttttttttttttagtttttgatgaatggttattatttatttttattaaatttaaataaggattgttgttttgtatgtttaattaggtaggtagagggaattggtttgtttaggaagtagtgattgagatgttttggttaagttagtgatagaggaggggagaaagaatttagattaatttgtatgtagtatattttatttttatgaaataaaatatatttgttttatatttgttgaaaagtaaaataataatattgtatgaaatgttatatatagggtaggttgtatatagtagttttagaaatattattgtatttattagagaaattattttaaaattgatatttatatattttttataataataataatatgttagaaatatatagtgtggtatttagtatatatatttttttgtttgtaagtgaaaaattttaattgtttttgtataatatgttttattttaaagtttaatttttaaaaatattgttgtgatattattaataattgtttttataaaattaatttgatattttgatatatatatatttttttagttatttaaatgttaataatgttaaatttaaaaaataataagtttatagtaatgttaaaatgttatatttagttaaatatttgtttgtgtatgtgtttttgtaattgttagaaatatttgtagtgaaagatgttagatattgaggatatttttttgaaattaaaggagttttttttttgatttagtggtttttttttttttatatagtttttttttttttttttttttttagtgtttatgattttttagtataatttttagttttttaagggtggagttgttttatttggtaaggttttaggattttggtgttgtgggtgtggtttatatgggttggtttattgtatattggtaagtatttaggttggaggttgggttttgtatgttggtgtagttgaagttggagtgttgttttgtttttagttttaggttggttaggtttgagttatatgtgtttttataaatatatggaggagttggtggtgtgtaaggataggtaggtgttggtattgtggaatttagtgatgggttatttaggttgtttaagttatttaggttgttgagattggagtttgggatgtttgttattgttgagggtattatgttggatgatatgtttatggatgagatagagttgggtggggaaaatatgttttgtgatgatagggggttgatgtttatagagttgaagaaggggaagtttttggtggatagggaggtggatgtaaggtttttggtggtttagttgttgtaggaatagtttgggtatatgttgttgtagggttgtatgagtttattgaattgtggtttgaagttatttttgtatagtttggtttgttggttgtgttttttttttttttatttggtttgatgatttttgaattaaatttgggggtggttggggtaagggagtaaatagatgttatagtgtagattattaaaatttttattggaggttaatttttgtttttttttgatatatatgttagtgtatttatatattttggttttgttttattgtattgttttgtatattaagatattagggttagtttttagttattggtttgggtttttattaagtgtaggagatttggtttgttttggtttgtgagttgggatttggagttatgttataaattttagttgaatgtatggagatttgtggatggtttgattatttagttaggtgtttttttaggtttaaaaatatttaatgtaaaataaatgtggggtagtaggtttttttaattttttttggggtattttgtaaatttgtttttattttaaagttatagatttatggatgaggagaaggggttggaagggtattagaggattgtttttttttttatgtaattttttttttttttttttgatttttattgttgttttttattttttggtatgtgtttttttaatagggattaggttgttaatatttttttttgtttagtaaaataattaaataaagagtaaaagattatttttttgttagtttgttaattttaggagtttggtatattaaattttgggaatttggaaagggtagttttggagattttttttttttttgttttgttttttttttattttaagtttattataggtttgtttgtgtgttaggtttagttgggttgtttggttttgtaggtggttatttaggttggttggtttttatttgtgtttggtggtttagttgtaattttgattttaatttatattgggtttttttgttgttttagatggtggtttttgtgtattggagagaggtttggtttgagatatttgagttgatattagtgatgttttatattatatatttttgttgggtttagttgtgtaatttgttttttttttttttttttttatttttgattttttttttatttttttttttttttgtatttgattgttataaaaagtatgttttatttttatttggtttgataagtagttgttttggaaggagaggtagttgtaaggagagtttagtgttgtggttataaagtattagggtggagttgtggaatagtgggtggggtgggagggtgtttttgaaggattttagaaaatttatagattttgtttttaattatttgttatttttattttaggttatttaaattttgtttaggtgagaagagtatgtgagaggtttgtttttttgatgtgtaagagagttaatgaaagattgattttgtttaaaattatgttgtttaggatttagttttggttttggatagttaaattaaaattatttttaatttttttttggttttttatttattagtatagttttatgttttgtataaatgttatttagagagtgtttttattttttttgatttgggagagtattttggtttttattttttttattgttgtttttttttttttgtttgttttgttttaattgggggttttattttttttatttagagtatttaattttttttttttaatagtaaagtttttggatgttgtttgatttgtttgattttgttttttgtttttagaattttaataaatttggaattttttattgattagtataaattaggatgttgttattgggttatttatttgagtttatttttgttaatttataaagtatagatttgttataaagttaaggtaagttttttttataaaattatgattataatttagaagagggggtgtgagttttaatttttagagtttaatttttgagagaagataaataaattaagtagaaaagttttttttttttttttttttttttttttaagaggattagtagttgtgtattaaaattttgtttttggagattataaaattaggaaatagggtgtgtgggagagatttgaatggttgaaataattgtaaagaaggtgtaagaagtgtgagtttaggagggaaaaagttgggttagggttgggataaaggttttttagggagggttaatttttttgtgtttttggtgggttttttttgttaaaggtttataggttggagtttgtttgtggtttttggtttggtagggattttattagttttgttttggtaattgtaagttaggaatataatgttttgtgtaggggattgtttatgtagtttagtttgtgagattgtgggatggtggggtagtgagttggtgttgttttgggagtttgagttagggtggtagttttgttggttttggagagggaattgtaattttgtaattaggttgttgtgaggttttttgtttttgtaaagttgtgttttattggtgtttttttaggtggtgttgttttttatatttttttttggtttatttggtttgtatttttataatattttttttttattttttttagattttgtgttggtttttatttggatttgggtttttgtaaggttggtttatatagtgatttttttgtgtgtggatatgtttgggtagtggtttttttggaaagtggtttttagtttttggagttgttggttggtaaagtgagtttgttgttgtttttgttgtttttttttagatgggtttttggtgtttatgtttttattttttttttgttggtttttatttttttttgaaaatgaaatatatatatttttttgttagtatgtttatttgtaatgtggatgttaattggattggtggtagaagttgtggaagagttgggttgtttggtgttggaggagggtgtgtgtggtggttttgggttgtgaggagtgttgtgtttgtggggtgtgtaggtgtaagtgtgggtgtttgtgttttattttttttttttttttagtgttgtatgttttatttatatgtttattttattgtagtggtatatttatttttatagtttgtgtttttaagtatatttatatatttttgtgtagatatattaaattttttgggatgtgtatatgtgtgtggtttatagattttttttttttttgtagaaagtttagatttttatgtggtttgggaaggttaggaaaagatgtggggatttggttgggtattgaagtttgttggtttttttttaaaaaaaaaaaaaaaatgtttttttgtgaagggtatttttgagtggttttaggtaattttttaatgagtggagttttttgggagttgaaagttgagaggaaaatagggatagaggttggtggtttttgaaggtttttgaattaagatgttgggatttttgtgatttaggaaatagaagggaggttagggtatgaatagagagggtggtagaattgtttgtgtttttagtgttttaggagttgggttggttgagggagaattaaagggatgtggggtagttaaaattttggtttttggaagttttgtggggagttaggtgaatgattatttttattatgtttttttttggaggggttgatttttttggggtgagagggagtgggtggtgtagagtagttgagtgggaatgtttgtagggtggtgtggtgttttatttgtggtttttgggttggaggtgttggagatggtgtgtatttttagtttgtgtttggaggagtttagtgattggggttgattgggagttagaattgaagttatggttaatggttggggatggtgataggaagatgaggagatggttgatagtttggtttttgttgtttggtgttttaagtgaagtgggttttttatgtagtttatggatgagggagtgtgatgttttattagtttttggttattgttttgttgagtttttgtagttgttgttgtttgttttgggttgtgttttaggtgtggagtttttttgttgtggggagagttaggggatgtaatttttgttgagtttttaagttaagttgtttttgttttttttggaaggtttaagtgaaaaagtttggagatggaaagttagtgggtaaatgaagatatgggatgtgggtagaagggtattatttagagtgtttttagggagtaggtttttaagttttaaagtgaaataagagtgggtaaagatttttttttttttttttttttttttttaagaatttttttaataaggaaagttaatgttgattgtgttttgtttgttttttttttatgtggtagttttgatagagaagtgttaagagtgatagggataggtaggtgatattagattttttgtggtggtagtagttgttgtagttatgatgtggttttttgagtgtattttttgtaatgtgtatatgtatattttttgggtggttgaataggagttgggttttgttgtagtttagttttaggtatttaggtgagtgatggattagatttgtggttttgtgtttttttgttggtttaatattttaaaattagaggtgggttttttggtgttgagatgttattttgttgtggttttttttagttttttttgtttttgtttttttttagatttttttttgggtgtgattgatgtggttttgtattaattaggatgttttgagttgtggtggagggattgttttgtttgtatttattagtagtgtggggttgggttattgttttgttgtgtgtattgggtttatataggtaagtttttgggaatttagtttttgtttagtttaaggtgatttggtttttagtatgaatttaaaggtgaagagatgaggttaggagttgaaggtttgggagaagagagtggaatggttaagaagagaaaggtataaggattaataagatatttattttttgtgttttattatatttatttttaattttttattttatataaaaaggagatatgttatttaaaattagaaaatttgaaaaatagtaataaattatttttttgattttaaattttttaaatagtttgttaagtgaatgttgtgttaatttgaagaagttttaattgtaaagaagatagagttttgaaaaggtaggttaataaattagaaattgagaagtaaatggatttgttaaaagaaaattattttgattttaaatgaataattgtttggtggtttattttggatttatataagaataaaaagttgttttagattatgttttttgtgatgtttattagtttttagatagaaaatatataatagaagagaaattttaatttagtgtttttaaaatgttgaaagtttatttattttatttaatgttgattaagatatatattttagattttttaaattttttgtatattgtattaagtttgttttaatttgagagagttatgttttaaatttgatttttttgtttattttattattaattagatttaaatttataaagtttgtagaattaataattttgagttaattatatatgaaatatgttttaatgaatttttatataattaagaatgttgttaaataattaattttaaggataatttttaatagttattttttttttttagtgagtttaaggttgttttgagttattaaagtttaagtaggtagaaggggtgtgtgtgagttaagggtgaaaagtttagaattgtgtttaattagtaaaagtaaaattttatttatataaaataaaaaaaattatttttggagatattaattttttatagtattgtttttaagtaaatttaatttttaaagaaattaaagaaagaaatttaaatatatttaaaataatttttgaaagtttttttgttttttagtataggttagttggagaggataaattaattttttttgggtttttgtatgggtgattgttttattatggagttagtgttattatttttgaatgtgtatttgtttgatattatagttaatgatttgtaatgttagtatgaagtatttttaaaatattttttttttgtttttgtttataagattgggaaatttatttgatgtggaataaagtggatgaagtagattataaatatatttgtaatttatgtgttttttttttgttttgattatttttaaattttatttgtaatttttttttattttaaatttgtagtttaaagatgtatatgagaattgttttttagtttttttttattagtattattttattttaagaataatttagttgtaagggaggaatttttttatagtaagttttaaattagtatttttgtttttaattttttattttattttattttattttatatatatagatatttgtttagagtaaaatatatttttatgtgataggtttgtattagttgaggtttatatatttagttatattaggttttgtaattttattattaaattatatatattatattagtagtttgttggtaaagaaggttaaattaatttatattttgtttattatttggtgtttaaatgatgtattttattttggagatttggtggagaattttttttttagattttatagtgttttattgaagataatgtttttatatttgtagtggtttttaatttgataagattttaatttgtttaagttttttaaataagggttttaaatgtttttagttgtttttttattgaattttttttaatttttttaagattataaagtatatgtgtaaagtaaatatttttttttattgtattgttagttgatgatttataattaagttaataagaatttagtttttttttgttgaatgtgtttattaattatattttagtttttttttttaaattttagaatagttgtggtttttataatattatgttttttaaagttttattttatgaagggattttattatattaaagaatgaaaaaaatttttattgtagttagtatatatagttttttattttttgttttttaagatttaaattttagagttgtaaatatttttggaagtttgggtgttaatgttttattttagaaagttgagaagttttatagagttatatagatttttaaatttattttttataaatttatagaattttgataaaagttttggtggttttattttattgatggaatttttattatgataaatatatatgtatgaaggattttaattagtttttaaagtggttgaaaaatttaagggtatgtgattgttttttatagtgttaatgtgtgtgagatgttggaagtattggggattagtagtagtttagatgtttaaaaagataaggtgttttaatttgtgtggatttattgaagttaagtggtgaataaagataattatttagataatttagattaaagtaaaagtaaaattatatttatttgtatatatatatttatatttattttatattatagatatatatatgtatatatatattggttttgtaaataattgatttaaagtgaggattttttttgtatttttttagtaggagttttaatatttttttaattttttaattattttatatatttatagtagtggtgattgggtgatattttttttaggttttttgtgtggtaggatattaatatgataagtttgtatggggaaaaggaggtatgtggtgggaattaagaaatattgtttagtgaaaattttgtggtatggtggtggttgattttggagatttaatgtatataagatttgtgggtgtataggtataggtagtatggatgagaaaggggttagaagaaaataaattttatgtattttgtgattttagtattattgtgatttttggttaagttttttttaattggttttagaaattattatgagtttagtttttaatatagaaatttttaatatggagaatattggtgggattttggtagggaaattagaggtgttgtatggtttatgtggggtaaagaaggaaagtttagtgttggtgtgaggttttgagtttgggagatattaggggttgttttgattggggttttttgtttatttttttaaagaaagattttagaggagggaaatgtgtgatatggggttagttgtgttttgtgttggtatttgttattgattattagttttaaagttttatttaattttatattttttagtgttagttgtgtaaagtttttttggttatggtagtgagtggttgggttgtgttgttaaattttttgtattaatttggtttgggatttaattaagtgatttttgatttttggaaagagtttgtttttagagtttatttagaagatggtttaattagatatttttttgagttgttaggttttagatgggtgggagttttgttttgtttaagttagtttaaggatgaggtttgtttggatttagtttggagttatgtgatgggtgtgagtgtgtgagtttttggtaaggtgtagaggttagatggagattttgtattttgtttgagaagtgttttattttttttaatatttggtttttttttgtatataaattaagttgaaaatagtttattatttattattttttatagttatggaattaaataatttagaaattaaaagttttattgtagttgtttttttttttattttttaaatggaatttaaaaagttttggtttgttaaaaggggaagattattttttgaattggaagtttgtagatatattgagtaatagttattttttttgggtttttgtaaatggtatttatttttttaatttatagttttagttgtttaattatttgagatttggggtaattatttgggggaatagtgtttagatggtagtgggagttattattttatagtggtttggggaagagaagagaaagagattagaggagggggtatttgttaaaattatttaatgaatatgttgttaatgtttttttatatttgtatgttattgttatagtttttttaggtgttattgagtttttagaaagtaattatttgttgaattaagtaaaataaggagaatggtatagtatatgtgtttggagaaggggaaggaagggtggaatatgaaattgagtatagatatttaggttaggaaagaaggaagtggtaaggggttaaatgaagttttatttttttgttatttttttaaataatagttggattaaatatttatttgtttttttttttttttttttttttttttttttagtttatgtttattttttttttttattttttttgtttttttttttttttgtttttttttttttagatatgttggtagttaatatttagtattagttgttatggtgattataaattatttaaatttaaaaatatttatttataatttgagatgaagtttttatttttttagtgaaataatattttaaaagttgttagttgataaaaaaaaaggaatttattttattgtagtaatttaagtaatatattatttttaaaggtttaaattaaaatgttagtttgttaaaaatatgttggtagagttttggatattttttttgttagatttttataaagaagttgattttgttatttttggttgttttttaatatatatatataattttgtatgttttttttttttttattaattttttttttttttattaattattttagtttttaaagattttatgtattgggttttaaaagaaaagaatttttttttggattagaaaatagttttattggttgttgaagtgaaagatgtggggtttagggggaaaggttattaggattataatggtggtggtggtaggaggttattttagaggagttaagaagaaaaaaaaatgtagggagaaggattggaggtggaaagatagagtaatagaaaattgagttgggtggttaggtgttgtggtgaagtttagttttgaaatgataggtatatatttttttatttttgttttttttttttttgagagaaaatttttttagttagagattttggggggtaggaggtgggtaaatgttgttgtagttgggttttttgttttttattttgggtttgttgttttttgtttattttggattatagggtatttgtttagatgaagagttattaattatttatttagttaatattaggaagatgataaagttttttatataggattaagaagatattagattgttttattagtatatttttgtttatgaataagtttttgttatatattttttttttttttgagttgttttaataattgttgtatatattagtagtgggtggtgaggaataatagttgaattagttttaagaaattttgtgtattgagttagtagtgaggaatgtgatttgtgaagattatttttgtgggtagggatttgtagggattgattatttttggataattggtataattttttttgggggtgaaaaattataatgtggtggggtattttttaagtgagttgtagatttgattggtgtggggggtgggggaggggaggggagaatgggatggtggaggttgggtggaggaaagaaaatggaaaattttttttatttttattttgttgttttttttttaagttttatgttttttttggtaagtatttgttttttttgtgttagttatagttagagttttttatttttttttatatatttttttttttttgataaggtttaggattttggttattattttatgtattattattttgtgttttgttagagatggtttgggttgattttgttggtgtttatgttaggattaaaatttttttatgatggtgaggaaaattgtattatttgtttttagggggtatattaggagtttatgtagtatatgttttgtaaatatttgttgattgaatgagaggtgtgggggtggggtggtggagaggggtttgtggttgttaaggttgttagggttaatttaggttttttgaagaaggttgggattgagttgttgttgtgtgtgaaggtgtgtgttgtggttgggggtgttataatgggttatggagtttattttttagagggaggaagtttgtgtatattagtgatttgggttgaatatttttagtttatttattgggttaaagttatttaataattaatgtgtttttgggggaggttgggggaagtatttgttttttgttgggatgtaaagttaggtgttaggtttaaaggggttgtagtgtagtttgattttagtatggaatttagagttgttgttttgaaattttttaagttagtgatagaggagggttagtttgttttttttttgagggtgaagattattttatgagttttttttaggatttttaaagtaagaaaagttaaagaaaggtttttttgttttagggggttgtttttagttggtttttatattattttttgttagttgtgtttatttttttttaaatttttggtttttaggggtttttagttgtttttgtgttatttttgttttggggttttatttaggttgggtatttgtttaatggatattaaggagaatgggatttattagggaaggaaggtagagtttggattgtttagaggtggattttgtttatatagaatgtttagtttttaatgaggatatggtatttttgggtggtgttgggggtagaggtggagagggtagtgtaatagattattatggttttttgaagaagttatatgttattgtgaattttttttttttttaaaagtaaagaaaaattttaaaaaaatataagaaataaatttttttgttttataagtaggttgtggttaggattttggatattttataagttaatttaaaattagggaaggataggtgttttattttttagtagtgttatagttttgtttatttgtgtgatttttttttgttgtttattagttttttaaaagttaattaaattaagatttttagtatttttttttattatatgtttttttttaattaatggtattaaatgtgtttaggtagtaatttttttttttggttaaaaagtagaaaaagatatattgagtgtaggggaagagttttttatgtgtattaaaataatgtgggtttgaaagtaatggttaagaaagtaattatttattatttttagttttttatgtgttagttattaaaagtgaatgattaggggtgtttgtgtggtttgtgattggtgtaagtagaatttttttgtttttagttgttttttgtttatttatgaggattttattttattgtaggtttttttatttgtttttagaatgtattttttatgtttaggaaatttggggtagggattgggggaaggagatattttgtgtttttttggtttttagtataataagaaatgttagttttggtttggtgattgtgagtttgttttgtgtgaagtgagattggggagtttttttagtttggttggagttagggttgagtttgtgtaaagtattttttttagaagttattgttgtttttgatttttaattatattttaaatatattatggtttaataatttatttttattattgattattaaatagaagaagaatttaatataatttaaatgatagaaattatgtgatgttatttttgtattgtttttatttaattttatggggttaattttggataagtgagtgtttaattggtttagtagggtgattggtggtgtagtgtagtgtttgggtgtgaagtattggattgttttagatgttttattttaataaatgattatttttttttagatttatggggaaattttaatgtaagatttttgttttttttttagtaatatggtttgtttttttgattggggttttaaattgtttttttttattttatattatatttgtatttttatattttaatttggaaagagggggttaggggttgagggttgtgggggggggggggttttatttgtttatattattaaaggttaatagttttttaaggttaggtatttatttattatggagttaggaaaatagaggaatagtaaatttgaggggtttttttttatgtatttgaaaagaaaggtatttttttttttttattttttatatttttttttttgttttatagaataagttttaatttaggaaaggtttgtggtgtaggttggagattttttaattttttatataagtttgtagattttttttggtaatgttttttgatttttttagagtgaaattagttaattaagtaatgatattgttaaaatttaaggtttggtaattagtattttaggtaggtttgtgttgataggggtaaatttttattttattttgggttgttaagtatagtggttgttttttagttttttagggatgttgttggttttttgttttttttttaattagttaaagtaaatttttgttaatttaagttttttttgtttgttttttgtgatgaattgtgtatttataagtttgggtggggtgtggttgagagtttgagtgattgagtgggttttggtggtgttgtgtgtagtgggatataatgagtgatagaggttgttgttggattatttttttatgttagtttagatgttgaggtttgttggagtgtgtgtaggggattagattatagggagtgagtgagagggagagagaggtgttgggttttaggagtgtagtataatttggggaaaggaattaatgtttttgggatggttgttttttgttttatttagaggtggagtgtttaagtttaagtagtaggtgtgttaggtttggtggttttgtttttttgtgttttgtttgaggtttagagttttggaggtgggtgtttagtgtgtggtttgtgttttttttttggttttattattggtgttaggatgttgttgtgggaagaatttgttgttggttgtttttttttggtttttaggagagtttgtgaatttgatttttttgattttggagtttttggagaagagatatttaatggttgttggttgtatgtttgggttatgtgtgtgtttgttttatgtgtggagagaggtgttttggattgtggttgaaaggagttggggatgggaggagggggaggggtgaggtaggttggaggagaaagagggataaagagtaaagatttagttagaggaaagagttgatggtatttttgttttttggattttttggtaatttggggtaggatggtgtattttttttgtgtttttttggttgttggtggttttagttgggaggagtaggttggggggttttggtatatagtgtgttgttgttttttagtttattgttttgttatagggagaggttattggtgatttggttttgattttttttttgtttaggttggttttttggggaagtgttttttgttggggttttgttgtagggttagtgtttttttgttgtttttatgtggtgtggttttttgtttgatgatttgggtaggagaagggggtttttatttaattgtatatatgttgatattagtttgtggtagttggtttttattttttgttatttgtaaaatagaagagaaggaaggttgtaagaagtggtggttgttgagtgagtagggtttagatgagattatgttatattagttgttaggtgtttattgtgtgttaggttttaggtgtgtttttttgatttgatagtttttggttgtgtagtagtatttttagtttagttttgggtttaggatatttatttattaagaggggatttttttttagagttgttgtaaaagtgtttagaggttagaggattataaagttatagtgtgttggggaggttgtggatttatttttaagaattttggtgttggggttaagaatttatttgaatgtaatggtagtgggagtgggtgggtggagaggatttttttttttgggaagttgtatgtaaagattattttttagtgtttgtttattagttggagtttggtaaatatttgtagaatattagtgttaatgtgtttttgttttagatagtagttttttttggttttttgtaattttgaaatgaatgggtttttggtttagggtgttttaggagtgagttgagtttgggttttttatttattaggagttatttttttatatttagttatatttttttttagagatattaatttggttatttatttatttattataaataattattttaaagtatgatttaagattgtagaggagagatattgggtggattgagtgagattgaggagagtagggtaaatgtttttggagggtttattgtttgttaaggatggagaaatagttttggtataattgttatttagtttttttttttttttttttgggtgagttaaattttttttatgtttttaattataatgtagtgagttaagtatttaatgtgtttttttttttttgttataggtaagttgggagaggtgggttttgaggggttttattgggtgggtagaagagttgtggttgttttaaagataagaaaagaaggtttagggttttttaggtttttttgattttagtgtttgtttttttttatgttaattagggtatgttgatgattggagggtttattttgtgtgggtgtggggattggggtgggagtaagtgttgttgggttggtggaggtatagaggtggggtagggagttgtgggtttgtttttggtttgagtattgtttttttgtgttttggttttttttgaagggagttgggttttggggagtttttggttaaggttgttgtttataggaggggttgtttggtgttgtggtgtggggatttagggtggggatggttaggtggtttttttatttgttagtgagaatgtgggtggggattttgttgatttgatttttgtgggtttgtgggtttagaagtagtagtttggtggttttagatttagtgattttgtagtaaaattataggattagtttttgattgagatgtttgtttgtgagatattataaaatttattattatagttttttattaatttgatatgaagtaatatagatgggattttattagtttagattttaaatgtttatttatgataattttggaggaaatttgtatgttattattattttgataattttttttttttatatgtttgaattggttgtattattagttggtagttggagtattgtagatggtaattgtaaatagtttttatttatttattttttttaaagaatgaaatatataaaagaaaaagattgtgttgtttggtgtaaagttagttaattattatatatttttttttttatttttttgtgttttagtgttgaagattaaataaagtaatataaaataaatttttaagaatttatagagttttattttaaggattgaaaagaaggttaaggtgtgttttttagtttatttttatatgtttttgtgatttggagatttattttgtagttaaaatgagttttgagatttgtatttttatgttttatttaatgattaggtttattagaagaattgagtttaaataattggggaagataattttttaaaaagagatttttaatttttgtttgttgatttttaaatttgttttattaagataagttttttgtgagaaatttggttgttagattttggaattggttttaatggttaattttataaattgagatgggagattttttttgatgggaggtagtttttatttttaaagtttatgttttagttggaatgtatatgttaaggatttttgttttggttaatttgggttttatattgtgagtatataaaaagtattatatggttaatggaggatgaggaattatggtaaagtaggtaggtaagttttaagaaataaaataatttgttaaaaaataatttttgatgattattgtaagattgaaagtgtaggaaaaatatagtttgaataattttagatttttttatattttttttttttttatatattttgttattttataataaaatttttaatggaaagtttaaaaataaatagtataggaatatgtgttttaaatgaattaaattgtgaaattagttagtaaattaatttgtagtaagtaattatttaaggaaattaaaatattgtttagtttagttttgtattttattatgtgtatgtgttttttataattaattaatataagtgttttaggaatatttgaagataaatatgtttaatttaaggaataaagtatttaaataatttaagtgtaattttgttgagttaaagtaaaatattttataaatgaagtggttatttaattttttagggaaagtttggttattgaaatgttgtatgtttatgttatattaataaaaatttttaatttattttgtttatgtgttttgtttttttgatattattggtatttgaattttagatggatttttgttaaaatgatattttgtgtgataaaagtatttttagttttgattgatagattaaaataaatgtaaggaaatttttttaaattagattaattttttataaaaatattttagaatgtatgaattttgatatttatatttataatggtaaaagttttttttgtttagtttagtaagataatatttatataaaagagtaaaaaaaaattatattattttatgatagtttgatttttaaattgtttaagaaagtaaagtggttaaattggaaaagaggaatatattttggaggtttagaattgaaaattttttttttaatttttagttggaaaataattttttgtatttatttaaagtgtattttttgaagtgttagattggagttgattggtgattaatttaaaggagttataatttaaagaaatggtgagagtttggtatttaggtttggtttttaggtaatttgtttgggtttgagaggttattaattgttagttaagatggaattttttttttttttttttttttttaatggataataatgggaagggggttaattttttagtagttgaaattttgtatttagttttttattttgagaatgttaatttttggtttgaggatttgtttttgtagtgttggtattgagatttaagggaagatattttgttttaaatgttagttatggtttggttttttttttgattttagtattttgtagattgttagtgtttgtggtgggggatgaaaggaatagggttttgtaaggtttgtttgttgattgtgttattttgggtgaaatttagttttaaaagttataaattatttatggtgaagattttttgaagtggaataaatttttagatttgtattattttatatttttgtgggatagatggtttttatttattggttattgggagagagttgttgtttttgtgttttattgttttttggggtgatttttagtgagttgagtttttggttgtatggtaagtgtttgaaagttgggtttgagaggattgtagggtttttgagggtgttaagttttgaaggagtttatgggtgtattggggtttttgaaatttagttgttattggtagtttttttttgtttttttttagtttttttgtttggttttgtattttttttttttttttttttttttattttttttttttttttttgtttttattttgtgtggggagtgatgtgatgttagtagagattttattaaattttattgtatagtggtgtgtgggtggttggttgagtttggttgtgtggttggtgatttaggagtgagtatagtgtttgggtgagtgttggggggagtgagtaggggtgatgagaaatgaggtaggggagggaagtagatgttagtgggttgaagagttgggagttggagttgggagagtgaaaggagaggggatttggtggggtatttaggagttaattgaggagtaggagtatggatttttattgtggaaaggaggattagaagggaggatgggatggaagagaagaaaaagtaatttgtgttaatttggtagttttaataaattaaagggggagtgttagggtagtggggagatagaaatgtatttttggggagtaaattaggatgggttgggaggaagtgatagggaaagtggtttaagagatggaataaaggataatgtttatggggttgtttgggatgaggtgtgtggagtgtgggtgtgagtgtgtgtgtgtgatttttttttaggtttgtagagttgaggaaagaggttatagtaaagagggattgtggagggaggaaagtgagagattggtagagggtgggagtggaggtgggtgtggtggggatgggagaggatgagtgaagagaaatttagaagaatggagtgagttagtgggagagggtgggagggttatagttgggagtgaatgagttaggtttgttagttggggaaggttgggatgttgggtttagtttagttgggatattgtgtttgaggttaaggtgggtggattaggtatgttgagagtgttggtgtataggtgggtatggttatgtattgatttagtgtttatgaagggtttgtattggataaggtttagatgtttatagagtttagaattttttttgttgtatttatatttaataagtttattttgggttatggatattttattttttaaaatgatgaggttaaggtttttggtgaggatggtattaaattgtatgggatagaagtgggggtgggggagagagttttttttaagtttatatttgtttttgtaaagtaaagagtatgtgaaattatagggtatatttttatttgaaaagtgtgttttatttttgaattttgattttttgattttttgatttgagtaaagatgtgtattttggtagtgagtagaatattttggttttgttttgtttttgagtggaaggattataaatataatttgtttggaggattaggtgtgaaggtttttgttaggtatatgggataatgtttttttaattttaagggtattttgttaatgtatgtttttggaaagtgttggaatatagttattgtttttggatttggatttttttattaatattaatttttgtttgagagtaaaatttaggtttgttattaaaaagatatttttttggtttttaattgagaataaagttttttttaaaagttgtattgttttttttaaattaatatattaatatttgtaattttagaaatatatagtgatttgggagaatgtgtataaaatagatatgtttaaaaaagtttggtgtttaaaattaattttagttattatataggtgttgggttttttttatttttgggggttgtttggaatatgttatgtgtttttttgaattattttgtgttttgaatttatttgagttagtagtaaaaataggtaaataaatttgtttaatttgttttgagtgttaaatttttttattttgaaatagttaatagttgatagatggatttattttatggaaagggttagtttttttagttatgaagaaaattgattagagatttatattttaagttatttttaatttttatgtaatatttgtgaaaatttaaattttttttttttatttagtggaaatttaaagtagtgttatttaaggggagagaaatgagggggaaaatgtttatgtgttgtttaattgtattttttttttgattttgagaatttttatttttggtttttgaaattttgttgaggtaagaaaattaaatttttttaataagttttataattgaattttagttataggatattggaaagtgtagtttgagaaagatatttttatttttgtttattgatgatttttgtagtttttttatttttttgagtaatgggttaataattttttttttttttttttttattttgtagagattaagaggtgtttgtagtagaatggttttgtttttagttggtggtgaggataggtaattttatggaaaagttggaagagaatgagaaaattaaagatagaaagatttagagatttgtggagagatatagggagagggaagggagttgtgttgaaaagatgtaaagatatgtgtgtgtaattttttttttttttaggttttagaggtttgtaaattagggttgagaggaaggggtttgggaagtttatgttttttttgttttttttttgtttggagttttgtttgttagaggttggttaattttagttttggttgttgtagatattgtgttgagtttttgggtttttgttttgtttagtgttagtgtagttgaagtgagtagttggtgggaaatgtaaatggtttttggagaaatagaagatatagaatgatttttattttttttttgagtgtgtggaaggagttggatatatgttttatgtttttaattttttttttatatttttagttatatttttattaaataattaattaatgtttagaattattagggaatatattaggtatgtaattgtagaagtagggtgttggggggttataaattattgagttgatttaagatgtggattttaggttttttttttgttaaagtagtaaaggaagagtgggttttggtgattgtatttagattttgattattttaaattagaagggggtggagggagtgtttaagtaaagtaagtaattttttgttttgtagatgtaaataagattgtagtattaaaggtattagtttttttagggttagattgtttggattgggagtttggggaaggggagatattaattttatgtatttgtgaattttaaggatgttatatttttatataaataattttagtgtggattttttggaatggggggagtaatatttttattttagaatattaaaatattttttttttaaagtgtatattttttttatttttttaaaattttgaattatgtttaaagataatagttttttagtaaattggagtattggattattttttttatttttttttattgatattttgatgatttgattttaatgtgtggggggtatagggaattaaatatagtttataaaattaagtttagatgaaatagtgttggttaagtgggtttagataatttttaatgagaattttaattatatttttttttttaatatgttgagataagtgatagaattgttagaatggtaattaaattggaaagtttagggagaataataattttgtgattaaattggggtaaaattgtggataaatgtggggtgatttttgttaattttttgttatttaagagttaggatttgggaaaggtatagtattattttagagtttgttgtgatgggttgtgtgttattatttattttttttattttggattatgattttaattttggtaagtaatttttttagttttttatttgataataagtgagtatgtaaatattaatggttagtgatgtttaattgttttaaatattattgatttgttggttgttttaaattgtttttttagtttaggttttgtttttgaattgtttattttagaggtttgatttatgtttttgatgttataatataataattgtttttttaaaaaaggtatttaagatgaattaattgatttgtatataaattaaaattattatgtgttgttgattttggtgttttataattattttgaaattagtatttaattatttgagttaaaagaatatataaatgtttgtattgatttattaatgaattatttaattaaaatgtttgggtaatgttgggtgttggaaagattgttaaattaagatatattataggagggatatgaagattagaaaggtaatagattaatattttgtatttaaaatggagtttttggtgatttttagttttaattttggagtaggggttttttttttttgttgttaaaaagattttgtgtttgtttgtgagtgagtgtatttaagtggaaggaatgtttttatggttatggtggtttaggttttttgtttggattgggattttatagttttaatttaggagtgttaaattttggaagattttgggttagttttggaggtgtgtggttttgtaagttgttaggttaagtttgttttttttgtttgtttttttggtaggttgggtgtgttatggtagtgagttttttgtgtaaatggagagttggaattaaagttgatatttaatagatatgttaattgagtatttatttttgttttgagaataggaataaaaggtagttttttttaagagaggtggtgtaaaggtatgttataggagtttagaaaaggttggtggtgggaaatttgtagtttgggggttagttaatatttttttttattttaagtatttattgatttgttgttgttatttttggtgatgtagaaggatatttgaaagaatttttgatggggttttgatttgagaaaggaggtgatttgtttaggtttttattaaatttttaattattatattaattgtttttttttattttttatttgatttttttttttttgtttatttttaattttttaattatttagaaatttttttattttttagtggttttttttttgtagtagttttttatttgaattttttttttgtttttttgtggtagggtttgtatattgatttttttgatttttggtatatttgggttttttgaaattttttaatttttttagatttgaggatggtaggttttattttttttattgtgtgtatatatttagagatatgaaaatttatatagattgtttttaaatttagggtatttaatagatgttttttttttagtttgttttttgatttgaaatgtttgtttgattttaatttggatattatttttttttgtttttttttttttaaagtagtttggatatgtgtgtaagtgagtttagaatagttttatttatattttttattaaattgtaaataaaagaagaattaatgaagtagattggtatatagattgtattaagagtttgaatttttagtttttggattttttatttaattttggttgttatttatattgatagagttattttaagtagaggtttagagaaatttgtattgtgggataataggtaaagttatagtaaaaagtggaataattttaaagttattttattagaatgtaaattgtatttttgggttttgtttgtaattatttagttttaatatatatagagttagataggaaaaaataggttaatatagttattggtattagagaagataaattttatgggttttttagtgaaaagaagatttttaaagtttataatttttgattatttaattttatttataattgtgggaatgaataagatattaattgttttatgtattttatttatattaattaatttgtgtttttattaaaagtagttatatagaattttttttaatttttggtagtaagtttagaaaatgaagtttatagttattttgaattggatatattttttgagttgattatttttgtaagtgtaggaatataatattgtttttttatggtttttttgtatttttttagggtttgtaagtttttattaggtttgatattattgtttgggtttatatttattataagtaaatttgattattatgttgattttaaaatagtttatttggttagtataattttagtttttaaattataaaaattttttaatatatgaagtttttagtttttattttttttagttttttgtttatttaaaatttttattttaattggtgtaagtaataataatttgtattattatttgtattttttttatttttttggagattgggttggattttagagagaatattagtattattattattataaataataaaatttaaaagtaaagtttttatttgtatgataattggtatttggaatgtttttgatttatttaatgttattttataaaggtattttgtaaatttttttggaatttttagtaagagtttgtagtaattggaataattttttgggaagatattttttttgatgggtttttagtttttggaggaatagattgagagtaattagggagggaggggatattggaaattggtagttatgttagttgaaataagtttgggtttagtaaggtgattgatgttgtggttgattttttattttgagtttttttttaattggggtattgattttttttattttgggattttaaggtatttggtgtgtatgtagattttttttttgtggtttttattatgtggttttgtagtaggtttttggtttaatgatattttatagttatagtttttatatttattattatgattttaatgtttaggtttttagtgtatttatattaaatttgttttattagtaagttggagtatataggagagatgggggtaagtaaggatttagtagagtttaaatttagatatgtttaaatggttttgattgtgtaaagtgtggtaatgttttttgttgttttagttttttattttaagttttatatgttttttggttaatgaagtgtgatataggttatatgttaggaataatagtatttgttgagaataaagtgaatttaggaaatttggtatatataaaatgtatttagttatttgaattagtaataatggtaaaaattaatatttatagagtgtttagttaatttagttattgtattaaatatttttgtattgataattatatttattttttatgttaatattataaggtaggtattgttattttataaatgaagatagtgaggtttgttatgattgtgttattggtttaaggttatttagttggttagagtataagtttataattgttggaggttatagtggataggatattgttttaggttatgtaggtagtaagtggtatagtgggaatttgaatttaggtttgtgtaattttaaagtttaaaatgttaattagtatattgaattaatggtaattggaattagaagattaggggtttttgggggaaggaaatatagaatttatttatggaatattttataaataaaagaataatgtagagataggaaagtaaatatattttttgagggatggagaaagttagaaatgttttaaatgttaaagaggaggaaatgagaaatgattggatgagaaagtagaaaagttaaattttggtatttgttttgggtagtttaggaagagaaaggtaagtttagggatatttttgagttataggaaaattaatgtttagatggttagtttggattaagtttaatataggattttaggaatatggtttattagaattgttttttagtaattttaagggagaataaaatttttgaattgggtttaagtagttttattttagaagtaaagagagatggaagtaaggattgagtaataagaatatttatattgtaagaatatgtaagttgagtaggagtgaaatttagaaaaatttgttaggattttggttgttgtgttaaattatgttatattttaagtagaaattagatttttattattattatttgtttaggtttagttagtaattttattattgtagtaaagttatttgaaattttaagagaaatgattttttgtgttgaagaagatattttgggtggaaggatgttagtagataaatggagtgtaaagatagtgattttaaggatatagtttgtggggagtaatattggattatatatttgttgtttgtggtagaatgttagttaggggagaatattaggtagttttttataagtttattttattataaaaagataggattgattttaaaggttatttttaatttaggtttgttttattattgaaaatgatttaaaattggatttattttggttttttttaggagggatagataaatataatttgtatatatggttttttagttttaggaagtataggaggagaatgaaagaattaatttagttttttgttttttggtaaaaatttttatatttgtgttgttgtaagaatttaagattattttgtttagaatgttgtggtatttttgaaagtaaggtttgagggtatatagagttttattttttatttttatgttgtggattttattgttttttttaaatgggaaagagaaattagaatttatagaaagtaaggtttggaaaggatttagagggtattttttttttttagtttatgtttaaattatttttagaaatatagttagttatattttttagtaaagagttttttatggttttttggtaatgtatttttatgttttataattttatagttatattgtatatttattgattaaattttaagtattgaagaaaatgatgttatattaaaaagttttaattagtagggggtatgttttttagagttttttaaatattttatatttttattttaaaaaaagatgaaaatattattagtttaatttaatagatggaaaattttgttatagagatttttagagagttatatttggttatgtagtgtgatgtttgaaagaattaaattaaaaataaagttaggaaattttatgtttagggtttttttagtagatatattattttttgggggttggttattatttttttgtttgagtaaagtatatgtttgattgtaattttatttgtttttttgtttgtttgtttgtgagtagtttattttttaatttattaatttatttttttgttagttttttaaaatattataagttaattaatgttgataaaattttatttttattatgagtgttatttgagtagattgagatggttgttatattttttaaatattatgtgtaataaatagtgttgttattgttttagtgttatgattttgtttttatttggaaattgtataaatattatattttttgttatgataggattatttttatttattaggatttttgatatttgtgttgttatttgggagaatgttgattattttgtttatgttatttttgaggttataataattgtttttttgtttagttgtgtttttttttttataggtgaatttagtttttttttttatgtttgattttaagaaattggtgttttattgaaagatgtttaaattttttgagagaaaatgttggagtaagaataatttgttatgtattgtttttatttgagtattaatgtttttttaattttatatgtttttaaattttttgagaattttttttttttgaatgtaatttatgaattaaaagtgattgtaatttttaaaatattatgttgtttatagtaaatatatataatttttatttgttaattaaaaaaagtaatagggtttttatttttatttttgatatttgttttttttattttttttttaagtattttttttttttttttagagatgtatttattgagagtattttgttatttttttttttttgtagttatgtatgattaaagttgtgtttttgaaattttttattttttttgttataattgataatttattttgttttttattaatttattaatgttattttattggtttttgatttatataaattaaatagattttagaaaatttaataaaaataaaaataatgttttttattttgaaatatttatttattgtttttttttagggtatatatattatattttttttttttatattttattttttttgaatttataagaatgtgttattgaatatagagaaaataatttaagaaaggaaaaggaatgatttgtttaaaatgaggaaaaagtagagttgaggtttaggattgtggtttaataagatgatttagttattttttggtagttttattttttggtaattttttaagttgagttttggatgatgtaaataatatttttagatttttaatgggtatatgttgaattaaaaagaaaaatttatggtattttttaattatgtgtaaatgagtaaagaaaaaggaaagaaaaggagtggttaaattgatatggtagggtttaggattgggggaagaagaaagagtaatagagagagtggaatagttaaaaaaagaatgagattatgttttttgtagaaatatggatggagttggaggttattatttttagtaaattaaattaggattagaaaattaaataatgtatgtttttatttataagtgggagttaaatgaggagaatttatagatataaagagaggaataatagatattggggtttattggaaggtggtggatgggagaggggagaggattagaaaaaataattattgggtatgaggtttagtatttgggtgataaaataatttgtataataaatttttgtgataggtttatttatataataaatttgtatatgtgttttgaatttgagatataatttaaagaaaaagagagtgtatttgtttgtaaattggttttagtagattgttttttgagttttttttgttttttaaattgaatttaagtggtattatatttttaaatgaaaattttatttttaattataggtgaagttaattttttatttttttaataatttttttattattttttgtattgtaagtaaggtaaagatttagtttaaatgttgttagtttagtttattttttaaaaaatatattttttgagaggtttgagaaaattaagaaagtatattttgtttagtttttttaaatattatttttttggaaatagtattttgtttagtttttttaaatattattttttaattagtgagttagtttagattttagagggtttttggaattagaaagaaggtaaggatgaatattaggtttaagattatttttatgttgttttattattaaattagaaaatttggatgttttgtaggtaggtatgtttatgagagttatttaaaaaagatatgttttttgaagtgttaagtttagtgattatgtagtttatg

SEQ ID NO: 14 - DNA, 12001 bp, Homo sapiens
gtgttagattggagttgattggtgattaatttaaaggagttataatttaaagaaatggtgagagtttggtatttaggtttggtttttaggtaatttgtttgggtttgagaggttattaattgttagttaagatggaattttttttttttttttttttttttaatggataataatgggaagggggttaattttttagtagttgaaattttgtatttagttttttattttgagaatgttaatttttggtttgaggatttgtttttgtagtgttggtattgagatttaagggaagatattttgttttaaatgttagttatggtttggttttttttttgattttagtattttgtagattgttagtgtttgtggtgggggatgaaaggaatagggttttgtaaggtttgtttgttgattgtgttattttgggtgaaatttagttttaaaagttataaattatttatggtgaagattttttgaagtggaataaatttttagatttgtattattttatatttttgtgggatagatggtttttatttattggttattgggagagagttgttgtttttgtgttttattgttttttggggtgatttttagtgagttgagtttttggttgtatggtaagtgtttgaaagttgggtttgagaggattgtagggtttttgagggtgttaagttttgaaggagtttatgggtgtattggggtttttgaaatttagttgttattggtagtttttttttgtttttttttagtttttttgtttggttttgtattttttttttttttttttttttttattttttttttttttttttgtttttattttgtgtggggagtgatgtgatgttagtagagattttattaaattttattgtatagtggtgtgtgggtggttggttgagtttggttgtgtggttggtgatttaggagtgagtatagtgtttgggtgagtgttggggggagtgagtaggggtgatgagaaatgaggtaggggagggaagtagatgttagtgggttgaagagttgggagttggagttgggagagtgaaaggagaggggatttggtggggtatttaggagttaattgaggagtaggagtatggatttttattgtggaaaggaggattagaagggaggatgggatggaagagaagaaaaagtaatttgtgttaatttggtagttttaataaattaaagggggagtgttagggtagtggggagatagaaatgtatttttggggagtaaattaggatgggttgggaggaagtgatagggaaagtggtttaagagatggaataaaggataatgtttatggggttgtttgggatgaggtgtgtggagtgtgggtgtgagtgtgtgtgtgtgatttttttttaggtttgtagagttgaggaaagaggttatagtaaagagggattgtggagggaggaaagtgagagattggtagagggtgggagtggaggtgggtgtggtggggatgggagaggatgagtgaagagaaatttagaagaatggagtgagttagtgggagagggtgggagggttatagttgggagtgaatgagttaggtttgttagttggggaaggttgggatgttgggtttagtttagttgggatattgtgtttgaggttaaggtgggtggattaggtatgttgagagtgttggtgtataggtgggtatggttatgtattgatttagtgtttatgaagggtttgtattggataaggtttagatgtttatagagtttagaattttttttgttgtatttatatttaataagtttattttgggttatggatattttattttttaaaatgatgaggttaaggtttttggtgaggatggtattaaattgtatgggatagaagtgggggtgggggagagagttttttttaagtttatatttgtttttgtaaagtaaagagtatgtgaaattatagggtatatttttatttgaaaagtgtgttttatttttgaattttgattttttgattttttgatttgagtaaagatgtgtattttggtagtgagtagaatattttggttttgttttgtttttgagtggaaggattataaatataatttgtttggaggattaggtgtgaaggtttttgttaggtatatgggataatgtttttttaattttaagggtattttgttaatgtatgtttttggaaagtgttggaatatagttattgtttttggatttggatttttttattaatattaatttttgtttgagagtaaaatttaggtttgttattaaaaagatatttttttggtttttaattgagaataaagttttttttaaaagttgtattgttttttttaaattaatatattaatatttgtaattttagaaatatatagtgatttgggagaatgtgtataaaatagatatgtttaaaaaagtttggtgtttaaaattaattttagttattatataggtgttgggttttttttatttttgggggttgtttggaatatgttatgtgtttttttgaattattttgtgttttgaatttatttgagttagtagtaaaaataggtaaataaatttgtttaatttgttttgagtgttaaatttttttattttgaaatagttaatagttgatagatggatttattttatggaaagggttagtttttttagttatgaagaaaattgattagagatttatattttaagttatttttaatttttatgtaatatttgtgaaaatttaaattttttttttttatttagtggaaatttaaagtagtgttatttaaggggagagaaatgagggggaaaatgtttatgtgttgtttaattgtattttttttttgattttgagaatttttatttttggtttttgaaattttgttgaggtaagaaaattaaatttttttaataagttttataattgaattttagttataggatattggaaagtgtagtttgagaaagatatttttatttttgtttattgatgatttttgtagtttttttatttttttgagtaatgggttaataattttttttttttttttttttattttgtagagattaagaggtgtttgtagtagaatggttttgtttttagttggtggtgaggataggtaattttatggaaaagttggaagagaatgagaaaattaaagatagaaagatttagagatttgtggagagatatagggagagggaagggagttgtgttgaaaagatgtaaagatatgtgtgtgtaattttttttttttttaggttttagaggtttgtaaattagggttgagaggaaggggtttgggaagtttatgttttttttgttttttttttgtttggagttttgtttgttagaggttggttaattttagttttggttgttgtagatattgtgttgagtttttgggtttttgttttgtttagtgttagtgtagttgaagtgagtagttggtgggaaatgtaaatggtttttggagaaatagaagatatagaatgatttttattttttttttgagtgtgtggaaggagttggatatatgttttatgtttttaattttttttttatatttttagttatatttttattaaataattaattaatgtttagaattattagggaatatattaggtatgtaattgtagaagtagggtgttggggggttataaattattgagttgatttaagatgtggattttaggttttttttttgttaaagtagtaaaggaagagtgggttttggtgattgtatttagattttgattattttaaattagaagggggtggagggagtgtttaagtaaagtaagtaattttttgttttgtagatgtaaataagattgtagtattaaaggtattagtttttttagggttagattgtttggattgggagtttggggaaggggagatattaattttatgtatttgtgaattttaaggatgttatatttttatataaataattttagtgtggattttttggaatggggggagtaatatttttattttagaatattaaaatattttttttttaaagtgtatattttttttatttttttaaaattttgaattatgtttaaagataatagttttttagtaaattggagtattggattattttttttatttttttttattgatattttgatgatttgattttaatgtgtggggggtatagggaattaaatatagtttataaaattaagtttagatgaaatagtgttggttaagtgggtttagataatttttaatgagaattttaattatatttttttttttaatatgttgagataagtgatagaattgttagaatggtaattaaattggaaagtttagggagaataataattttgtgattaaattggggtaaaattgtggataaatgtggggtgatttttgttaattttttgttatttaagagttaggatttgggaaaggtatagtattattttagagtttgttgtgatgggttgtgtgttattatttattttttttattttggattatgattttaattttggtaagtaatttttttagttttttatttgataataagtgagtatgtaaatattaatggttagtgatgtttaattgttttaaatattattgatttgttggttgttttaaattgtttttttagtttaggttttgtttttgaattgtttattttagaggtttgatttatgtttttgatgttataatataataattgtttttttaaaaaaggtatttaagatgaattaattgatttgtatataaattaaaattattatgtgttgttgattttggtgttttataattattttgaaattagtatttaattatttgagttaaaagaatatataaatgtttgtattgatttattaatgaattatttaattaaaatgtttgggtaatgttgggtgttggaaagattgttaaattaagatatattataggagggatatgaagattagaaaggtaatagattaatattttgtatttaaaatggagtttttggtgatttttagttttaattttggagtaggggttttttttttttgttgttaaaaagattttgtgtttgtttgtgagtgagtgtatttaagtggaaggaatgtttttatggttatggtggtttaggttttttgtttggattgggattttatagttttaatttaggagtgttaaattttggaagattttgggttagttttggaggtgtgtggttttgtaagttgttaggttaagtttgttttttttgtttgtttttttggtaggttgggtgtgttatggtagtgagttttttgtgtaaatggagagttggaattaaagttgatatttaatagatatgttaattgagtatttatttttgttttgagaataggaataaaaggtagttttttttaagagaggtggtgtaaaggtatgttataggagtttagaaaaggttggtggtgggaaatttgtagtttgggggttagttaatatttttttttattttaagtatttattgatttgttgttgttatttttggtgatgtagaaggatatttgaaagaatttttgatggggttttgatttgagaaaggaggtgatttgtttaggtttttattaaatttttaattattatattaattgtttttttttattttttatttgatttttttttttttgtttatttttaattttttaattatttagaaatttttttattttttagtggttttttttttgtagtagttttttatttgaattttttttttgtttttttgtggtagggtttgtatattgatttttttgatttttggtatatttgggttttttgaaattttttaatttttttagatttgaggatggtaggttttattttttttattgtgtgtatatatttagagatatgaaaatttatatagattgtttttaaatttagggtatttaatagatgttttttttttagtttgttttttgatttgaaatgtttgtttgattttaatttggatattatttttttttgtttttttttttttaaagtagtttggatatgtgtgtaagtgagtttagaatagttttatttatattttttattaaattgtaaataaaagaagaattaatgaagtagattggtatatagattgtattaagagtttgaatttttagtttttggattttttatttaattttggttgttatttatattgatagagttattttaagtagaggtttagagaaatttgtattgtgggataataggtaaagttatagtaaaaagtggaataattttaaagttattttattagaatgtaaattgtatttttgggttttgtttgtaattatttagttttaatatatatagagttagataggaaaaaataggttaatatagttattggtattagagaagataaattttatgggttttttagtgaaaagaagatttttaaagtttataatttttgattatttaattttatttataattgtgggaatgaataagatattaattgttttatgtattttatttatattaattaatttgtgtttttattaaaagtagttatatagaattttttttaatttttggtagtaagtttagaaaatgaagtttatagttattttgaattggatatattttttgagttgattatttttgtaagtgtaggaatataatattgtttttttatggtttttttgtatttttttagggtttgtaagtttttattaggtttgatattattgtttgggtttatatttattataagtaaatttgattattatgttgattttaaaatagtttatttggttagtataattttagtttttaaattataaaaattttttaatatatgaagtttttagtttttattttttttagttttttgtttatttaaaatttttattttaattggtgtaagtaataataatttgtattattatttgtattttttttatttttttggagattgggttggattttagagagaatattagtattattattattataaataataaaatttaaaagtaaagtttttatttgtatgataattggtatttggaatgtttttgatttatttaatgttattttataaaggtattttgtaaatttttttggaatttttagtaagagtttgtagtaattggaataattttttgggaagatattttttttgatgggtttttagtttttggaggaatagattgagagtaattagggagggaggggatattggaaattggtagttatgttagttgaaataagtttgggtttagtaaggtgattgatgttgtggttgattttttattttgagtttttttttaattggggtattgattttttttattttgggattttaaggtatttggtgtgtatgtagattttttttttgtggtttttattatgtggttttgtagtaggtttttggtttaatgatattttatagttatagtttttatatttattattatgattttaatgtttaggtttttagtgtatttatattaaatttgttttattagtaagttggagtatataggagagatgggggtaagtaaggatttagtagagtttaaatttagatatgtttaaatggttttgattgtgtaaagtgtggtaatgttttttgttgttttagttttttattttaagttttatatgttttttggttaatgaagtgtgatataggttatatgttaggaataatagtatttgttgagaataaagtgaatttaggaaatttggtatatataaaatgtatttagttatttgaattagtaataatggtaaaaattaatatttatagagtgtttagttaatttagttattgtattaaatatttttgtattgataattatatttattttttatgttaatattataaggtaggtattgttattttataaatgaagatagtgaggtttgttatgattgtgttattggtttaaggttatttagttggttagagtataagtttataattgttggaggttatagtggataggatattgttttaggttatgtaggtagtaagtggtatagtgggaatttgaatttaggtttgtgtaattttaaagtttaaaatgttaattagtatattgaattaatggtaattggaattagaagattaggggtttttgggggaaggaaatatagaatttatttatggaatattttataaataaaagaataatgtagagataggaaagtaaatatattttttgagggatggagaaagttagaaatgttttaaatgttaaagaggaggaaatgagaaatgattggatgagaaagtagaaaagttaaattttggtatttgttttgggtagtttaggaagagaaaggtaagtttagggatatttttgagttataggaaaattaatgtttagatggttagtttggattaagtttaatataggattttaggaatatggtttattagaattgttttttagtaattttaagggagaataaaatttttgaattgggtttaagtagttttattttagaagtaaagagagatggaagtaaggattgagtaataagaatatttatattgtaagaatatgtaagttgagtaggagtgaaatttagaaaaatttgttaggattttggttgttgtgttaaattatgttatattttaagtagaaattagatttttattattattatttgtttaggtttagttagtaattttattattgtagtaaagttatttgaaattttaagagaaatgattttttgtgttgaagaagatattttgggtggaaggatgttagtagataaatggagtgtaaagatagtgattttaaggatatagtttgtggggagtaatattggattatatatttgttgtttgtggtagaatgttagttaggggagaatattaggtagttttttataagtttattttattataaaaagataggattgattttaaaggttatttttaatttaggtttgttttattattgaaaatgatttaaaattggatttattttggttttttttaggagggatagataaatataatttgtatatatggttttttagttttaggaagtataggaggagaatgaaagaattaatttagttttttgttttttggtaaaaatttttatatttgtgttgttgtaagaatttaagattattttgtttagaatgttgtggtatttttgaaagtaaggtttgagggtatatagagttttattttttatttttatgttgtggattttattgttttttttaaatgggaaagagaaattagaatttatagaaagtaaggtttggaaaggatttagagggtattttttttttttagtttatgtttaaattatttttagaaatatagttagttatattttttagtaaagagttttttatggttttttggtaatgtatttttatgttttataattttatagttatattgtatatttattgattaaattttaagtattgaagaaaatgatgttatattaaaaagttttaattagtagggggtatgttttttagagttttttaaatattttatatttttattttaaaaaaagatgaaaatattattagtttaatttaatagatggaaaattttgttatagagatttttagagagttatatttggttatgtagtgtgatgtttgaaagaattaaattaaaaataaagttaggaaattttatgtttagggtttttttagtagatatattattttttgggggttggttattatttttttgtttgagtaaagtatatgtttgattgtaattttatttgtttttttgtttgtttgtttgtgagtagtttattttttaatttattaatttatttttttgttagttttttaaaatattataagttaattaatgttgataaaattttatttttattatgagtgttatttgagtagattgagatggttgttatattttttaaatattatgtgtaataaatagtgttgttattgttttagtgttatgattttgtttttatttggaaattgtataaatattatattttttgttatgataggattatttttatttattaggatttttgatatttgtgttgttatttgggagaatgttgattattttgtttatgttatttttgaggttataataattgtttttttgtttagttgtgtttttttttttataggtgaatttagtttttttttttatgtttgattttaagaaattggtgttttattgaaagatgtttaaattttttgagagaaaatgttggagtaagaataatttgttatgtattgtttttatttgagtattaatgtttttttaattttatatgtttttaaattttttgagaattttttttttttgaatgtaatttatgaattaaaagtgattgtaatttttaaaatattatgttgtttatagtaaatatatataatttttatttgttaattaaaaaaagtaatagggtttttatttttatttttgatatttgttttttttattttttttttaagtattttttttttttttttagagatgtatttattgagagtattttgttatttttttttttttgtagttatgtatgattaaagttgtgtttttgaaattttttattttttttgttataattgataatttattttgttttttattaatttattaatgttattttattggtttttgatttatataaattaaatagattttagaaaatttaataaaaataaaaataatgttttttattttgaaatatttatttattgtttttttttagggtatatatattatattttttttttttatattttattttttttgaatttataagaatgtgttattgaatatagagaaaataatttaagaaaggaaaaggaatgatttgtttaaaatgaggaaaaagtagagttgaggtttaggattgtggtttaataagatgatttagttattttttggtagttttattttttggtaattttttaagttgagttttggatgatgtaaataatatttttagatttttaatgggtatatgttgaattaaaaagaaaaatttatggtattttttaattatgtgtaaatgagtaaagaaaaaggaaagaaaaggagtggttaaattgatatggtagggtttaggattgggggaagaagaaagagtaatagagagagtggaatagttaaaaaaagaatgagattatgttttttgtagaaatatggatggagttggaggttattatttttagtaaattaaattaggattagaaaattaaataatgtatgtttttatttataagtgggagttaaatgaggagaatttatagatataaagagaggaataatagatattggggtttattggaaggtggtggatgggagaggggagaggattagaaaaaataattattgggtatgaggtttagtatttgggtgataaaataatttgtataataaatttttgtgataggtttatttatataataaatttgtatatgtgttttgaatttgagatataatttaaagaaaaagagagtgtatttgtttgtaaattggttttagtagattgttttttgagttttttttgttttttaaattgaatttaagtggtattatatttttaaatgaaaattttatttttaattataggtgaagttaattttttatttttttaataatttttttattattttttgtattgtaagtaaggtaaagatttagtttaaatgttgttagtttagtttattttttaaaaaatatattttttgagaggtttgagaaaattaagaaagtatattttgtttagtttttttaaatattatttttttggaaatagtattttgtttagtttttttaaatattattttttaattagtgagttagtttagattttagagggtttttggaattagaaagaaggtaaggatgaatattaggtttaagattatttttatgttgttttattattaaattagaaaatttggatgttttgtaggtaggtatgtttatgagagttatttaaaaaagatatgttttttgaagtgttaagtttagtgattatgtagtttatg

SEQ ID NO: 15 - DNA, 4001 bp, Homo sapiens
tagagtatttaattttttttttttaatagtaaagtttttggatgttgtttgatttgtttgattttgttttttgtttttagaattttaataaatttggaattttttattgattagtataaattaggatgttgttattgggttatttatttgagtttatttttgttaatttataaagtatagatttgttataaagttaaggtaagttttttttataaaattatgattataatttagaagagggggtgtgagttttaatttttagagtttaatttttgagagaagataaataaattaagtagaaaagttttttttttttttttttttttttttttaagaggattagtagttgtgtattaaaattttgtttttggagattataaaattaggaaatagggtgtgtgggagagatttgaatggttgaaataattgtaaagaaggtgtaagaagtgtgagtttaggagggaaaaagttgggttagggttgggataaaggttttttagggagggttaatttttttgtgtttttggtgggttttttttgttaaaggtttataggttggagtttgtttgtggtttttggtttggtagggattttattagttttgttttggtaattgtaagttaggaatataatgttttgtgtaggggattgtttatgtagtttagtttgtgagattgtgggatggtggggtagtgagttggtgttgttttgggagtttgagttagggtggtagttttgttggttttggagagggaattgtaattttgtaattaggttgttgtgaggttttttgtttttgtaaagttgtgttttattggtgtttttttaggtggtgttgttttttatatttttttttggtttatttggtttgtatttttataatattttttttttattttttttagattttgtgttggtttttatttggatttgggtttttgtaaggttggtttatatagtgatttttttgtgtgtggatatgtttgggtagtggtttttttggaaagtggtttttagtttttggagttgttggttggtaaagtgagtttgttgttgtttttgttgtttttttttagatgggtttttggtgtttatgtttttattttttttttgttggtttttatttttttttgaaaatgaaatatatatatttttttgttagtatgtttatttgtaatgtggatgttaattggattggtggtagaagttgtggaagagttgggttgtttggtgttggaggagggtgtgtgtggtggttttgggttgtgaggagtgttgtgtttgtggggtgtgtaggtgtaagtgtgggtgtttgtgttttattttttttttttttttagtgttgtatgttttatttatatgtttattttattgtagtggtatatttatttttatagtttgtgtttttaagtatatttatatatttttgtgtagatatattaaattttttgggatgtgtatatgtgtgtggtttatagattttttttttttttgtagaaagtttagatttttatgtggtttgggaaggttaggaaaagatgtggggatttggttgggtattgaagtttgttggtttttttttaaaaaaaaaaaaaaaatgtttttttgtgaagggtatttttgagtggttttaggtaattttttaatgagtggagttttttgggagttgaaagttgagaggaaaatagggatagaggttggtggtttttgaaggtttttgaattaagatgttgggatttttgtgatttaggaaatagaagggaggttagggtatgaatagagagggtggtagaattgtttgtgtttttagtgttttaggagttgggttggttgagggagaattaaagggatgtggggtagttaaaattttggtttttggaagttttgtggggagttaggtgaatgattatttttattatgtttttttttggaggggttgatttttttggggtgagagggagtgggtggtgtagagtagttgagtgggaatgtttgtagggtggtgtggtgttttatttgtggtttttgggttggaggtgttggagatggtgtgtatttttagtttgtgtttggaggagtttagtgattggggttgattgggagttagaattgaagttatggttaatggttggggatggtgataggaagatgaggagatggttgatagtttggtttttgttgtttggtgttttaagtgaagtgggttttttatgtagtttatggatgagggagtgtgatgttttattagtttttggttattgttttgttgagtttttgtagttgttgttgtttgttttgggttgtgttttaggtgtggagtttttttgttgtggggagagttaggggatgtaatttttgttgagtttttaagttaagttgtttttgttttttttggaaggtttaagtgaaaaagtttggagatggaaagttagtgggtaaatgaagatatgggatgtgggtagaagggtattatttagagtgtttttagggagtaggtttttaagttttaaagtgaaataagagtgggtaaagatttttttttttttttttttttttttttaagaatttttttaataaggaaagttaatgttgattgtgttttgtttgttttttttttatgtggtagttttgatagagaagtgttaagagtgatagggataggtaggtgatattagattttttgtggtggtagtagttgttgtagttatgatgtggttttttgagtgtattttttgtaatgtgtatatgtatattttttgggtggttgaataggagttgggttttgttgtagtttagttttaggtatttaggtgagtgatggattagatttgtggttttgtgtttttttgttggtttaatattttaaaattagaggtgggttttttggtgttgagatgttattttgttgtggttttttttagttttttttgtttttgtttttttttagatttttttttgggtgtgattgatgtggttttgtattaattaggatgttttgagttgtggtggagggattgttttgtttgtatttattagtagtgtggggttgggttattgttttgttgtgtgtattgggtttatataggtaagtttttgggaatttagtttttgtttagtttaaggtgatttggtttttagtatgaatttaaaggtgaagagatgaggttaggagttgaaggtttgggagaagagagtggaatggttaagaagagaaaggtataaggattaataagatatttattttttgtgttttattatatttatttttaattttttattttatataaaaaggagatatgttatttaaaattagaaaatttgaaaaatagtaataaattatttttttgattttaaattttttaaatagtttgttaagtgaatgttgtgttaatttgaagaagttttaattgtaaagaagatagagttttgaaaaggtaggttaataaattagaaattgagaagtaaatggatttgttaaaagaaaattattttgattttaaatgaataattgtttggtggtttattttggatttatataagaataaaaagttgttttagattatgttttttgtgatgtttattagtttttagatagaaaatatataatagaagagaaattttaatttagtgtttttaaaatgttgaaagtttatttattttatttaatgttgattaagatatatattttagattttttaaattttttgtatattgtattaagtttgttttaatttgagagagttatgttttaaatttgatttttttgtttattttattattaattagatttaaatttataaagtttgtagaattaataattttgagttaattatatatgaaatatgttttaatgaatttttatataattaagaatgttgttaaataattaattttaaggataatttttaatagttattttttttttttagtgagtttaaggttgttttgagttattaaagtttaagtaggtagaaggggtgtgtgtgagttaagggtgaaaa

SEQ ID NO: 16 - DNA, 408 bp, Homo sapiens
tcctcaactctgcaggcctgaaagaaggtcacacacgcacgctcacacccacactccacacgcctcgtcccaaacaaccccatgaacattgtcctttgttccgtctcttgggccactttccctgtcgcttcctcccagcccgtcctgatttgctccccaaaagtacgtttctgtctccccgctgccctggcgctccccctttgatttattagggctgccgggttggcgcagattgctttttcttctcttccatcccatcctcccttctggtcctcctttccacagtgggagtccgtgctcctgctcctcggttggctcctaagtgccccgccaggtcccctctcctttcgctctcccggctccggctcccgactcttcggcccgctggcatctgcttccctcccctgc

SEQ ID NO: 17 - DNA, 144 bp, Homo sapiens
ttctggtcctcctttccacagtgggagtccgtgctcctgctcctcggttggctcctaagtgccccgccaggtcccctctcctttcgctctcccggctccggctcccgactcttcggcccgctggcatctgcttccctcccctgc

SEQ ID NO: 18 - DNA, 162 bp, Homo sapiens
tggcatctgcttccctcccctgcctcgtttctcgtcgcccctgctcgctccccccggcgctcgcccgggcgctgtgctcgctcctggatcgccagccgcgcagcgggctcgccggcgcccgcgcgccactgtgcagtggagtttggtggaatctctgctgac

SEQ ID NO: 19 - DNA, 408 bp, Homo sapiens
tttttaattttgtaggtttgaaagaaggttatatacgtacgtttatatttatattttatacgtttcgttttaaataattttatgaatattgttttttgtttcgttttttgggttattttttttgtcgtttttttttagttcgttttgatttgttttttaaaagtacgtttttgttttttcgttgttttggcgttttttttttgatttattagggttgtcgggttggcgtagattgttttttttttttttttattttatttttttttttggtttttttttttatagtgggagttcgtgtttttgtttttcggttggtttttaagtgtttcgttaggtttttttttttttcgttttttcggtttcggttttcgatttttcggttcgttggtatttgttttttttttttgt

SEQ ID NO: 20 - DNA, 144 bp, Homo sapiens
ttttggtttttttttttatagtgggagttcgtgtttttgtttttcggttggtttttaagtgtttcgttaggtttttttttttttcgttttttcggtttcggttttcgatttttcggttcgttggtatttgttttttttttttgt

SEQ ID NO: 21 - DNA, 162 bp, Homo sapiens
tggtatttgttttttttttttgtttcgtttttcgtcgtttttgttcgtttttttcggcgttcgttcgggcgttgtgttcgtttttggatcgttagtcgcgtagcgggttcgtcggcgttcgcgcgttattgtgtagtggagtttggtggaatttttgttgat

SEQ ID NO: 22 - DNA, 408 bp, Homo sapiens
acaaaaaaaaaaaacaaataccaacgaaccgaaaaatcgaaaaccgaaaccgaaaaaacgaaaaaaaaaaaaacctaacgaaacacttaaaaaccaaccgaaaaacaaaaacacgaactcccactataaaaaaaaaaaccaaaaaaaaaaataaaataaaaaaaaaaaaaaaacaatctacgccaacccgacaaccctaataaatcaaaaaaaaaacgccaaaacaacgaaaaaacaaaaacgtacttttaaaaaacaaatcaaaacgaactaaaaaaaaacgacaaaaaaaataacccaaaaaacgaaacaaaaaacaatattcataaaattatttaaaacgaaacgtataaaatataaatataaacgtacgtatataaccttctttcaaacctacaaaattaaaaa

SEQ ID NO: 23 - DNA, 144 bp, Homo sapiens
acaaaaaaaaaaaacaaataccaacgaaccgaaaaatcgaaaaccgaaaccgaaaaaacgaaaaaaaaaaaaacctaacgaaacacttaaaaaccaaccgaaaaacaaaaacacgaactcccactataaaaaaaaaaaccaaaa

SEQ ID NO: 24 - DNA, 162 bp, Homo sapiens
atcaacaaaaattccaccaaactccactacacaataacgcgcgaacgccgacgaacccgctacgcgactaacgatccaaaaacgaacacaacgcccgaacgaacgccgaaaaaaacgaacaaaaacgacgaaaaacgaaacaaaaaaaaaaaacaaatacca

SEQ ID NO: 25 - DNA, 408 bp, Homo sapiens
tttttaattttgtaggtttgaaagaaggttatatatgtatgtttatatttatattttatatgttttgttttaaataattttatgaatattgttttttgttttgttttttgggttattttttttgttgtttttttttagtttgttttgatttgttttttaaaagtatgtttttgtttttttgttgttttggtgttttttttttgatttattagggttgttgggttggtgtagattgttttttttttttttttattttatttttttttttggtttttttttttatagtgggagtttgtgtttttgttttttggttggtttttaagtgttttgttaggttttttttttttttgtttttttggttttggtttttgattttttggtttgttggtatttgttttttttttttgt

SEQ ID NO: 26 - DNA, 144 bp, Homo sapiens
ttttggtttttttttttatagtgggagtttgtgtttttgttttttggttggtttttaagtgttttgttaggttttttttttttttgtttttttggttttggtttttgattttttggtttgttggtatttgttttttttttttgt

SEQ ID NO: 27 - DNA, 162 bp, Homo sapiens
tggtatttgttttttttttttgttttgttttttgttgtttttgtttgttttttttggtgtttgtttgggtgttgtgtttgtttttggattgttagttgtgtagtgggtttgttggtgtttgtgtgttattgtgtagtggagtttggtggaatttttgttgat

SEQ ID NO: 28 - DNA, 408 bp, Homo sapiens
acaaaaaaaaaaaacaaataccaacaaaccaaaaaatcaaaaaccaaaaccaaaaaaacaaaaaaaaaaaaaacctaacaaaacacttaaaaaccaaccaaaaaacaaaaacacaaactcccactataaaaaaaaaaaccaaaaaaaaaaataaaataaaaaaaaaaaaaaaacaatctacaccaacccaacaaccctaataaatcaaaaaaaaaacaccaaaacaacaaaaaaacaaaaacatacttttaaaaaacaaatcaaaacaaactaaaaaaaaacaacaaaaaaaataacccaaaaaacaaaacaaaaaacaatattcataaaattatttaaaacaaaacatataaaatataaatataaacatacatatataaccttctttcaaacctacaaaattaaaaa

SEQ ID NO: 29 - DNA, 144 bp, Homo sapiens
acaaaaaaaaaaaacaaataccaacaaaccaaaaaatcaaaaaccaaaaccaaaaaaacaaaaaaaaaaaaaacctaacaaaacacttaaaaaccaaccaaaaaacaaaaacacaaactcccactataaaaaaaaaaaccaaaa

SEQ ID NO: 30 - DNA, 162 bp, Homo sapiens
atcaacaaaaattccaccaaactccactacacaataacacacaaacaccaacaaacccactacacaactaacaatccaaaaacaaacacaacacccaaacaaacaccaaaaaaaacaaacaaaaacaacaaaaaacaaaacaaaaaaaaaaaacaaatacca

SEQ ID NO: 31 - DNA, 22 bp, Homo sapiens
gtaggggagggaagtagatgtt

SEQ ID NO: 32 - DNA, 24 bp, Homo sapiens
ttctaatcctcctttccacaataa

SEQ ID NO: 33 - DNA, 20 bp, Homo sapiens
agtcggagtcgggagagcga

SEQ ID NO: 34 - DNA, 27 bp, Homo sapiens
agttggagttgggagagtgaaaggaga

SEQ ID NO: 35 - DNA, 144 bp, Homo sapiens
gcaggggagggaagcagatgccagcgggccgaagagtcgggagccggagccgggagagcgaaaggagaggggacctggcggggcacttaggagccaaccgaggagcaggagcacggactcccactgtggaaaggaggaccagaa

SEQ ID NO: 36 - DNA, 144 bp, Homo sapiens
gtaggggagggaagtagatgttagcgggtcgaagagtcgggagtcggagtcgggagagcgaaaggagaggggatttggcggggtatttaggagttaatcgaggagtaggagtacggatttttattgtggaaaggaggattagaa

SEQ ID NO: 37 - DNA, 144 bp, Homo sapiens
gtaggggagggaagtagatgttagtgggttgaagagttgggagttggagttgggagagtgaaaggagaggggatttggtggggtatttaggagttaattgaggagtaggagtatggatttttattgtggaaaggaggattagaa

SEQ ID NO: 38 - DNA, 21 bp, Homo sapiens
gtaggggagggaagtagatgt

SEQ ID NO: 39 - DNA, 22 bp, Homo sapiens
gagtgatagggataggtaggtg

SEQ ID NO: 40 - DNA, 23 bp, Homo sapiens
tcctcaactctacaaacctaaaa

SEQ ID NO: 41 - DNA, 27 bp, Homo sapiens
ccttaaactaaacaaaaactaaattcc

SEQ ID NO: 42 - DNA, 408 bp, Homo sapiens
gcaggggagggaagcagatgccagcgggccgaagagtcgggagccggagccgggagagcgaaaggagaggggacctggcggggcacttaggagccaaccgaggagcaggagcacggactcccactgtggaaaggaggaccagaagggaggatgggatggaagagaagaaaaagcaatctgcgccaacccggcagccctaataaatcaaagggggagcgccagggcagcggggagacagaaacgtacttttggggagcaaatcaggacgggctgggaggaagcgacagggaaagtggcccaagagacggaacaaaggacaatgttcatggggttgtttgggacgaggcgtgtggagtgtgggtgtgagcgtgcgtgtgtgaccttctttcaggcctgcagagttgagga

SEQ ID NO: 43 - DNA, 477 bp, Homo sapiens
gagtgacagggacaggtaggtgatattagatcccctgcggcggcagcagccgctgcagccacgacgcggccctctgagcgcaccctccgcaacgcgcacacgcacacccctcgggcggtcgaacaggagccgggccttgccgcagctcagctccaggcacccaggcgagcgacggaccagatctgcggctccgcgcttccctgttggcctaacatcttaaaaccagaggcgggcttcctggtgccgagacgtcactccgccgcggccctccccagccctctccgcctccgcctcctcccagacccttctccgggtgcgactgacgtggctccgcaccaatcaggacgccccgagccgcggtggagggactgtcctgcctgcacctatcagcagtgcggggccgggctactgcctcgccgtgcgcactgggtctacacaggcaagctcccgggaattcagctcctgcccagcccaagg

SEQ ID NO: 44 - DNA, 408 bp, Homo sapiens
gtaggggagggaagtagatgttagcgggtcgaagagtcgggagtcggagtcgggagagcgaaaggagaggggatttggcggggtatttaggagttaatcgaggagtaggagtacggatttttattgtggaaaggaggattagaagggaggatgggatggaagagaagaaaaagtaatttgcgttaattcggtagttttaataaattaaagggggagcgttagggtagcggggagatagaaacgtatttttggggagtaaattaggacgggttgggaggaagcgatagggaaagtggtttaagagacggaataaaggataatgtttatggggttgtttgggacgaggcgtgtggagtgtgggtgtgagcgtgcgtgtgtgatttttttttaggtttgtagagttgagga

SEQ ID NO: 45 - DNA, 477 bp, Homo sapiens
gagtgatagggataggtaggtgatattagattttttgcggcggtagtagtcgttgtagttacgacgcggttttttgagcgtatttttcgtaacgcgtatacgtatatttttcgggcggtcgaataggagtcgggttttgtcgtagtttagttttaggtatttaggcgagcgacggattagatttgcggtttcgcgtttttttgttggtttaatattttaaaattagaggcgggttttttggtgtcgagacgttatttcgtcgcggttttttttagtttttttcgttttcgtttttttttagattttttttcgggtgcgattgacgtggtttcgtattaattaggacgtttcgagtcgcggtggagggattgttttgtttgtatttattagtagtgcggggtcgggttattgtttcgtcgtgcgtattgggtttatataggtaagttttcgggaatttagtttttgtttagtttaagg

SEQ ID NO: 46 - DNA, 408 bp, Homo sapiens; identical to SEQ ID NO: 19

SEQ ID NO: 47 - DNA, 477 bp, Homo sapiens
ttttgggttgggtaggagttgaattttcgggagtttgtttgtgtagatttagtgcgtacggcgaggtagtagttcggtttcgtattgttgataggtgtaggtaggatagtttttttatcgcggttcggggcgttttgattggtgcggagttacgttagtcgtattcggagaagggtttgggaggaggcggaggcggagagggttggggagggtcgcggcggagtgacgtttcggtattaggaagttcgtttttggttttaagatgttaggttaatagggaagcgcggagtcgtagatttggttcgtcgttcgtttgggtgtttggagttgagttgcggtaaggttcggtttttgttcgatcgttcgaggggtgtgcgtgtgcgcgttgcggagggtgcgtttagagggtcgcgtcgtggttgtagcggttgttgtcgtcgtaggggatttaatattatttatttgtttttgttattt

SEQ ID NO: 48 - DNA, 408 bp, Homo sapiens
gtaggggagggaagtagatgttagtgggttgaagagttgggagttggagttgggagagtgaaaggagaggggatttggtggggtatttaggagttaattgaggagtaggagtatggatttttattgtggaaaggaggattagaagggaggatgggatggaagagaagaaaaagtaatttgtgttaatttggtagttttaataaattaaagggggagtgttagggtagtggggagatagaaatgtatttttggggagtaaattaggatgggttgggaggaagtgatagggaaagtggtttaagagatggaataaaggataatgtttatggggttgtttgggatgaggtgtgtggagtgtgggtgtgagtgtgtgtgtgtgatttttttttaggtttgtagagttgagga

SEQ ID NO: 49 - DNA, 477 bp, Homo sapiens
gagtgatagggataggtaggtgatattagattttttgtggtggtagtagttgttgtagttatgatgtggttttttgagtgtattttttgtaatgtgtatatgtatattttttgggtggttgaataggagttgggttttgttgtagtttagttttaggtatttaggtgagtgatggattagatttgtggttttgtgtttttttgttggtttaatattttaaaattagaggtgggttttttggtgttgagatgttattttgttgtggttttttttagttttttttgtttttgtttttttttagatttttttttgggtgtgattgatgtggttttgtattaattaggatgttttgagttgtggtggagggattgttttgtttgtatttattagtagtgtggggttgggttattgttttgttgtgtgtattgggtttatataggtaagtttttgggaatttagtttttgtttagtttaagg

SEQ ID NO: 50 - DNA, 408 bp, Homo sapiens; identical to SEQ ID NO: 25

SEQ ID NO: 51 - DNA, 477 bp, Homo sapiens
ttttgggttgggtaggagttgaatttttgggagtttgtttgtgtagatttagtgtgtatggtgaggtagtagtttggttttgtattgttgataggtgtaggtaggatagtttttttattgtggtttggggtgttttgattggtgtggagttatgttagttgtatttggagaagggtttgggaggaggtggaggtggagagggttggggagggttgtggtggagtgatgttttggtattaggaagtttgtttttggttttaagatgttaggttaatagggaagtgtggagttgtagatttggtttgttgtttgtttgggtgtttggagttgagttgtggtaaggtttggtttttgtttgattgtttgaggggtgtgtgtgtgtgtgttgtggagggtgtgtttagagggttgtgttgtggttgtagtggttgttgttgttgtaggggatttaatattatttatttgtttttgttattt

SEQ ID NO: 52 - DNA, 16 bp, Homo sapiens
agtagtgcggggtcgg

SEQ ID NO: 53 - DNA, 17 bp, Homo sapiens
agtagtgtggggttggg

SEQ ID NO: 54 - DNA, 17 bp, Homo sapiens
tgtagttacgacgcggt

SEQ ID NO: 55 - DNA, 22 bp, Homo sapiens
gttgtagttatgatgtggtttt

SEQ ID NO: 56 - DNA, 16 bp, Homo sapiens
tttcgggcggtcgaat

SEQ ID NO: 57 - DNA, 20 bp, Homo sapiens
ttttgggtggttgaatagga

SEQ ID NO: 58 - DNA, 16 bp, Homo sapiens
taggcgagcgacggat

SEQ ID NO: 59 - DNA, 21 bp, Homo sapiens
taggtgagtgatggattagat

SEQ ID NO: 60 - DNA, 19 bp, Homo sapiens
tgtcgagacgttatttcgt

SEQ ID NO: 61 - DNA, 22 bp, Homo sapiens
tggtgttgagatgttattttgt

SEQ ID NO: 62 - DNA, 18 bp, Homo sapiens
agttgggagagtgaaagg

SEQ ID NO: 63 - DNA, 16 bp, Homo sapiens
gagtcgggagagcgaa

SEQ ID NO: 64 - DNA, 19 bp, Homo sapiens
tttgcgttaattcggtagt

SEQ ID NO: 65 - DNA, 23 bp, Homo sapiens
tttgtgttaatttggtagtttta

SEQ ID NO: 66 - DNA, 18 bp, Homo sapiens
agcgttagggtagcgggg

SEQ ID NO: 67 - DNA, 18 bp, Homo sapiens
ggagtgttagggtagtgg

SEQ ID NO: 68 - DNA, 17 bp, Homo sapiens
gggatgaggtgtgtgga

SEQ ID NO: 69 - DNA, 16 bp, Homo sapiens
ttgggacgaggcgtgt

SEQ ID NO: 70 - DNA, 18 bp, Homo sapiens
agcgggtcgaagagtcgg

SEQ ID NO: 71 - DNA, 18 bp, Homo sapiens
agtgggttgaagagttgg